European Patent Specification EP 3 516 056 B1, published November 27, 2024. Title: A GUIDE-RNA EXPRESSION SYSTEM FOR A HOST CELL. Applicant: DSM IP ASSETS B.V., MIT. The sequence listing filed with the application follows.

SEQUENCE LISTING (76 sequences)

SEQ ID NO: 1 - DNA, 28 bp, Artificial Sequence
  Nucleotide sequence of forward primer used to amplify the 5' piece for integration into the INT1 locus
ttaccaatcctttcataagctaattatg

SEQ ID NO: 2 - DNA, 80 bp, Artificial Sequence
  Nucleotide sequence of reverse primer used to amplify the 5' piece for integration into the INT1 locus
ggcacaaacgcctgtgggtgtggtactggatatgcaaagcgattggaagtcgcttagggtttcaaagatccatacttctc

SEQ ID NO: 3 - DNA, 80 bp, Artificial Sequence
  Nucleotide sequence of forward primer used to amplify the 3' piece for integration into the INT1 locus
tgtttcttgtatatagtaatatgtaatatttgcttcgtacgcttagtcctcattttactttttttagaatgacctgttcc

SEQ ID NO: 4 - DNA, 23 bp, Artificial Sequence
  Nucleotide sequence of reverse primer used to amplify the 3' piece for integration into the INT1 locus
ttgtgaccgccctgctgcaaaac

SEQ ID NO: 5 - DNA, 9360 bp, Artificial Sequence
  Nucleotide sequence of the GFP-dCas9-Mxi1 expression unit integrated in the genome
  misc_feature (1)..(418): 5' INT1 integration site
  misc_feature (419)..(1814): GFP expression cassette
  misc_feature (1819)..(1864): connector sequence
  misc_feature (1869)..(1918): connector sequence
  misc_feature (1923)..(3735): hygromycin B resistance marker cassette
  misc_feature (3747)..(3796): connector sequence
  misc_feature (3797)..(4401): GAL1 promoter
  misc_feature (4402)..(8736): dCAS9-Mxi1
  misc_feature (8737)..(8977): terminator
  misc_feature (8798)..(9028): connector sequence
  misc_feature (9029)..(9362): 3' INT1 integration site
ttaccaatcctttcataagctaattatgccatccatatagcaagagaatccggtgggggcgccatgcctatccggcggcaacattattactctggtatacgggcgtaactccataatatgccaccacttacctttaacatgttcatggtaggtaccccacccagccataaggaaattttcaaaggcgttggatcaaaaaataggcctttatttcatcgcgtgattgaggagcataacatgtttagtgaaggtttcttttggaaaacttcagtcgctcattattagaaccagggaggtccaggctttgctggtgggagagaaagcttatgaagctggggttgcagatttgtcgattggtcgccagtacacagttttaaaaagtcagagaatgtagagaagtatggatctttgaaaccctaagcgacttccaatcgctttgcatatccagtaccacacccacaggcgtttgtgccattcatctttcacctgccattagtaacccgacttctcattgagcgggttacggcagccacaggccacattccgaatgtctgggtgagcggtcccttttccagcatccactaaatatctcggatcccgctttttaatctggcttcctgaaaaaaatcaatggagtgatgcaaactgactggagcaaaaagctgacacaaggcaatcgacctacgtgtctgtctattttctcacaccttctattaccttctaactctctgggttggaaaaaactgaaaaaaaggttgtctccagtttccacaaatcatccccctgtttgattaataaatatataaagacgacaactatcgatcataaactcataaaactataactcctttacacttcttattttatagttattctattttaattcttattgattttaaaaccccaagaacttagtttcgaaaacacacacacacaaacaattaaaaatgtctaaaggtgaagaattattcactggtgttgtcccaattttggttgaattagatggtgatgttaatggtcacaaattttctgtctccggtgaaggtgaaggtgatgctacttacggtaaattgaccttaaaattgatttgtactactggtaaattgccagttccatggccaaccttagtcactactttaggttatggtttgcaatgttttgctagatacccagatcatatgaaacaacatgactttttcaagtctgccatgccagaaggttatgttcaagaaagaactatttttttcaaagatgacggtaactacaagaccagagctgaagtcaagtttgaaggtgataccttagttaatagaatcgaattaaaaggtattgattttaaagaagatggtaacattttaggtcacaaattggaatacaactataactctcacaatgtttacatcactgctgacaaacaaaagaatggtatcaaagctaacttcaaaattagacacaacattgaagatggtggtgttcaattagctgaccattatcaacaaaatactccaattggtgatggtccagtcttgttaccagacaaccattacttatcctatcaatctgccttatccaaagatccaaacgaaaagagagatcacatggtcttgttagaatttgttactgctgctggtattacccatggtatggatgaattgtacaaataaactggttgatggaaaatataattttattgggcaaacttttgtttatctgatgtgttttatactattatctttttaattaatgattctatatacaaacctgtatattttttctttaaccaatttttttttttatagacctagagctgtactcctcaacgttgtccaggtttgtatccacgtgtgtccgttccgccaatattccgccggatcgatgtacacaaccgactgcacccaaacgaacacaaatcttagcagtgctatttaaaaacctgtgttatgctcaaataacggttactgatccaaaaccttatatatgacggcaagtgtctcactgttgcattacgcgttgtttcttttctttgttcttgtaagcgcgattttaccagaactagatggcgctcgtgatcctgaaacggggagaaattttgagaacaccgctttattaggcgaagcggtgggcacagctcacgcgtaaggtgttcccattatttctcaaagtgatgcgaatttcagagaacacattaacctgggggccataaacgcgacgtgctaccattttcgttacgtatacttaggccagagattacaacatgactactaatatcaaacataactctatatataagggatgaagatgtatgctttcttagaatttcaaacatgttccgttaaagttttacttttcgatttcaatttcgactgcatgatgcttttcttagagagtgttttgttattaaatagtatcataaattcttgtctttttacataagaattaggaaagtacagaacaagagcaaatttaatatataatgggtaaaaagcctgaactcaccgcgacgtctgtcgagaagtttctgatcgaaaagttcgacagcgtctccgacctgatgcagctctcggagggcgaagaatctcgtgctttcagcttcgatgtaggagggcgtggatatgtcctgcgggtaaatagctgcgccgatggtttctacaaagatcgttatgtttatcggcactttgcatcggccgcgctcccgattccggaagtgcttgacattggggaattcagcgagagcctgacctattgcatctcccgccgtgcacagggtgtcacgttgcaagacctgcctgaaaccgaactgcccgctgttctgcagccggtcgcggaggcaatggatgcgatcgctgcggccgatcttagccagacgagcgggttcggcccattcggaccgcaaggaatcggtcaatacactacatggcgtgatttcatatgcgcgattgctgatccccatgtgtatcactggcaaactgtgatggacgacaccgtcagtgcgtccgtcgcgcaggctctcgatgagctgatgctttgggccgaggactgccccgaagtccggcacctcgtgcacgcggatttcggctccaacaatgtcctgacggacaatggccgcataacagcggtcattgactggagcgaggcgatgttcggggattcccaatacgaggtcgccaacatcttcttctggaggccgtggttggcttgtatggagcagcagacgcgctacttcgagcggaggcatccggagcttgcaggatcgccgcggctccgggcgtatatgctccgcattggtcttgaccaactctatcagagcttggttgacggcaatttcgatgatgcagcttgggcgcagggtcgatgcgacgcaatcgtccgatccggagccgggactgtcgggcgtacacaaatcgcccgcagaagcgcggccgtctggaccgatggctgtgtagaagtactcgccgatagtggaaaccgacgccccagcactcgtccgagggcaaaggaataaacagtactgacaataaaaagattcttgttttcaagaacttgtcatttgtatagtttttttatattgtagttgttctattttaatcaaatgttagcgtgatttatattttttttcgcctcgacatcatctgcccagatgcgaagttaagtgcgcagaaagtaatatcatgcgtcaatcgtatgtgaatgctggtcgctatactgctgtcgattcgatactaacgccgccatccagtgtcgacctcacgctttccggcatcttccagaccacagtatatccatccgcctcctgttggtgcacatggcattaccaccatatacatatccatatctaatcttacttatatgttgtggaaatgtaaagagccccattatcttagcctaaaaaaaccttctctttggaactttcagtaatacgcttaactgctcattgctatattgaagtacggattagaagccgccgagcgggcgacagccctccgacggaagtctctcctccgtgcgtcctcgtgttcaccggtcgcgttcctgaaacgcagatgtgcctcgcgccgcactgctccgaacaataaagattctacaatactagcttttatggttatgaagaggaaaaattggcagtaacctggccccacaaaccttcaaatcaacgaatcaaattaacaaccataggataataatgcgattagttttttagccttatttctggggtaattaatcagcgaagcgatgatttttgatctattaacagatatataaatgcaaaagctgcataaccactttaactaatactttcaacattttcggtttgtattacttcttattcaaatgtcataaaagtatcaacaaaaaattgttaatatacctctatactttaacgtcaaggagaaaaaactataaatgtctagagccccaaagaagaagagaaaagttagacccggggataagaaatactctattggtttggctatcggtacaaactctgttggttgggctgttattactgatgaatacaaggttccatccaagaagttcaaggttttgggtaacactgatagacactccatcaaaaagaacttgattggtgccttgttgttcgattctggtgaaactgctgaagctactagattgaaaagaaccgctagaagaagatacaccagaagaaagaacagaatctgctacttgcaagaaatcttctccaacgaaatggccaaggttgatgattcattcttccacagattggaagaatccttcttggtcgaagaagataagaagcacgaaagacatccaatcttcggtaacatcgttgatgaagttgcttaccacgaaaagtacccaactatctaccatttgagaaagaagttggttgactctaccgataaggctgatttgagattgatctatttggctttggcccacatgattaagttcagaggtcatttcttgatcgaaggtgatttgaacccagataactccgatgttgataagttgttcatccaattagtccaaacctacaatcaattattcgaagaaaacccaatcaacgcctctggtgttgatgctaaagctattttgtctgccagattgtccaagtccagaagattagaaaatttgatcgcccaattaccaggtgaaaagaagaatggtttgttcggtaatttgattgccttgtctttgggtttgactccaaacttcaagtccaatttcgatttggctgaagatgccaagttgcaattatctaaggatacctacgatgacgatttggataacttgttggctcaaatcggtgatcaatacgctgatttgtttttggctgctaagaacttgtccgatgccattttgttgtccgatattttgagagtcaacaccgaaattactaaggctccattgtctgcctctatgatcaaaagatacgatgaacaccaccaagacttgactttgttgaaggctttggtcagacaacaattacctgaaaagtacaaagaaattttcttcgatcaatccaagaacggttacgccggttatattgatggtggtgcttctcaagaagaattttacaagttcatcaagccaatcttggaaaagatggacggtactgaagaattattggtcaagttgaacagagaagatttgttgagaaagcaaagaaccttcgacaacggttctattccacatcaaattcacttgggtgaattgcacgcaattttgagaagacaagaagatttttatccattcttgaaggacaacagagaaaagatcgaaaagattctgaccttcagaatcccttactacgttggtccattggctagaggtaattcaagatttgcctggatgactagaaagtccgaagaaactattactccttggaacttcgaagaagttgtagataagggtgcttctgcccaatcctttattgaaagaatgaccaacttcgacaagaacttgccaaacgaaaaggttttgccaaagcactctttgttgtacgaatacttcaccgtctacaacgaattgactaaggttaagtacgtcaccgaaggtatgagaaaaccagcttttttatccggtgaacaaaagaaggctatcgtcgatttgttgttcaagaccaacagaaaggttactgtcaagcaattaaaagaagattacttcaagaaaatcgaatgcttcgactccgttgaaatttctggtgtcgaagatagattcaatgcctctttaggtacttaccatgacttgttgaaaatcatcaaggacaaggatttcttggacaacgaagaaaacgaagatattttggaagatattgtcttgacattgaccttgtttgaagatagagaaatgattgaagaaagattgaaaacctacgcccacttgttcgatgataaggttatgaagcaattaaagagaagaagatacactggttggggtagattgtccagaaaattgattaacggtatcagagacaagcaatccggtaagaccattttggactttttgaagtctgatggtttcgctaacagaaacttcatgcaattaatccacgacgattccttgactttcaaagaagatatacaaaaggcccaagtctctggtcaaggtgattctttacatgaacatatcgctaacttggctggttctccagctattaagaagggtattttacaaaccgttaaggtcgttgacgaattggtcaaagttatgggtagacataagccagaaaacatcgttatcgaaatggctagagaaaatcaaaccacccaaaagggtcaaaagaactccagagaaagaatgaagagaatcgaagaaggtatcaaagaattgggttcccaaattttgaaagaacacccagttgaaaacacccaattacaaaacgaaaagttgtacttgtactacttgcaaaacggtagagatatgtacgttgaccaagaattggacatcaacagattgtctgattacgatgttgacgctatcgttccacaatcttttttgaaggatgactccattgacaacaaggtcttgactagatccgataagaatagaggtaagtccgataacgttccatctgaagaagtcgttaagaaaatgaagaactattggagacaattattgaacgccaagttgatcacccaaagaaagtttgacaatttgaccaaggctgaaagaggtggtttgtctgaattggataaggcaggtttcatcaaaagacaattagtagaaaccagacaaatcaccaagcacgttgctcaaattttggatagtagaatgaacactaagtacgacgaaaacgacaaattgatcagagaagttaaggtcattaccttgaagtccaagttggtttccgatttcagaaaggacttccaattctacaaggtcagagaaatcaacaactaccatcatgcacatgatgcttacttgaatgctgttgttggtactgccttgattaagaagtatccaaagttggaatccgaatttgtctacggtgattacaaggtttacgacgttagaaagatgatcgccaagtccgaacaagaaattggtaaagctactgccaaatacttcttctactccaatattatgaatttctttaagaccgaaatcactttggccaacggtgaaattagaaaaagaccattgattgaaactaatggtgaaacaggtgaaatcgtttgggataagggtagagattttgccactgttagaaaggtattgtccatgccacaagtaaacatcgtcaaaaagaccgaagttcaaactggtggtttctccaaagaatccattttgcctaagagaaactccgataagttgatcgctagaaaaaaagactgggacccaaaaaagtacggtggttttgattctccaactgttgcttactctgttttggttgttgctaaggtcgaaaagggtaagagtaagaagttgaagtccgtcaaagaattattaggtatcactatcatggaaagatcctcattcgaaaagaatcctatcgactttttggaagccaagggttacaaagaagtcaagaaggacttgatcattaagttgccaaagtacagtttgttcgaattggaaaatggtagaaagagaatgttggcttctgccggtgaattacaaaagggtaatgaattggctttgccatccaagtacgttaatttcttatacttggcctcccactacgaaaaattgaaaggttctcctgaagataacgaacaaaagcaattatttgtcgaacaacacaagcactacttggacgaaatcattgaacaaatttccgaattttccaaaagagtcattttggctgacgccaatttggacaaagttttgtcagcttacaacaagcacagagataagccaattagagaacaagctgaaaacatcattcacttgttcactttgactaacttgggtgctccagctgcttttaagtatttcgataccactatcgacagaaagagatacacctctaccaaagaagttttggacgctactttgatccaccaatctattactggtttgtacgaaactagaatcgacttgtctcaattaggtggtgatgagggagctcccaagaaaaagcgcaaggtaggtagttccaagcttggcggcagcggcggcagcatggaacgtgtgagaatgattaatgtgcaaaggctgttagaagccgcagagtttttagaaagaagagaaagagaatgcgaacacgggtatgccagttctttccctagcatgccctctcccagaggctaaataggctaatatgaatgtatttgatctctattttattaatacgaaaccccttaataattgatattttcgatacatatttggcagtagttagctacgtaacagagtattattttcatttcaagttatgcatgaactctctaatttcacataccatgctaccactacccttggaggttttgttcatatcttttataataaagctaaaaccgaaaaggtgaagggaaaaaaaactattagagcctgtttcttgtatatagtaatatgtaatatttgcttcgtacgcttagtcctcattttactttttttagaatgacctgttcccgacactatgtaagatctagcttttaacatattatggaaacctgaaatgtaaaatctgaatttttgtatatgtgtttatatttgggtagttcttttgaggaaagcatgcatagacttgctgtacgaactttatgtgacttgtagtgacgctgtttcatgagactttagccctttgaacatattatcatatctcagcttgaaatactatagatttacttttgcagccatttcttggtgctccaaggttgtgcgtatctattacttaatttctgtccttgccaagttttgcagcagggcggtcac

SEQ ID NO: 6 - DNA, 11243 bp, Artificial Sequence
  Nucleotide sequence of the GFP-dCas9-Mxi1-T7RNAp expression unit integrated in the genome
  misc_feature (1)..(418): 5' INT1 integration site
  misc_feature (419)..(468): connector sequence
  misc_feature (473)..(1814): GFP expression cassette
  misc_feature (1819)..(1868): connector sequence
  misc_feature (1869)..(1918): connector sequence
  misc_feature (1923)..(3735): hygromycin B resistance marker cassette
  misc_feature (3747)..(3796): connector sequence
  misc_feature (3797)..(4401): GAL1 promoter
  misc_feature (4402)..(8733): dCAS9-Mxi1
  misc_feature (8734)..(8787): 2A peptide sequence
  misc_feature (8788)..(10617): T7 RNA polymerase
  misc_feature (10618)..(10858): terminator
  misc_feature (10859)..(10909): connector sequence
  misc_feature (10910)..(11243): 3' INT1 integration site
ttaccaatcctttcataagctaattatgccatccatatagcaagagaatccggtgggggcgccatgcctatccggcggcaacattattactctggtatacgggcgtaactccataatatgccaccacttacctttaacatgttcatggtaggtaccccacccagccataaggaaattttcaaaggcgttggatcaaaaaataggcctttatttcatcgcgtgattgaggagcataacatgtttagtgaaggtttcttttggaaaacttcagtcgctcattattagaaccagggaggtccaggctttgctggtgggagagaaagcttatgaagctggggttgcagatttgtcgattggtcgccagtacacagttttaaaaagtcagagaatgtagagaagtatggatctttgaaaccctaagcgacttccaatcgctttgcatatccagtaccacacccacaggcgtttgtgccattcatctttcacctgccattagtaacccgacttctcattgagcgggttacggcagccacaggccacattccgaatgtctgggtgagcggtcccttttccagcatccactaaatatctcggatcccgctttttaatctggcttcctgaaaaaaatcaatggagtgatgcaaactgactggagcaaaaagctgacacaaggcaatcgacctacgtgtctgtctattttctcacaccttctattaccttctaactctctgggttggaaaaaactgaaaaaaaggttgtctccagtttccacaaatcatccccctgtttgattaataaatatataaagacgacaactatcgatcataaactcataaaactataactcctttacacttcttattttatagttattctattttaattcttattgattttaaaaccccaagaacttagtttcgaaaacacacacacacaaacaattaaaaatgtctaaaggtgaagaattattcactggtgttgtcccaattttggttgaattagatggtgatgttaatggtcacaaattttctgtctccggtgaaggtgaaggtgatgctacttacggtaaattgaccttaaaattgatttgtactactggtaaattgccagttccatggccaaccttagtcactactttaggttatggtttgcaatgttttgctagatacccagatcatatgaaacaacatgactttttcaagtctgccatgccagaaggttatgttcaagaaagaactatttttttcaaagatgacggtaactacaagaccagagctgaagtcaagtttgaaggtgataccttagttaatagaatcgaattaaaaggtattgattttaaagaagatggtaacattttaggtcacaaattggaatacaactataactctcacaatgtttacatcactgctgacaaacaaaagaatggtatcaaagctaacttcaaaattagacacaacattgaagatggtggtgttcaattagctgaccattatcaacaaaatactccaattggtgatggtccagtcttgttaccagacaaccattacttatcctatcaatctgccttatccaaagatccaaacgaaaagagagatcacatggtcttgttagaatttgttactgctgctggtattacccatggtatggatgaattgtacaaataaactggttgatggaaaatataattttattgggcaaacttttgtttatctgatgtgttttatactattatctttttaattaatgattctatatacaaacctgtatattttttctttaaccaatttttttttttatagacctagagctgtactcctcaacgttgtccaggtttgtatccacgtgtgtccgttccgccaatattccgccggatcgatgtacacaaccgactgcacccaaacgaacacaaatcttagcagtgctatttaaaaacctgtgttatgctcaaataacggttactgatccaaaaccttatatatgacggcaagtgtctcactgttgcattacgcgttgtttcttttctttgttcttgtaagcgcgattttaccagaactagatggcgctcgtgatcctgaaacggggagaaattttgagaacaccgctttattaggcgaagcggtgggcacagctcacgcgtaaggtgttcccattatttctcaaagtgatgcgaatttcagagaacacattaacctgggggccataaacgcgacgtgctaccattttcgttacgtatacttaggccagagattacaacatgactactaatatcaaacataactctatatataagggatgaagatgtatgctttcttagaatttcaaacatgttccgttaaagttttacttttcgatttcaatttcgactgcatgatgcttttcttagagagtgttttgttattaaatagtatcataaattcttgtctttttacataagaattaggaaagtacagaacaagagcaaatttaatatataatgggtaaaaagcctgaactcaccgcgacgtctgtcgagaagtttctgatcgaaaagttcgacagcgtctccgacctgatgcagctctcggagggcgaagaatctcgtgctttcagcttcgatgtaggagggcgtggatatgtcctgcgggtaaatagctgcgccgatggtttctacaaagatcgttatgtttatcggcactttgcatcggccgcgctcccgattccggaagtgcttgacattggggaattcagcgagagcctgacctattgcatctcccgccgtgcacagggtgtcacgttgcaagacctgcctgaaaccgaactgcccgctgttctgcagccggtcgcggaggcaatggatgcgatcgctgcggccgatcttagccagacgagcgggttcggcccattcggaccgcaaggaatcggtcaatacactacatggcgtgatttcatatgcgcgattgctgatccccatgtgtatcactggcaaactgtgatggacgacaccgtcagtgcgtccgtcgcgcaggctctcgatgagctgatgctttgggccgaggactgccccgaagtccggcacctcgtgcacgcggatttcggctccaacaatgtcctgacggacaatggccgcataacagcggtcattgactggagcgaggcgatgttcggggattcccaatacgaggtcgccaacatcttcttctggaggccgtggttggcttgtatggagcagcagacgcgctacttcgagcggaggcatccggagcttgcaggatcgccgcggctccgggcgtatatgctccgcattggtcttgaccaactctatcagagcttggttgacggcaatttcgatgatgcagcttgggcgcagggtcgatgcgacgcaatcgtccgatccggagccgggactgtcgggcgtacacaaatcgcccgcagaagcgcggccgtctggaccgatggctgtgtagaagtactcgccgatagtggaaaccgacgccccagcactcgtccgagggcaaaggaataaacagtactgacaataaaaagattcttgttttcaagaacttgtcatttgtatagtttttttatattgtagttgttctattttaatcaaatgttagcgtgatttatattttttttcgcctcgacatcatctgcccagatgcgaagttaagtgcgcagaaagtaatatcatgcgtcaatcgtatgtgaatgctggtcgctatactgctgtcgattcgatactaacgccgccatccagtgtcgacctcacgctttccggcatcttccagaccacagtatatccatccgcctcctgttggtgcacatggcattaccaccatatacatatccatatctaatcttacttatatgttgtggaaatgtaaagagccccattatcttagcctaaaaaaaccttctctttggaactttcagtaatacgcttaactgctcattgctatattgaagtacggattagaagccgccgagcgggcgacagccctccgacggaagtctctcctccgtgcgtcctcgtgttcaccggtcgcgttcctgaaacgcagatgtgcctcgcgccgcactgctccgaacaataaagattctacaatactagcttttatggttatgaagaggaaaaattggcagtaacctggccccacaaaccttcaaatcaacgaatcaaattaacaaccataggataataatgcgattagttttttagccttatttctggggtaattaatcagcgaagcgatgatttttgatctattaacagatatataaatgcaaaagctgcataaccactttaactaatactttcaacattttcggtttgtattacttcttattcaaatgtcataaaagtatcaacaaaaaattgttaatatacctctatactttaacgtcaaggagaaaaaactataaatgtctagagccccaaagaagaagagaaaagttagacccggggataagaaatactctattggtttggctatcggtacaaactctgttggttgggctgttattactgatgaatacaaggttccatccaagaagttcaaggttttgggtaacactgatagacactccatcaaaaagaacttgattggtgccttgttgttcgattctggtgaaactgctgaagctactagattgaaaagaaccgctagaagaagatacaccagaagaaagaacagaatctgctacttgcaagaaatcttctccaacgaaatggccaaggttgatgattcattcttccacagattggaagaatccttcttggtcgaagaagataagaagcacgaaagacatccaatcttcggtaacatcgttgatgaagttgcttaccacgaaaagtacccaactatctaccatttgagaaagaagttggttgactctaccgataaggctgatttgagattgatctatttggctttggcccacatgattaagttcagaggtcatttcttgatcgaaggtgatttgaacccagataactccgatgttgataagttgttcatccaattagtccaaacctacaatcaattattcgaagaaaacccaatcaacgcctctggtgttgatgctaaagctattttgtctgccagattgtccaagtccagaagattagaaaatttgatcgcccaattaccaggtgaaaagaagaatggtttgttcggtaatttgattgccttgtctttgggtttgactccaaacttcaagtccaatttcgatttggctgaagatgccaagttgcaattatctaaggatacctacgatgacgatttggataacttgttggctcaaatcggtgatcaatacgctgatttgtttttggctgctaagaacttgtccgatgccattttgttgtccgatattttgagagtcaacaccgaaattactaaggctccattgtctgcctctatgatcaaaagatacgatgaacaccaccaagacttgactttgttgaaggctttggtcagacaacaattacctgaaaagtacaaagaaattttcttcgatcaatccaagaacggttacgccggttatattgatggtggtgcttctcaagaagaattttacaagttcatcaagccaatcttggaaaagatggacggtactgaagaattattggtcaagttgaacagagaagatttgttgagaaagcaaagaaccttcgacaacggttctattccacatcaaattcacttgggtgaattgcacgcaattttgagaagacaagaagatttttatccattcttgaaggacaacagagaaaagatcgaaaagattctgaccttcagaatcccttactacgttggtccattggctagaggtaattcaagatttgcctggatgactagaaagtccgaagaaactattactccttggaacttcgaagaagttgtagataagggtgcttctgcccaatcctttattgaaagaatgaccaacttcgacaagaacttgccaaacgaaaaggttttgccaaagcactctttgttgtacgaatacttcaccgtctacaacgaattgactaaggttaagtacgtcaccgaaggtatgagaaaaccagcttttttatccggtgaacaaaagaaggctatcgtcgatttgttgttcaagaccaacagaaaggttactgtcaagcaattaaaagaagattacttcaagaaaatcgaatgcttcgactccgttgaaatttctggtgtcgaagatagattcaatgcctctttaggtacttaccatgacttgttgaaaatcatcaaggacaaggatttcttggacaacgaagaaaacgaagatattttggaagatattgtcttgacattgaccttgtttgaagatagagaaatgattgaagaaagattgaaaacctacgcccacttgttcgatgataaggttatgaagcaattaaagagaagaagatacactggttggggtagattgtccagaaaattgattaacggtatcagagacaagcaatccggtaagaccattttggactttttgaagtctgatggtttcgctaacagaaacttcatgcaattaatccacgacgattccttgactttcaaagaagatatacaaaaggcccaagtctctggtcaaggtgattctttacatgaacatatcgctaacttggctggttctccagctattaagaagggtattttacaaaccgttaaggtcgttgacgaattggtcaaagttatgggtagacataagccagaaaacatcgttatcgaaatggctagagaaaatcaaaccacccaaaagggtcaaaagaactccagagaaagaatgaagagaatcgaagaaggtatcaaagaattgggttcccaaattttgaaagaacacccagttgaaaacacccaattacaaaacgaaaagttgtacttgtactacttgcaaaacggtagagatatgtacgttgaccaagaattggacatcaacagattgtctgattacgatgttgacgctatcgttccacaatcttttttgaaggatgactccattgacaacaaggtcttgactagatccgataagaatagaggtaagtccgataacgttccatctgaagaagtcgttaagaaaatgaagaactattggagacaattattgaacgccaagttgatcacccaaagaaagtttgacaatttgaccaaggctgaaagaggtggtttgtctgaattggataaggcaggtttcatcaaaagacaattagtagaaaccagacaaatcaccaagcacgttgctcaaattttggatagtagaatgaacactaagtacgacgaaaacgacaaattgatcagagaagttaaggtcattaccttgaagtccaagttggtttccgatttcagaaaggacttccaattctacaaggtcagagaaatcaacaactaccatcatgcacatgatgcttacttgaatgctgttgttggtactgccttgattaagaagtatccaaagttggaatccgaatttgtctacggtgattacaaggtttacgacgttagaaagatgatcgccaagtccgaacaagaaattggtaaagctactgccaaatacttcttctactccaatattatgaatttctttaagaccgaaatcactttggccaacggtgaaattagaaaaagaccattgattgaaactaatggtgaaacaggtgaaatcgtttgggataagggtagagattttgccactgttagaaaggtattgtccatgccacaagtaaacatcgtcaaaaagaccgaagttcaaactggtggtttctccaaagaatccattttgcctaagagaaactccgataagttgatcgctagaaaaaaagactgggacccaaaaaagtacggtggttttgattctccaactgttgcttactctgttttggttgttgctaaggtcgaaaagggtaagagtaagaagttgaagtccgtcaaagaattattaggtatcactatcatggaaagatcctcattcgaaaagaatcctatcgactttttggaagccaagggttacaaagaagtcaagaaggacttgatcattaagttgccaaagtacagtttgttcgaattggaaaatggtagaaagagaatgttggcttctgccggtgaattacaaaagggtaatgaattggctttgccatccaagtacgttaatttcttatacttggcctcccactacgaaaaattgaaaggttctcctgaagataacgaacaaaagcaattatttgtcgaacaacacaagcactacttggacgaaatcattgaacaaatttccgaattttccaaaagagtcattttggctgacgccaatttggacaaagttttgtcagcttacaacaagcacagagataagccaattagagaacaagctgaaaacatcattcacttgttcactttgactaacttgggtgctccagctgcttttaagtatttcgataccactatcgacagaaagagatacacctctaccaaagaagttttggacgctactttgatccaccaatctattactggtttgtacgaaactagaatcgacttgtctcaattaggtggtgatgagggagctcccaagaaaaagcgcaaggtaggtagttccaagcttggcggcagcggcggcagcatggaacgtgtgagaatgattaatgtgcaaaggctgttagaagccgcagagtttttagaaagaagagaaagagaatgcgaacacgggtatgccagttctttccctagcatgccctctcccagaggcgagggtaggggtagtctgttgacttgtggggacgttgaggagaatcctggacccatgccaaagaagaaaaggaaggttcgtcctgggaacacgattaacatcgctaagaacgacttctctgacatcgaactggctgctatcccgttcaacactctggctgaccattacggtgagcgtttagctcgcgaacagttggcccttgagcatgagtcttacgagatgggtgaagcacgcttccgcaagatgtttgagcgtcaacttaaagctggtgaggttgcggataacgctgccgccaagcctctcatcactaccctactccctaagatgattgcacgcatcaacgactggtttgaggaagtgaaagctaagcgcggcaagcgcccgacagccttccagttcctgcaagaaatcaagccggaagccgtagcgtacatcaccattaagaccactctggcttgcctaaccagtgctgacaatacaaccgttcaggctgtagcaagcgcaatcggtcgggccattgaggacgaggctcgcttcggtcgtatccgtgaccttgaagctaagcacttcaagaaaaacgttgaggaacaactcaacaagcgcgtagggcacgtctacaagaaagcatttatgcaagttgtcgaggctgacatgctctctaagggtctactcggtggcgaggcgtggtcttcgtggcataaggaagactctattcatgtaggagtacgctgcatcgagatgctcattgagtcaaccggaatggttagcttacaccgccaaaatgctggcgtagtaggtcaagactctgagactatcgaactcgcacctgaatacgctgaggctatcgcaacccgtgcaggtgcgctggctggcatctctccgatgttccaaccttgcgtagttcctcctaagccgtggactggcattactggtggtggctattgggctaacggtcgtcgtcctctggcgctggtgcgtactcacagtaagaaagcactgatgcgctacgaagacgtttacatgcctgaggtgtacaaagcgattaacattgcgcaaaacaccgcatggaaaatcaacaagaaagtcctagcggtcgccaacgtaatcaccaagtggaagcattgtccggtcgaggacatccctgcgattgagcgtgaagaactcccgatgaaaccggaagacatcgacatgaatcctgaggctctcaccgcgtggaaacgtgctgccgctgctgtgtaccgcaaggacaaggctcgcaagtctcgccgtatcagccttgagttcatgcttgagcaagccaataagtttgctaaccataaggccatctggttcccttacaacatggactggcgcggtcgtgtttacgctgtgtcaatgttcaacccgcaaggtaacgatatgaccaaaggactgcttacgctggcgaaaggtaaaccaatcggtaaggaaggttactactggctgaaaatccacggtgcaaactgtgcgggtgtcgataaggttccgttccctgagcgcatcaagttcattgaggaaaaccacgagaacatcatggcttgcgctaagtctccactggagaacacttggtgggctgagcaagattctccgttctgcttccttgcgttctgctttgagtacgctggggtacagcaccacggcctgagctataactgctcccttccgctggcgtttgacgggtcttgctctggcatccagcacttctccgcgatgctccgagatgaggtaggtggtcgcgcggttaacttgcttcctagtgaaaccgttcaggacatctacgggattgttgctaacacgattaacatcgctaagaacgaagaaagtcaacgagattctacaagcagacgcaatcaatgggaccgataaataggctaatatgaatgtatttgatctctattttattaatacgaaaccccttaataattgatattttcgatacatatttggcagtagttagctacgtaacagagtattattttcatttcaagttatgcatgaactctctaatttcacataccatgctaccactacccttggaggttttgttcatatcttttataataaagctaaaaccgaaaaggtgaagggaaaaaaaactattagagcctgtttcttgtatatagtaatatgtaatatttgcttcgtacgcttagtcctcattttactttttttagaatgacctgttcccgacactatgtaagatctagcttttaacatattatggaaacctgaaatgtaaaatctgaatttttgtatatgtgtttatatttgggtagttcttttgaggaaagcatgcatagacttgctgtacgaactttatgtgacttgtagtgacgctgtttcatgagactttagccctttgaacatattatcatatctcagcttgaaatactatagatttacttttgcagccatttcttggtgctccaaggttgtgcgtatctattacttaatttctgtccttgccaagttttgcagcagggcggtcacaa

SEQ ID NO: 7 - DNA, 6063 bp, Artificial Sequence
  Nucleotide sequence of the SNR52 gRNA expression vector pRN1120-AG1
  misc_feature (2)..(21): guide-sequence (genomic target sequence)
catatatttattaatcaaacagttttagagctagaaatagcaagttaaaataaggctagtccgttatcaacttgaaaaagtggcaccgagtcggtgcttttgtttttttgttttttatgtctggggggcccggtacccagcttttgttccctttagtgagggttaattccgagcttggcgtaatcatggtcatagctgtttcctgtgtgaaattgttatccgctcacaattccacacaacataggagccggaagcataaagtgtaaagcctggggtgcctaatgagtgaggtaactcacattaattgcgttgcgctcactgcccgctttccagtcgggaaacctgtcgtgccagctgcattaatgaatcggccaacgcgcggggagaggcggtttgcgtattgggcgctcttccgcttcctcgctcactgactcgctgcgctcggtcgttcggctgcggcgagcggtatcagctcactcaaaggcggtaatacggttatccacagaatcaggggataacgcaggaaagaacatgtgagcaaaaggccagcaaaaggccaggaaccgtaaaaaggccgcgttgctggcgtttttccataggctcggcccccctgacgagcatcacaaaaatcgacgctcaagtcagaggtggcgaaacccgacaggactataaagataccaggcgttcccccctggaagctccctcgtgcgctctcctgttccgaccctgccgcttaccggatacctgtccgcctttctcccttcgggaagcgtggcgctttctcaatgctcacgctgtaggtatctcagttcggtgtaggtcgttcgctccaagctgggctgtgtgcacgaaccccccgttcagcccgaccgctgcgccttatccggtaactatcgtcttgagtccaacccggtaagacacgacttatcgccactggcagcagccactggtaacaggattagcagagcgaggtatgtaggcggtgctacagagttcttgaagtggtggcctaactacggctacactagaaggacagtatttggtatctgcgctctgctgaagccagttaccttcggaaaaagagttggtagctcttgatccggcaaacaaaccaccgctggtagcggtggtttttttgtttgcaagcagcagattacgcgcagaaaaaaaggatctcaagaagatcctttgatcttttctacggggtctgacgctcagtggaacgaaaactcacgttaagggattttggtcatgagattatcaaaaaggatcttcacctagatccttttaaattaaaaatgaagttttaaatcaatctaaagtatatatgagtaaacttggtctgacagttaccaatgcttaatcagtgaggcacctatctcagcgatctgtctatttcgttcatccatagttgcctgactgcccgtcgtgtagataactacgatacgggagggcttaccatctggccccagtgctgcaatgataccgcgagacccacgctcaccggctccagatttatcagcaataaaccagccagccggaagggccgagcgcagaagtggtcctgcaactttatccgcctccatccagtctattaattgttgccgggaagctagagtaagtagttcgccagttaatagtttgcgcaacgttgttgccattgctacaggcatcgtggtgtcacgctcgtcgtttggtatggcttcattcagctccggttcccaacgatcaaggcgagttacatgatcccccatgttgtgaaaaaaagcggttagctccttcggtcctccgatcgttgtcagaagtaagttggccgcagtgttatcactcatggttatggcagcactgcataattctcttactgtcatgccatccgtaagatgcttttctgtgactggtgagtactcaaccaagtcattctgagaatagtgtatgcggcgaccgagttgctcttgcccggcgtcaatacgggataataccgcgccacatagcagaactttaaaagtgctcatcattggaaaacgttcttcggggcgaaaactctcaaggatcttaccgctgttgagatccagttcgatgtaacccactcgtgcacccaactgatcttcagcatcttttactttcaccagcgtttctgggtgagcaaaaacaggaaggcaaaatgccgcaaaaaagggaataagggcgacacggaaatgttgaatactcatactcttcctttttcaatattattgaagcatttatcagggttattgtctcatgagcggatacatatttgaatgtatttagaaaaataaacaaataggggttccgcgcacatttccccgaaaagtgccacctgacgtctaagaaaccattattatcatgacattaacctataaaaataggcgtatcacgaggccctttcgtctcgcgcgtttcggtgatgacggtgaaaacctctgacacatgcagctcccggagacggtcacagcttgtctgtaagcggatgccgggagcagacaagcccgtcagggcgcgtcagcgggtgttggcgggtgtcggggctggcttaactatgcggcatcagagcagattgtactgagagtgcaccatatcgactacgtcgtaaggccgtttctgacagagtaaaattcttgagggaactttcaccattatgggaaatggttcaagaaggtattgacttaaactccatcaaatggtcaggtcattgagtgttttttatttgttgtatttttttttttttagagaaaatcctccaatatcaaattaggaatcgtagtttcatgattttctgttacacctaactttttgtgtggtgccctcctccttgtcaatattaatgttaaagtgcaattctttttccttatcacgttgagccattagtatcaatttgcttacctgtattcctttactatcctcctttttctccttcttgataaatgtatgtagattgcgtatatagtttcgtctaccctatgaacatattccattttgtaatttcgtgtcgtttctattatgaatttcatttataaagtttatgtacacctaggatccgtcgacactggatggcggcgttagtatcgaatcgacagcagtatagcgaccagcattcacatacgattgacgcatgatattactttctgcgcacttaacttcgcatctgggcagatgatgtcgaggcgaaaaaaaatataaatcacgctaacatttgattaaaatagaacaactacaatataaaaaaactatacaaatgacaagttcttgaaaacaagaatctttttattgtcagtactaggggcagggcatgctcatgtagagcgcctgctcgccgtccgaggcggtgccgtcgtacagggcggtgtccaggccgcagagggtgaaccccatccgccggtacgcgtggatcgccggtgcgttgacgttggtgacctccagccagaggtgcccggcgccccgctcgcgggcgaactccgtcgcgagccccatcaacgcgcgcccgaccccgtgcccccggtgctccggggcgacctcgatgtcctcgacggtcagccggcggttccagccggagtacgagacgaccacgaagcccgccaggtcgccgtcgtccccgtacgcgacgaacgtccgggagtccgggtcgccgtcctccccggcgtccgattcgtcgtccgattcgtcgtcggggaacaccttggtcaggggcgggtccaccggcacctcccgcagggtgaagccgtccccggtggcggtgacgcggaagacggtgtcggtggtgaaggacccatccagtgcctcgatggcctcggcgtcccccgggacactggtgcggtaccggtaagccgtgtcgtcaagagtggtcattttacatggttgtttatgttcggatgtgatgtgagaactgtatcctagcaagattttaaaaggaagtatatgaaagaagaacctcagtggcaaatcctaaccttttatatttctctacaggggcgcggcgtggggacaattcaacgcgtctgtgaggggagcgtttccctgctcgcaggtctgcagcgaggagccgtaatttttgcttcgcgccgtgcggccatcaaaatgtatggatgcaaatgattatacatggggatgtatgggctaaatgtacgggcgacagtcacatcatgcccctgagctgcgcacgtcaagactgtcaaggagggtattctgggcctccatgtcgctggccgggtgacccggcggggacgaggccttaagttcgaacgtacgagctccggcattgcgaataccgctttccacaaacattgctcaaaagtatctctttgctatatatctctgtgctatatccctatataacctacccatccacctttcgctccttgaacttgcatctaaactcgacctctacattttttatgtttatctctagtattactctttagacaaaaaaattgtagtaagaactattcatagagtgaatcgaaaacaatacgaaaatgtaaacatttcctatacgtagtatatagagacaaaatagaagaaaccgttcataattttctgaccaatgaagaatcatcaacgctatcactttctgttcacaaagtatgcgcaatccacatcggtatagaatataatcggggatgcctttatcttgaaaaaatgcacccgcagcttcgctagtaatcagtaaacgcgggaagtggagtcaggctttttttatggaagagaaaatagacaccaaagtagccttcttctaaccttaacggacctacagtgcaaaaagttatcaagagactgcattatagagcgcacaaaggagaaaaaaagtaatctaagatgctttgttagaaaaatagcgctctcgggatgcatttttgtagaacaaaaaagaagtatagattctttgttggtaaaatagcgctctcgcgttgcatttctgttctgtaaaaatgcagctcagattctttgtttgaaaaattagcgctctcgcgttgcatttttgttttacaaaaatgaagcacagattcttcgttggtaaaatagcgctttcgcgttgcatttctgttctgtaaaaatgcagctcagattctttgtttgaaaaattagcgctctcgcgttgcatttttgttctacaaaatgaagcacagatgcttcgttaacaaagatatgctattgaagtgcaagatggaaacgcagaaaatgaaccggggatgcgacgtgcaagattacctatgcaatagatgcaatagtttctccaggaaccgaaatacatacattgtcttccgtaaagcgctagactatatattattatacaggttcaaatatactatctgtttcagggaaaactcccaggttcggatgttcaaaattcaatgatgggtaacaagtacgatcgtaaatctgtaaaacagtttgtcggatattaggctgtatctcctcaaagcgtattcgaatatcattgagaagctgcagcgtcacatcggataataatgatggcagccattgtagaagtgccttttgcatttctagtctctttctcggtctagctagttttactacatcgcgaagatagaatcttagatcacactgcctttgctgagctggatcaatagagtaacaaaagagtggtaaggcctcgttaaaggacaaggacctgagcggaagtgtatcgtacagtagacggagtatactaggtatagtctatagtccgtggaattaattctcatgtttgacagcttatcatcgataatccggagctagcatgcggccgctctagaactagtggatcccccgggctgcagtctttgaaaagataatgtatgattatgctttcactcatatttatacagaaacttgatgttttctttcgagtatatacaaggtgattacatgtacgtttgaagtacaactctagattttgtagtgccctcttgggctagcggtaaaggtgcgcattttttcacaccctacaatgttctgttcaaaagattttggtcaaacgctgtagaagtgaaagttggtgcgcatgtttcggcgttcgaaacttctccgcagtgaaagataaatgat

SEQ ID NO: 8 - DNA, 5906 bp, Artificial Sequence
  Nucleotide sequence of the T7 gRNA expression vector pAG701
  misc_feature (1)..(18): T7 promoter
  misc_feature (18)..(38): guide-sequence (genomic target sequence)
  misc_feature (39)..(118): guide RNA structural component
  misc_feature (119)..(186): self-cleaving ribozyme (HDVr)
  misc_feature (187)..(233): T7 terminator
taatacgactcactatagatatatttattaatcaaacagttttagagctagaaatagcaagttaaaataaggctagtccgttatcaacttgaaaaagtggcaccgagtcggtgcttttggccggcatggtcccagcctcctcgctggcgccggctgggcaacatgcttcggcatggcgaatgggacaaaaaatcaaactggctcaccttcgggtgggcctttttgcgtttataggggggcccggtacccagcttttgttccctttagtgagggttaattccgagcttggcgtaatcatggtcatagctgtttcctgtgtgaaattgttatccgctcacaattccacacaacataggagccggaagcataaagtgtaaagcctggggtgcctaatgagtgaggtaactcacattaattgcgttgcgctcactgcccgctttccagtcgggaaacctgtcgtgccagctgcattaatgaatcggccaacgcgcggggagaggcggtttgcgtattgggcgctcttccgcttcctcgctcactgactcgctgcgctcggtcgttcggctgcggcgagcggtatcagctcactcaaaggcggtaatacggttatccacagaatcaggggataacgcaggaaagaacatgtgagcaaaaggccagcaaaaggccaggaaccgtaaaaaggccgcgttgctggcgtttttccataggctcggcccccctgacgagcatcacaaaaatcgacgctcaagtcagaggtggcgaaacccgacaggactataaagataccaggcgttcccccctggaagctccctcgtgcgctctcctgttccgaccctgccgcttaccggatacctgtccgcctttctcccttcgggaagcgtggcgctttctcaatgctcacgctgtaggtatctcagttcggtgtaggtcgttcgctccaagctgggctgtgtgcacgaaccccccgttcagcccgaccgctgcgccttatccggtaactatcgtcttgagtccaacccggtaagacacgacttatcgccactggcagcagccactggtaacaggattagcagagcgaggtatgtaggcggtgctacagagttcttgaagtggtggcctaactacggctacactagaaggacagtatttggtatctgcgctctgctgaagccagttaccttcggaaaaagagttggtagctcttgatccggcaaacaaaccaccgctggtagcggtggtttttttgtttgcaagcagcagattacgcgcagaaaaaaaggatctcaagaagatcctttgatcttttctacggggtctgacgctcagtggaacgaaaactcacgttaagggattttggtcatgagattatcaaaaaggatcttcacctagatccttttaaattaaaaatgaagttttaaatcaatctaaagtatatatgagtaaacttggtctgacagttaccaatgcttaatcagtgaggcacctatctcagcgatctgtctatttcgttcatccatagttgcctgactgcccgtcgtgtagataactacgatacgggagggcttaccatctggccccagtgctgcaatgataccgcgagacccacgctcaccggctccagatttatcagcaataaaccagccagccggaagggccgagcgcagaagtggtcctgcaactttatccgcctccatccagtctattaattgttgccgggaagctagagtaagtagttcgccagttaatagtttgcgcaacgttgttgccattgctacaggcatcgtggtgtcacgctcgtcgtttggtatggcttcattcagctccggttcccaacgatcaaggcgagttacatgatcccccatgttgtgaaaaaaagcggttagctccttcggtcctccgatcgttgtcagaagtaagttggccgcagtgttatcactcatggttatggcagcactgcataattctcttactgtcatgccatccgtaagatgcttttctgtgactggtgagtactcaaccaagtcattctgagaatagtgtatgcggcgaccgagttgctcttgcccggcgtcaatacgggataataccgcgccacatagcagaactttaaaagtgctcatcattggaaaacgttcttcggggcgaaaactctcaaggatcttaccgctgttgagatccagttcgatgtaacccactcgtgcacccaactgatcttcagcatcttttactttcaccagcgtttctgggtgagcaaaaacaggaaggcaaaatgccgcaaaaaagggaataagggcgacacggaaatgttgaatactcatactcttcctttttcaatattattgaagcatttatcagggttattgtctcatgagcggatacatatttgaatgtatttagaaaaataaacaaataggggttccgcgcacatttccccgaaaagtgccacctgacgtctaagaaaccattattatcatgacattaacctataaaaataggcgtatcacgaggccctttcgtctcgcgcgtttcggtgatgacggtgaaaacctctgacacatgcagctcccggagacggtcacagcttgtctgtaagcggatgccgggagcagacaagcccgtcagggcgcgtcagcgggtgttggcgggtgtcggggctggcttaactatgcggcatcagagcagattgtactgagagtgcaccatatcgactacgtcgtaaggccgtttctgacagagtaaaattcttgagggaactttcaccattatgggaaatggttcaagaaggtattgacttaaactccatcaaatggtcaggtcattgagtgttttttatttgttgtatttttttttttttagagaaaatcctccaatatcaaattaggaatcgtagtttcatgattttctgttacacctaactttttgtgtggtgccctcctccttgtcaatattaatgttaaagtgcaattctttttccttatcacgttgagccattagtatcaatttgcttacctgtattcctttactatcctcctttttctccttcttgataaatgtatgtagattgcgtatatagtttcgtctaccctatgaacatattccattttgtaatttcgtgtcgtttctattatgaatttcatttataaagtttatgtacacctaggatccgtcgacactggatggcggcgttagtatcgaatcgacagcagtatagcgaccagcattcacatacgattgacgcatgatattactttctgcgcacttaacttcgcatctgggcagatgatgtcgaggcgaaaaaaaatataaatcacgctaacatttgattaaaatagaacaactacaatataaaaaaactatacaaatgacaagttcttgaaaacaagaatctttttattgtcagtactaggggcagggcatgctcatgtagagcgcctgctcgccgtccgaggcggtgccgtcgtacagggcggtgtccaggccgcagagggtgaaccccatccgccggtacgcgtggatcgccggtgcgttgacgttggtgacctccagccagaggtgcccggcgccccgctcgcgggcgaactccgtcgcgagccccatcaacgcgcgcccgaccccgtgcccccggtgctccggggcgacctcgatgtcctcgacggtcagccggcggttccagccggagtacgagacgaccacgaagcccgccaggtcgccgtcgtccccgtacgcgacgaacgtccgggagtccgggtcgccgtcctccccggcgtccgattcgtcgtccgattcgtcgtcggggaacaccttggtcaggggcgggtccaccggcacctcccgcagggtgaagccgtccccggtggcggtgacgcggaagacggtgtcggtggtgaaggacccatccagtgcctcgatggcctcggcgtcccccgggacactggtgcggtaccggtaagccgtgtcgtcaagagtggtcattttacatggttgtttatgttcggatgtgatgtgagaactgtatcctagcaagattttaaaaggaagtatatgaaagaagaacctcagtggcaaatcctaaccttttatatttctctacaggggcgcggcgtggggacaattcaacgcgtctgtgaggggagcgtttccctgctcgcaggtctgcagcgaggagccgtaatttttgcttcgcgccgtgcggccatcaaaatgtatggatgcaaatgattatacatggggatgtatgggctaaatgtacgggcgacagtcacatcatgcccctgagctgcgcacgtcaagactgtcaaggagggtattctgggcctccatgtcgctggccgggtgacccggcggggacgaggccttaagttcgaacgtacgagctccggcattgcgaataccgctttccacaaacattgctcaaaagtatctctttgctatatatctctgtgctatatccctatataacctacccatccacctttcgctccttgaacttgcatctaaactcgacctctacattttttatgtttatctctagtattactctttagacaaaaaaattgtagtaagaactattcatagagtgaatcgaaaacaatacgaaaatgtaaacatttcctatacgtagtatatagagacaaaatagaagaaaccgttcataattttctgaccaatgaagaatcatcaacgctatcactttctgttcacaaagtatgcgcaatccacatcggtatagaatataatcggggatgcctttatcttgaaaaaatgcacccgcagcttcgctagtaatcagtaaacgcgggaagtggagtcaggctttttttatggaagagaaaatagacaccaaagtagccttcttctaaccttaacggacctacagtgcaaaaagttatcaagagactgcattatagagcgcacaaaggagaaaaaaagtaatctaagatgctttgttagaaaaatagcgctctcgggatgcatttttgtagaacaaaaaagaagtatagattctttgttggtaaaatagcgctctcgcgttgcatttctgttctgtaaaaatgcagctcagattctttgtttgaaaaattagcgctctcgcgttgcatttttgttttacaaaaatgaagcacagattcttcgttggtaaaatagcgctttcgcgttgcatttctgttctgtaaaaatgcagctcagattctttgtttgaaaaattagcgctctcgcgttgcatttttgttctacaaaatgaagcacagatgcttcgttaacaaagatatgctattgaagtgcaagatggaaacgcagaaaatgaaccggggatgcgacgtgcaagattacctatgcaatagatgcaatagtttctccaggaaccgaaatacatacattgtcttccgtaaagcgctagactatatattattatacaggttcaaatatactatctgtttcagggaaaactcccaggttcggatgttcaaaattcaatgatgggtaacaagtacgatcgtaaatctgtaaaacagtttgtcggatattaggctgtatctcctcaaagcgtattcgaatatcattgagaagctgcagcgtcacatcggataataatgatggcagccattgtagaagtgccttttgcatttctagtctctttctcggtctagctagttttactacatcgcgaagatagaatcttagatcacactgcctttgctgagctggatcaatagagtaacaaaagagtggtaaggcctcgttaaaggacaaggacctgagcggaagtgtatcgtacagtagacggagtatactaggtatagtctatagtccgtggaattaattctcatgtttgacagcttatcatcgataatccggagctagcatgcggccgctctagaactagtggatcccccgggctgcag

SEQ ID NO: 9 - DNA, 20 bp, Artificial Sequence
  Nucleotide sequence of the 20-nt guide-sequence that targets the Saccharomyces bayanus TDH3 (SbTDH3) promoter that was used for constitutive expression of GFP in tester strains AG1 and AG2
atatatttattaatcaaaca

SEQ ID NO: 10 - DNA, 20 bp, Artificial Sequence
  Nucleotide sequence of a random 20-nt guide-sequence that was used for normalization
gctagatggacttgccgctg

SEQ ID NO: 11 - DNA, 23 bp, Artificial Sequence
  Nucleotide sequence of a strong T7 promoter that was used for gRNA expression; this sequence replaced the T7 promoter sequence that is indicated in bold in SEQ ID NO: 8
taatacgactcactataggggaa

SEQ ID NO: 12 - DNA, 23 bp, Artificial Sequence
  Nucleotide sequence of a medium strength T7 promoter that was used for gRNA expression; this sequence replaced the T7 promoter sequence that is indicated in bold in SEQ ID NO: 8
taatacgactcactataggggaa

SEQ ID NO: 13 - DNA, 23 bp, Artificial Sequence
  Nucleotide sequence of a weak strength T7 promoter that was used for gRNA expression; this sequence replaced the T7 promoter sequence that is indicated in bold in SEQ ID NO: 8
taatacgactcactaatactgaa

SEQ ID NO: 14 - DNA, 5441 bp, Artificial Sequence
  Nucleotide sequence of CAS9 including a C-terminal SV40 nuclear localization signal codon pair optimized for expression in S. cerevisiae. The sequence includes the Kl11 promoter from K. lactis and GND2 terminator sequence from S. cerevisiae.
ttttctttttttgcggtcacccccatgtggcggggaggcagaggagtaggtagagcaacgaatcctactatttatccaaattagtctaggaactctttttctagattttttagatttgagggcaagcgctgttaacgactcagaaatgtaagcactacggagtagaacgagaaatccgccataggtggaaatcctagcaaaatcttgcttaccctagctagcctcaggtaagctagccttagcctgtcaaatttttttcaaaatttggtaagtttctactagcaaagcaaacacggttcaacaaaccgaaaactccactcattatacgtggaaaccgaaacaaaaaaacaaaaaccaaaatactcgccaatgagaaagttgctgcgtttctactttcgaggaagaggaactgagaggattgactacgaaaggggcaaaaacgagtcgtattctcccattattgtctgctaccacgcggtctagtagaataagcaaccagtcaacgctaagacaggtaatcaaaataccagtctgctggctacgggctagtttttacctcttttagaacccactgtaaaagtccgttgtaaagcccgttctcactgttggcgtttttttttttttggtttagtttcttatttttcatttttttctttcatgaccaaaaacaaacaaatctcgcgatttgtactgcggccactggggcgtggccaaaaaaatgacaaatttagaaaccttagtttctgatttttcctgttatgaggagatatgataaaaaatattactgctttattgttttttttttatctactgaaatagagaaacttacccaaggaggaggcaaaaaaaagagtatatatacagcagctaccattcagattttaatatattcttttctcttcttctacactattattataataattttactatattcatttttagcttaaaacctcatagaatattattcttcagtcactcgcttaaatacttatcaaaaatggacaagaaatactctattggtttggatatcgggaccaactccgtcggttgggctgtcatcaccgacgaatacaaggttccatccaagaaattcaaggtcttgggtaacactgacagacactctatcaagaagaatttgatcggtgctttgttgttcgactccggtgaaaccgctgaagctaccagattgaagcgtaccgctcgtcgtagatacactagacgtaaaaaccgtatttgttacttgcaagaaatcttttctaacgaaatggccaaggttgacgactctttcttccacagattggaagaatctttcttggttgaagaagacaagaagcacgaaagacatccaatcttcggtaacatcgttgacgaagttgcttaccacgaaaaataccctaccatctaccatttgagaaagaagttggtcgattccaccgacaaggctgatttgagattgatctatttggccttggctcacatgatcaagttcagaggtcacttcttgattgaaggtgacttgaacccagacaactctgacgtcgacaaattgttcatccaattggtccaaacctacaaccaattattcgaggaaaacccaattaacgcttctggtgttgatgctaaggccatcttatctgcccgtttgtccaagtctagacgtttggaaaacttgattgctcaattgcctggtgaaaagaaaaacggtttgttcggtaacttgatcgctttgtccttgggtttgaccccaaacttcaagtccaacttcgacttggctgaagatgccaagttgcaattgtccaaggacacctacgacgacgacttagacaacttgttggctcaaatcggtgaccaatacgccgacttgttcttggctgccaaaaacttatctgacgctatcttgttgtctgacatcttgagagttaacactgaaattaccaaggctccattgtctgcttctatgatcaaaagatacgacgaacaccaccaagatctgactttgttgaaggctttggttagacaacaattgccagaaaagtacaaggaaatcttcttcgaccaatccaaaaatggttacgccggttacattgacggtggtgcttctcaggaagaattctacaagttcatcaagccaattttggaaaagatggatggtactgaagaattattggttaagttgaacagagaagacttattgagaaagcaacgtaccttcgataacggttctatcccacaccaaatccacttgggtgaattgcacgccattttgagaagacaggaagatttctatccattcctaaaggacaacagagaaaagatcgaaaagatcttaactttcagaatcccatactacgtcggtccattggccagaggtaattctagattcgcttggatgaccagaaagtctgaagaaaccatcaccccatggaacttcgaagaagtcgtcgacaagggtgcttctgcccaatctttcatcgaaagaatgaccaactttgataagaacttgccaaacgagaaggtcttgccaaagcactctttgttgtacgaatacttcaccgtctacaacgaattaaccaaggttaaatacgttactgaaggtatgagaaagccagctttcctatccggtgaacaaaagaaggctattgttgacttgttgtttaagaccaacagaaaggtcactgttaagcaattgaaggaagactacttcaagaagattgaatgtttcgattccgtcgaaatctccggtgttgaagaccgtttcaatgcttctttgggcacctaccacgatttgttaaagatcatcaaggacaaggactttttagataacgaagaaaacgaagacatcttggaagatatcgttttgaccttgactcttttcgaggacagagaaatgattgaagagagattgaagacctacgctcacttgttcgacgataaagttatgaagcaactaaagagaagaagatacactggttggggtagattgtccagaaagttgattaacggtatcagagacaagcaatccggtaagactattttagactttttgaaatccgatggtttcgctaacagaaactttatgcaattgattcacgacgattctttgactttcaaggaagacattcaaaaagcccaagtctctggtcaaggtgattctttgcacgaacacatcgctaacttggctggttctccagctattaagaagggtatcttacaaaccgtcaaggtcgttgatgaattggtcaaagtcatgggtagacacaagccagaaaatattgtcatcgaaatggctagagaaaaccaaactactcaaaagggtcaaaagaactctagagaacgtatgaagagaattgaagaaggtatcaaggagttgggttctcaaattttgaaagaacacccagtcgaaaacactcaattacaaaacgaaaagctatacttgtactacttgcaaaacggtcgtgacatgtacgtcgaccaagaattggatatcaacagattgtctgactacgatgtcgatcatatcgtcccacaatcgttcttgaaggacgattccattgacaacaaagttttgactagatctgacaagaacagaggtaagtctgataacgttccatctgaagaagttgttaagaagatgaagaactactggagacaattgttgaatgctaagttgatcactcaaagaaagttcgacaacttgaccaaggctgaaagaggtggtttgtccgaattggacaaagccggtttcatcaagagacaattagtcgaaactagacaaatcaccaagcatgttgctcaaatcttggattccagaatgaacactaagtacgatgaaaacgacaaactaattagagaagttaaggtcatcactttgaagtctaagttggtttctgacttcagaaaggacttccaattttacaaggtcagagaaatcaacaactaccatcacgctcacgatgcctacttgaacgctgttgtcggtactgccttaatcaaaaagtacccaaagttggaatctgaattcgtttacggtgactacaaggtttacgatgttagaaagatgatcgccaagtctgaacaagaaattggtaaggccactgctaagtacttcttctactctaacatcatgaactttttcaagactgaaatcactttagctaacggtgaaattagaaagcgtccattgattgaaaccaatggtgaaactggtgaaattgtctgggacaagggtagagatttcgctaccgtcagaaaggttttgtctatgccacaagttaacatcgtcaagaagactgaagttcaaactggtggtttctctaaggaatccattttgccaaagagaaactctgacaagttgattgctagaaagaaggactgggatcctaagaagtacggtggtttcgactctccaactgttgcttactccgttttggtcgttgctaaggttgaaaagggtaagtctaagaagttgaagtctgttaaggaattgttgggtatcaccatcatggaaagatcctccttcgaaaagaacccaatcgactttttggaagctaagggttacaaggaagtcaagaaggatttgatcattaagttaccaaaatactccttgttcgaattggaaaacggtagaaagagaatgttggcctccgctggtgaactacaaaaaggtaacgaattggctttaccatctaagtacgttaacttcttgtacttggcttcccactacgaaaagttgaaaggttccccagaagacaacgaacaaaagcaattgtttgttgaacaacacaagcactacttggatgaaattattgaacaaatctccgaattctccaagagagtcattttggctgatgctaacttagataaggttttatccgcttacaacaagcacagagacaaaccaatcagagaacaagctgaaaacatcattcatttgttcactttaaccaacttgggtgctccagctgctttcaaatacttcgacactaccattgacagaaagagatacacttccaccaaagaagttttagatgctactttgattcaccaatctattaccggtttgtacgaaaccagaattgacttgtctcaattgggtggtgattccagagctgatccaaagaagaagagaaaggtgtaaaggagttaaaggcaaagttttcttttctagagccgttcccacaaataattatacgtatatgcttcttttcgtttactatatatctatatttacaagcctttattcactgatgcaatttgtttccaaatacttttttggagatctcataactagatatcatgatggcgcaacttggcgctatcttaattactctggctgccaggcccgtgtagagggccgcaagaccttctgtacgccatatagtctctaagaacttgaacaagtttctagacctattgccgcctttcggatcgctattgtt

SEQ ID NO: 15 - DNA, 11742 bp, Artificial Sequence
  Nucleotide sequence of vector pCSN061.
tcgcgcgtttcggtgatgacggtgaaaacctctgacacatgcagctcccggagacggtcacagcttgtctgtaagcggatgccgggagcagacaagcccgtcagggcgcgtcagcgggtgttggcgggtgtcggggctggcttaactatgcggcatcagagcagattgtactgagagtgcaccataaacgacattactatatatataatataggaagcatttaatagacagcatcgtaatatatgtgtactttgcagttatgacgccagatggcagtagtggaagatattctttattgaaaaatagcttgtcaccttacgtacaatcttgatccggagcttttctttttttgccgattaagaattaattcggtcgaaaaaagaaaaggagagggccaagagggagggcattggtgactattgagcacgtgagtatacgtgattaagcacacaaaggcagcttggagtatgtctgttattaatttcacaggtagttctggtccattggtgaaagtttgcggcttgcagagcacagaggccgcagaatgtgctctagattccgatgctgacttgctgggtattatatgtgtgcccaatagaaagagaacaattgacccggttattgcaaggaaaatttcaagtcttgtaaaagcatataaaaatagttcaggcactccgaaatacttggttggcgtgtttcgtaatcaacctaaggaggatgttttggctctggtcaatgattacggcattgatatcgtccaactgcatggagatgagtcgtggcaagaataccaagagttcctcggtttgccagttattaaaagactcgtatttccaaaagactgcaacatactactcagtgcagcttcacagaaacctcattcgtttattcccttgtttgattcagaagcaggtgggacaggtgaacttttggattggaactcgatttctgactgggttggaaggcaagagagccccgaaagcttacattttatgttagctggtggactgacgccagaaaatgttggtgatgcgcttagattaaatggcgttattggtgttgatgtaagcggaggtgtggagacaaatggtgtaaaagactctaacaaaatagcaaatttcgtcaaaaatgctaagaaataggttattactgagtagtatttatttaagtattgtttgtgcacttgcctatgcggtgtgaaataccgcacagatgcgtaaggagaaaataccgcatcaggaaattgtaaacgttaatattttgttaaaattcgcgttaaatttttgttaaatcagctcattttttaaccaataggccgaaatcggcaaaatcccttataaatcaaaagaatagaccgagatagggttgagtgttgttccagtttggaacaagagtccactattaaagaacgtggactccaacgtcaaagggcgaaaaaccgtctatcagggcgatggcccactacgtgaaccatcaccctaatcaagttttttggggtcgaggtgccgtaaagcactaaatcggaaccctaaagggagcccccgatttagagcttgacggggaaagccggcgaacgtggcgagaaaggaagggaagaaagcgaaaggagcgggcgctagggcgctggcaagtgtagcggtcacgctgcgcgtaaccaccacacccgccgcgcttaatgcgccgctacagggcgcgtcgcgccattcgccattcaggctgcgcaactgttgggaagggcgatcggtgcgggcctcttcgctattacgccagctggcgaaagggggatgtgctgcaaggcgattaagttgggtaacgccagggttttcccagtcacgacgttgtaaaacgacggccagtgagcgcgcgtaatacgactcactatagggcgaattgggtaccttttctttttttgcggtcacccccatgtggcggggaggcagaggagtaggtagagcaacgaatcctactatttatccaaattagtctaggaactctttttctagattttttagatttgagggcaagcgctgttaacgactcagaaatgtaagcactacggagtagaacgagaaatccgccataggtggaaatcctagcaaaatcttgcttaccctagctagcctcaggtaagctagccttagcctgtcaaatttttttcaaaatttggtaagtttctactagcaaagcaaacacggttcaacaaaccgaaaactccactcattatacgtggaaaccgaaacaaaaaaacaaaaaccaaaatactcgccaatgagaaagttgctgcgtttctactttcgaggaagaggaactgagaggattgactacgaaaggggcaaaaacgagtcgtattctcccattattgtctgctaccacgcggtctagtagaataagcaaccagtcaacgctaagacaggtaatcaaaataccagtctgctggctacgggctagtttttacctcttttagaacccactgtaaaagtccgttgtaaagcccgttctcactgttggcgtttttttttttttggtttagtttcttatttttcatttttttctttcatgaccaaaaacaaacaaatctcgcgatttgtactgcggccactggggcgtggccaaaaaaatgacaaatttagaaaccttagtttctgatttttcctgttatgaggagatatgataaaaaatattactgctttattgttttttttttatctactgaaatagagaaacttacccaaggaggaggcaaaaaaaagagtatatatacagcagctaccattcagattttaatatattcttttctcttcttctacactattattataataattttactatattcatttttagcttaaaacctcatagaatattattcttcagtcactcgcttaaatacttatcaaaaatggacaagaaatactctattggtttggatatcgggaccaactccgtcggttgggctgtcatcaccgacgaatacaaggttccatccaagaaattcaaggtcttgggtaacactgacagacactctatcaagaagaatttgatcggtgctttgttgttcgactccggtgaaaccgctgaagctaccagattgaagcgtaccgctcgtcgtagatacactagacgtaaaaaccgtatttgttacttgcaagaaatcttttctaacgaaatggccaaggttgacgactctttcttccacagattggaagaatctttcttggttgaagaagacaagaagcacgaaagacatccaatcttcggtaacatcgttgacgaagttgcttaccacgaaaaataccctaccatctaccatttgagaaagaagttggtcgattccaccgacaaggctgatttgagattgatctatttggccttggctcacatgatcaagttcagaggtcacttcttgattgaaggtgacttgaacccagacaactctgacgtcgacaaattgttcatccaattggtccaaacctacaaccaattattcgaggaaaacccaattaacgcttctggtgttgatgctaaggccatcttatctgcccgtttgtccaagtctagacgtttggaaaacttgattgctcaattgcctggtgaaaagaaaaacggtttgttcggtaacttgatcgctttgtccttgggtttgaccccaaacttcaagtccaacttcgacttggctgaagatgccaagttgcaattgtccaaggacacctacgacgacgacttagacaacttgttggctcaaatcggtgaccaatacgccgacttgttcttggctgccaaaaacttatctgacgctatcttgttgtctgacatcttgagagttaacactgaaattaccaaggctccattgtctgcttctatgatcaaaagatacgacgaacaccaccaagatctgactttgttgaaggctttggttagacaacaattgccagaaaagtacaaggaaatcttcttcgaccaatccaaaaatggttacgccggttacattgacggtggtgcttctcaggaagaattctacaagttcatcaagccaattttggaaaagatggatggtactgaagaattattggttaagttgaacagagaagacttattgagaaagcaacgtaccttcgataacggttctatcccacaccaaatccacttgggtgaattgcacgccattttgagaagacaggaagatttctatccattcctaaaggacaacagagaaaagatcgaaaagatcttaactttcagaatcccatactacgtcggtccattggccagaggtaattctagattcgcttggatgaccagaaagtctgaagaaaccatcaccccatggaacttcgaagaagtcgtcgacaagggtgcttctgcccaatctttcatcgaaagaatgaccaactttgataagaacttgccaaacgagaaggtcttgccaaagcactctttgttgtacgaatacttcaccgtctacaacgaattaaccaaggttaaatacgttactgaaggtatgagaaagccagctttcctatccggtgaacaaaagaaggctattgttgacttgttgtttaagaccaacagaaaggtcactgttaagcaattgaaggaagactacttcaagaagattgaatgtttcgattccgtcgaaatctccggtgttgaagaccgtttcaatgcttctttgggcacctaccacgatttgttaaagatcatcaaggacaaggactttttagataacgaagaaaacgaagacatcttggaagatatcgttttgaccttgactcttttcgaggacagagaaatgattgaagagagattgaagacctacgctcacttgttcgacgataaagttatgaagcaactaaagagaagaagatacactggttggggtagattgtccagaaagttgattaacggtatcagagacaagcaatccggtaagactattttagactttttgaaatccgatggtttcgctaacagaaactttatgcaattgattcacgacgattctttgactttcaaggaagacattcaaaaagcccaagtctctggtcaaggtgattctttgcacgaacacatcgctaacttggctggttctccagctattaagaagggtatcttacaaaccgtcaaggtcgttgatgaattggtcaaagtcatgggtagacacaagccagaaaatattgtcatcgaaatggctagagaaaaccaaactactcaaaagggtcaaaagaactctagagaacgtatgaagagaattgaagaaggtatcaaggagttgggttctcaaattttgaaagaacacccagtcgaaaacactcaattacaaaacgaaaagctatacttgtactacttgcaaaacggtcgtgacatgtacgtcgaccaagaattggatatcaacagattgtctgactacgatgtcgatcatatcgtcccacaatcgttcttgaaggacgattccattgacaacaaagttttgactagatctgacaagaacagaggtaagtctgataacgttccatctgaagaagttgttaagaagatgaagaactactggagacaattgttgaatgctaagttgatcactcaaagaaagttcgacaacttgaccaaggctgaaagaggtggtttgtccgaattggacaaagccggtttcatcaagagacaattagtcgaaactagacaaatcaccaagcatgttgctcaaatcttggattccagaatgaacactaagtacgatgaaaacgacaaactaattagagaagttaaggtcatcactttgaagtctaagttggtttctgacttcagaaaggacttccaattttacaaggtcagagaaatcaacaactaccatcacgctcacgatgcctacttgaacgctgttgtcggtactgccttaatcaaaaagtacccaaagttggaatctgaattcgtttacggtgactacaaggtttacgatgttagaaagatgatcgccaagtctgaacaagaaattggtaaggccactgctaagtacttcttctactctaacatcatgaactttttcaagactgaaatcactttagctaacggtgaaattagaaagcgtccattgattgaaaccaatggtgaaactggtgaaattgtctgggacaagggtagagatttcgctaccgtcagaaaggttttgtctatgccacaagttaacatcgtcaagaagactgaagttcaaactggtggtttctctaaggaatccattttgccaaagagaaactctgacaagttgattgctagaaagaaggactgggatcctaagaagtacggtggtttcgactctccaactgttgcttactccgttttggtcgttgctaaggttgaaaagggtaagtctaagaagttgaagtctgttaaggaattgttgggtatcaccatcatggaaagatcctccttcgaaaagaacccaatcgactttttggaagctaagggttacaaggaagtcaagaaggatttgatcattaagttaccaaaatactccttgttcgaattggaaaacggtagaaagagaatgttggcctccgctggtgaactacaaaaaggtaacgaattggctttaccatctaagtacgttaacttcttgtacttggcttcccactacgaaaagttgaaaggttccccagaagacaacgaacaaaagcaattgtttgttgaacaacacaagcactacttggatgaaattattgaacaaatctccgaattctccaagagagtcattttggctgatgctaacttagataaggttttatccgcttacaacaagcacagagacaaaccaatcagagaacaagctgaaaacatcattcatttgttcactttaaccaacttgggtgctccagctgctttcaaatacttcgacactaccattgacagaaagagatacacttccaccaaagaagttttagatgctactttgattcaccaatctattaccggtttgtacgaaaccagaattgacttgtctcaattgggtggtgattccagagctgatccaaagaagaagagaaaggtgtaaaggagttaaaggcaaagttttcttttctagagccgttcccacaaataattatacgtatatgcttcttttcgtttactatatatctatatttacaagcctttattcactgatgcaatttgtttccaaatacttttttggagatctcataactagatatcatgatggcgcaacttggcgctatcttaattactctggctgccaggcccgtgtagagggccgcaagaccttctgtacgccatatagtctctaagaacttgaacaagtttctagacctattgccgcctttcggatcgctattgttgcggccgccagctgaagcttcgtacgctgcaggtcgacgaattctaccgttcgtataatgtatgctatacgaagttatagatctgtttagcttgcctcgtccccgccgggtcacccggccagcgacatggaggcccagaataccctccttgacagtcttgacgtgcgcagctcaggggcatgatgtgactgtcgcccgtacatttagcccatacatccccatgtataatcatttgcatccatacattttgatggccgcacggcgcgaagcaaaaattacggctcctcgctgcagacctgcgagcagggaaacgctcccctcacagacgcgttgaattgtccccacgccgcgcccctgtagagaaatataaaaggttaggatttgccactgaggttcttctttcatatacttccttttaaaatcttgctaggatacagttctcacatcacatccgaacataaacaaccatgggtaaggaaaagactcacgtttcgaggccgcgattaaattccaacatggatgctgatttatatgggtataaatgggctcgcgataatgtcgggcaatcaggtgcgacaatctatcgattgtatgggaagcccgatgcgccagagttgtttctgaaacatggcaaaggtagcgttgccaatgatgttacagatgagatggtcagactaaactggctgacggaatttatgcctcttccgaccatcaagcattttatccgtactcctgatgatgcatggttactcaccactgcgatccccggcaaaacagcattccaggtattagaagaatatcctgattcaggtgaaaatattgttgatgcgctggcagtgttcctgcgccggttgcattcgattcctgtttgtaattgtccttttaacagcgatcgcgtatttcgtctcgctcaggcgcaatcacgaatgaataacggtttggttgatgcgagtgattttgatgacgagcgtaatggctggcctgttgaacaagtctggaaagaaatgcataagcttttgccattctcaccggattcagtcgtcactcatggtgatttctcacttgataaccttatttttgacgaggggaaattaataggttgtattgatgttggacgagtcggaatcgcagaccgataccaggatcttgccatcctatggaactgcctcggtgagttttctccttcattacagaaacggctttttcaaaaatatggtattgataatcctgatatgaataaattgcagtttcatttgatgctcgatgagtttttctaatcagtactgacaataaaaagattcttgttttcaagaacttgtcatttgtatagtttttttatattgtagttgttctattttaatcaaatgttagcgtgatttatattttttttcgcctcgacatcatctgcccagatgcgaagttaagtgcgcagaaagtaatatcatgcgtcaatcgtatgtgaatgctggtcgctatactgctgtcgattcgatactaacgccgccatccagtgtcgaaaacgagctcataacttcgtataatgtatgctatacgaacggtagaattcgaatcagatccactagtggcctatgcggccgccaccgcggtggagctccagcttttgttccctttagtgagggttaattgcgcgcttggcgtaatcatggtcatagctgtttcctgtgtgaaattgttatccgctcacaattccacacaacataggagccggaagcataaagtgtaaagcctggggtgcctaatgagtgaggtaactcacattaattgcgttgcgctcactgcccgctttccagtcgggaaacctgtcgtgccagctgcattaatgaatcggccaacgcgcggggagaggcggtttgcgtattgggcgctcttccgcttcctcgctcactgactcgctgcgctcggtcgttcggctgcggcgagcggtatcagctcactcaaaggcggtaatacggttatccacagaatcaggggataacgcaggaaagaacatgtgagcaaaaggccagcaaaaggccaggaaccgtaaaaaggccgcgttgctggcgtttttccataggctccgcccccctgacgagcatcacaaaaatcgacgctcaagtcagaggtggcgaaacccgacaggactataaagataccaggcgtttccccctggaagctccctcgtgcgctctcctgttccgaccctgccgcttaccggatacctgtccgcctttctcccttcgggaagcgtggcgctttctcatagctcacgctgtaggtatctcagttcggtgtaggtcgttcgctccaagctgggctgtgtgcacgaaccccccgttcagcccgaccgctgcgccttatccggtaactatcgtcttgagtccaacccggtaagacacgacttatcgccactggcagcagccactggtaacaggattagcagagcgaggtatgtaggcggtgctacagagttcttgaagtggtggcctaactacggctacactagaaggacagtatttggtatctgcgctctgctgaagccagttaccttcggaaaaagagttggtagctcttgatccggcaaacaaaccaccgctggtagcggtggtttttttgtttgcaagcagcagattacgcgcagaaaaaaaggatctcaagaagatcctttgatcttttctacggggtctgacgctcagtggaacgaaaactcacgttaagggattttggtcatgagattatcaaaaaggatcttcacctagatccttttaaattaaaaatgaagttttaaatcaatctaaagtatatatgagtaaacttggtctgacagttaccaatgcttaatcagtgaggcacctatctcagcgatctgtctatttcgttcatccatagttgcctgactccccgtcgtgtagataactacgatacgggagggcttaccatctggccccagtgctgcaatgataccgcgagacccacgctcaccggctccagatttatcagcaataaaccagccagccggaagggccgagcgcagaagtggtcctgcaactttatccgcctccatccagtctattaattgttgccgggaagctagagtaagtagttcgccagttaatagtttgcgcaacgttgttgccattgctacaggcatcgtggtgtcacgctcgtcgtttggtatggcttcattcagctccggttcccaacgatcaaggcgagttacatgatcccccatgttgtgcaaaaaagcggttagctccttcggtcctccgatcgttgtcagaagtaagttggccgcagtgttatcactcatggttatggcagcactgcataattctcttactgtcatgccatccgtaagatgcttttctgtgactggtgagtactcaaccaagtcattctgagaatagtgtatgcggcgaccgagttgctcttgcccggcgtcaatacgggataataccgcgccacatagcagaactttaaaagtgctcatcattggaaaacgttcttcggggcgaaaactctcaaggatcttaccgctgttgagatccagttcgatgtaacccactcgtgcacccaactgatcttcagcatcttttactttcaccagcgtttctgggtgagcaaaaacaggaaggcaaaatgccgcaaaaaagggaataagggcgacacggaaatgttgaatactcatactcttcctttttcaatattattgaagcatttatcagggttattgtctcatgagcggatacatatttgaatgtatttagaaaaataaacaaataggggttccgcgcacatttccccgaaaagtgccacctgggtccttttcatcacgtgctataaaaataattataatttaaattttttaatataaatatataaattaaaaatagaaagtaaaaaaagaaattaaagaaaaaatagtttttgttttccgaagatgtaaaagactctagggggatcgccaacaaatactaccttttatcttgctcttcctgctctcaggtattaatgccgaattgtttcatcttgtctgtgtagaagaccacacacgaaaatcctgtgattttacattttacttatcgttaatcgaatgtatatctatttaatctgcttttcttgtctaataaatatatatgtaaagtacgctttttgttgaaattttttaaacctttgtttatttttttttcttcattccgtaactcttctaccttctttatttactttctaaaatccaaatacaaaacataaaaataaataaacacagagtaaattcccaaattattccatcattaaaagatacgaggcgcgtgtaagttacaggcaagcgatccgtcctaagaaaccattattatcatgacattaacctataaaaataggcgtatcacgaggccctttcgtc

SEQ ID NO: 16 - DNA, 5712 bp, Artificial Sequence
  Nucleotide sequence of vector pRN1120
tcgcgcgtttcggtgatgacggtgaaaacctctgacacatgcagctcccggagacggtcacagcttgtctgtaagcggatgccgggagcagacaagcccgtcagggcgcgtcagcgggtgttggcgggtgtcggggctggcttaactatgcggcatcagagcagattgtactgagagtgcaccatatcgactacgtcgtaaggccgtttctgacagagtaaaattcttgagggaactttcaccattatgggaaatggttcaagaaggtattgacttaaactccatcaaatggtcaggtcattgagtgttttttatttgttgtatttttttttttttagagaaaatcctccaatatcaaattaggaatcgtagtttcatgattttctgttacacctaactttttgtgtggtgccctcctccttgtcaatattaatgttaaagtgcaattctttttccttatcacgttgagccattagtatcaatttgcttacctgtattcctttactatcctcctttttctccttcttgataaatgtatgtagattgcgtatatagtttcgtctaccctatgaacatattccattttgtaatttcgtgtcgtttctattatgaatttcatttataaagtttatgtacacctaggatccgtcgacactggatggcggcgttagtatcgaatcgacagcagtatagcgaccagcattcacatacgattgacgcatgatattactttctgcgcacttaacttcgcatctgggcagatgatgtcgaggcgaaaaaaaatataaatcacgctaacatttgattaaaatagaacaactacaatataaaaaaactatacaaatgacaagttcttgaaaacaagaatctttttattgtcagtactaggggcagggcatgctcatgtagagcgcctgctcgccgtccgaggcggtgccgtcgtacagggcggtgtccaggccgcagagggtgaaccccatccgccggtacgcgtggatcgccggtgcgttgacgttggtgacctccagccagaggtgcccggcgccccgctcgcgggcgaactccgtcgcgagccccatcaacgcgcgcccgaccccgtgcccccggtgctccggggcgacctcgatgtcctcgacggtcagccggcggttccagccggagtacgagacgaccacgaagcccgccaggtcgccgtcgtccccgtacgcgacgaacgtccgggagtccgggtcgccgtcctccccggcgtccgattcgtcgtccgattcgtcgtcggggaacaccttggtcaggggcgggtccaccggcacctcccgcagggtgaagccgtccccggtggcggtgacgcggaagacggtgtcggtggtgaaggacccatccagtgcctcgatggcctcggcgtcccccgggacactggtgcggtaccggtaagccgtgtcgtcaagagtggtcattttacatggttgtttatgttcggatgtgatgtgagaactgtatcctagcaagattttaaaaggaagtatatgaaagaagaacctcagtggcaaatcctaaccttttatatttctctacaggggcgcggcgtggggacaattcaacgcgtctgtgaggggagcgtttccctgctcgcaggtctgcagcgaggagccgtaatttttgcttcgcgccgtgcggccatcaaaatgtatggatgcaaatgattatacatggggatgtatgggctaaatgtacgggcgacagtcacatcatgcccctgagctgcgcacgtcaagactgtcaaggagggtattctgggcctccatgtcgctggccgggtgacccggcggggacgaggccttaagttcgaacgtacgagctccggcattgcgaataccgctttccacaaacattgctcaaaagtatctctttgctatatatctctgtgctatatccctatataacctacccatccacctttcgctccttgaacttgcatctaaactcgacctctacattttttatgtttatctctagtattactctttagacaaaaaaattgtagtaagaactattcatagagtgaatcgaaaacaatacgaaaatgtaaacatttcctatacgtagtatatagagacaaaatagaagaaaccgttcataattttctgaccaatgaagaatcatcaacgctatcactttctgttcacaaagtatgcgcaatccacatcggtatagaatataatcggggatgcctttatcttgaaaaaatgcacccgcagcttcgctagtaatcagtaaacgcgggaagtggagtcaggctttttttatggaagagaaaatagacaccaaagtagccttcttctaaccttaacggacctacagtgcaaaaagttatcaagagactgcattatagagcgcacaaaggagaaaaaaagtaatctaagatgctttgttagaaaaatagcgctctcgggatgcatttttgtagaacaaaaaagaagtatagattctttgttggtaaaatagcgctctcgcgttgcatttctgttctgtaaaaatgcagctcagattctttgtttgaaaaattagcgctctcgcgttgcatttttgttttacaaaaatgaagcacagattcttcgttggtaaaatagcgctttcgcgttgcatttctgttctgtaaaaatgcagctcagattctttgtttgaaaaattagcgctctcgcgttgcatttttgttctacaaaatgaagcacagatgcttcgttaacaaagatatgctattgaagtgcaagatggaaacgcagaaaatgaaccggggatgcgacgtgcaagattacctatgcaatagatgcaatagtttctccaggaaccgaaatacatacattgtcttccgtaaagcgctagactatatattattatacaggttcaaatatactatctgtttcagggaaaactcccaggttcggatgttcaaaattcaatgatgggtaacaagtacgatcgtaaatctgtaaaacagtttgtcggatattaggctgtatctcctcaaagcgtattcgaatatcattgagaagctgcagcgtcacatcggataataatgatggcagccattgtagaagtgccttttgcatttctagtctctttctcggtctagctagttttactacatcgcgaagatagaatcttagatcacactgcctttgctgagctggatcaatagagtaacaaaagagtggtaaggcctcgttaaaggacaaggacctgagcggaagtgtatcgtacagtagacggagtatactaggtatagtctatagtccgtggaattaattctcatgtttgacagcttatcatcgataatccggagctagcatgcggccgctctagaactagtggatcccccgggctgcaggaattcgatatcaagcttatcgataccgtcgacctcgagggggggcccggtacccagcttttgttccctttagtgagggttaattccgagcttggcgtaatcatggtcatagctgtttcctgtgtgaaattgttatccgctcacaattccacacaacataggagccggaagcataaagtgtaaagcctggggtgcctaatgagtgaggtaactcacattaattgcgttgcgctcactgcccgctttccagtcgggaaacctgtcgtgccagctgcattaatgaatcggccaacgcgcggggagaggcggtttgcgtattgggcgctcttccgcttcctcgctcactgactcgctgcgctcggtcgttcggctgcggcgagcggtatcagctcactcaaaggcggtaatacggttatccacagaatcaggggataacgcaggaaagaacatgtgagcaaaaggccagcaaaaggccaggaaccgtaaaaaggccgcgttgctggcgtttttccataggctcggcccccctgacgagcatcacaaaaatcgacgctcaagtcagaggtggcgaaacccgacaggactataaagataccaggcgttcccccctggaagctccctcgtgcgctctcctgttccgaccctgccgcttaccggatacctgtccgcctttctcccttcgggaagcgtggcgctttctcaatgctcacgctgtaggtatctcagttcggtgtaggtcgttcgctccaagctgggctgtgtgcacgaaccccccgttcagcccgaccgctgcgccttatccggtaactatcgtcttgagtccaacccggtaagacacgacttatcgccactggcagcagccactggtaacaggattagcagagcgaggtatgtaggcggtgctacagagttcttgaagtggtggcctaactacggctacactagaaggacagtatttggtatctgcgctctgctgaagccagttaccttcggaaaaagagttggtagctcttgatccggcaaacaaaccaccgctggtagcggtggtttttttgtttgcaagcagcagattacgcgcagaaaaaaaggatctcaagaagatcctttgatcttttctacggggtctgacgctcagtggaacgaaaactcacgttaagggattttggtcatgagattatcaaaaaggatcttcacctagatccttttaaattaaaaatgaagttttaaatcaatctaaagtatatatgagtaaacttggtctgacagttaccaatgcttaatcagtgaggcacctatctcagcgatctgtctatttcgttcatccatagttgcctgactgcccgtcgtgtagataactacgatacgggagggcttaccatctggccccagtgctgcaatgataccgcgagacccacgctcaccggctccagatttatcagcaataaaccagccagccggaagggccgagcgcagaagtggtcctgcaactttatccgcctccatccagtctattaattgttgccgggaagctagagtaagtagttcgccagttaatagtttgcgcaacgttgttgccattgctacaggcatcgtggtgtcacgctcgtcgtttggtatggcttcattcagctccggttcccaacgatcaaggcgagttacatgatcccccatgttgtgaaaaaaagcggttagctccttcggtcctccgatcgttgtcagaagtaagttggccgcagtgttatcactcatggttatggcagcactgcataattctcttactgtcatgccatccgtaagatgcttttctgtgactggtgagtactcaaccaagtcattctgagaatagtgtatgcggcgaccgagttgctcttgcccggcgtcaatacgggataataccgcgccacatagcagaactttaaaagtgctcatcattggaaaacgttcttcggggcgaaaactctcaaggatcttaccgctgttgagatccagttcgatgtaacccactcgtgcacccaactgatcttcagcatcttttactttcaccagcgtttctgggtgagcaaaaacaggaaggcaaaatgccgcaaaaaagggaataagggcgacacggaaatgttgaatactcatactcttcctttttcaatattattgaagcatttatcagggttattgtctcatgagcggatacatatttgaatgtatttagaaaaataaacaaataggggttccgcgcacatttccccgaaaagtgccacctgacgtctaagaaaccattattatcatgacattaacctataaaaataggcgtatcacgaggccctttcgtc

SEQ ID NO: 17 - DNA, 3705 bp, Artificial Sequence
  Nucleotide sequence of T7-RNA polymerase (T7 RNAP) expression unit. The sequence includes the codon pair optimized T7 RNAP gene under control of TDH3 promoter and EnoI terminator sequence for expression in S. cerevisiae
cgagctcataacttcgtataatgtatgctatacgaacggtagaattcgaatcagatccactagtgtgcttagtcaaaaaattagccttttaattctgctgtaacccgtacatgcccaaaatagggggcgggttacacagaatatataacatcgtaggtgtctgggtgaacagtttattcctggcatccactaaatataatggagcccgctttttaagctggcatccagaaaaaaaaagaatcccagcaccaaaatattgttttcttcaccaaccatcagttcataggtccattctcttagcgcaactacagagaacaggggcacaaacaggcaaaaaacgggcacaacctcaatggagtgatgcaacctgcctggagtaaatgatgacacaaggcaattgacccacgcatgtatctatctcattttcttacaccttctattaccttctgctctctctgatttggaaaaagctgaaaaaaaaggttgaaaccagttccctgaaattattcccctacttgactaataagtatataaagacggtaggtattgattgtaattctgtaaatctatttcttaaacttcttaaattctacttttatagttagtcttttttttagttttaaaacaccaagaacttagtttcgaataaacacacataaacaaacaaaatgaacacaatcaatattgccaaaaatgaccccaagaaaaaacgtaaggtttttagcgatatcgagctagctgcaattcctttcaacacgctagctgatcattatggtgagcgtctggcaagagaacagctggccctagagcacgaaagttatgaaatgggagaagccaggtttagaaaaatgttcgaaagacaactaaaagccggcgaggtggctgacaacgcagccgctaagcccctgatcacgacattactaccaaaaatgattgcccgtataaacgactggtttgaggaggtgaaagctaagcgtggcaagaggcccacagcgttccagttccttcaagaaattaagcctgaagcggtcgcatatattacgattaaaaccactctagcttgtcttacaagcgcggataacacaacagtacaggctgtagctagcgcgataggcagggcaatagaggacgaggccaggttcgggcgtattcgtgatctagaagctaaacattttaaaaaaaacgtggaagaacagttaaacaagagagttgggcatgtgtacaagaaagcgttcatgcaggtcgtggaggctgacatgctttcaaaaggcctgttgggaggagaagcatggagtagctggcacaaggaggactcaatccatgtcggcgtgaggtgtattgagatgttgatagagagtacaggcatggtgtcattacaccgtcaaaacgcaggtgttgtgggccaagattctgagacgatcgaattagcaccagaatacgcggaggccatagcgactcgtgccggggcgttggcaggaatatctccaatgtttcagccatgtgtagtacctccgaagccatggactggaattaccggtgggggctattgggctaatggtagaaggccgttggcactggtcagaacccactcaaaaaaagctttgatgcgttatgaagatgtttacatgcccgaggtctataaggctatcaatatcgctcaaaacactgcgtggaaaattaataagaaagttttggctgttgcgaacgttataacaaagtggaaacactgcccagtcgaggacatccctgcgatcgagcgtgaagaattgcccatgaaacctgaagatattgatatgaaccctgaagctctgacagcgtggaaaagagcagcagccgctgtttacagaaaagataaggcaagaaaaagtaggaggatctcactagagttcatgcttgagcaggccaataagtttgccaaccacaaggccatctggtttccttataacatggactggcgtggtagggtttacgcagtctccatgtttaatcctcaaggcaacgatatgaccaaggggctgcttaccttagcaaaggggaaacccattgggaaggagggatactactggctaaaaatacatggtgcaaattgtgcaggggttgataaagtcccatttccggaaagaataaaattcattgaggagaaccatgagaacataatggcctgtgctaaatcaccacttgagaatacatggtgggcggagcaagacagtcccttttgttttctggcattctgctttgagtatgcaggggtgcagcaccatggattgagctataactgttcactacccttggcatttgatgggagttgtagtgggattcaacatttcagcgctatgttgagggatgaagtcggaggtagggccgtcaatcttctaccgtctgagacggttcaagacatttacgggatagtggctaaaaaagtcaacgagattcttcaggccgacgcgattaatggcactgataacgaggtagtaacagtgactgacgaaaacacgggagaaatatccgagaaagttaaacttgggaccaaggcgctggcaggtcaatggctggcgtacggcgttacgaggtctgttacgaaaaggagtgtcatgacattagcgtatggatctaaggaatttggatttagacagcaggtactggaggacaccatacagccagcgatcgactctggcaaaggtttaatgtttacacaacccaaccaggctgctgggtatatggcaaaattgatctgggaatccgtttcagtaactgtagtagctgcagttgaggctatgaactggctgaaaagcgccgccaaactgttagcggcagaggtaaaggacaagaaaacgggcgaaatattgagaaagagatgcgcggtccattgggtcacgcctgatgggttcccagtctggcaggaatacaagaaaccaattcaaaccagactgaaccttatgtttctggggcagtttcgtttgcagcccaccatcaataccaacaaagattcagaaattgacgcgcacaaacaagagtcagggatagctccaaacttcgtgcattcacaagacgggagtcacctgagaaagacggtggtttgggcccatgagaagtatggtatcgagtctttcgccctgattcacgactcctttggtactataccagcagacgctgcaaaccttttcaaagctgttagagagactatggtcgacacatatgagtcttgcgatgtattagctgacttctatgaccaattcgcggaccagctacatgaatcccagctagacaaaatgccggcattacccgccaaagggaatctgaatctaagagatattctggaaagcgatttcgccttcgcttaaaagcttttgattaagccttctagtccaaaaaacacgtttttttgtcatttatttcattttcttagaatagtttagtttattcattttatagtcacgaatgttttatgattctatatagggttgcaaacaagcatttttcattttatgttaaaacaatttcaggtttaccttttattctgcttgtggtgacgcgtgtatccgcccgctcttttggtcacccatgtatttaattgcataaataattcttaaaagtggagctagtctatttctatttacatacctctcatttctcatttcctcccctcccgcggtggagctccagcttttgttccctttagtgagggttaattgcgcgcttggcgta

SEQ ID NO: 18 - DNA, 3705 bp, Artificial Sequence
  Nucleotide sequence of T7-RNApolymerase (T7 RNAP) expression unit. The sequence includes the codon pair optimized T7 RNAP gene under control of enoI promoter and EnoI terminator sequence for expression in S. cerevisiae
cgagctcataacttcgtataatgtatgctatacgaacggtagaattcgaatcagatccactagtgtgcccgcggaaccgccagatattcattacttgacgcaaaagcgtttgaaataatgacgaaaaagaaggaagaaaaaaaaagaaaaataccgcttctaggcgggttatctactgatccgagcttccactaggatagcacccaaacacctgcatatttggacgacctttacttacaccaccaaaaaccactttcgcctctcccgcccctgataacgtccactaattgagcgattacctgagcggtcctcttttgtttgcagcatgagacttgcatactgcaaatcgtaagtagcaacgtgtcaaggtcaaaactgtatggaaaccttgtcacctcacttaattctagctagcctaccctgcaagtcaagaggtgtccgtgattcctagccacctcaaggtatgcctctccccggaaactgtggccttttctggcacacatgatctccacgatttcaacatataaatagcttttgataatggcaatattaatcaaatttattttacttctttcttgtaacatctctcttgtaatcccttattccttctagctatttttcataaaaaaccaagcaactgcttatcaacacacaaacactaaatcaaaatgaacacaatcaatattgccaaaaatgaccccaagaaaaaacgtaaggtttttagcgatatcgagctagctgcaattcctttcaacacgctagctgatcattatggtgagcgtctggcaagagaacagctggccctagagcacgaaagttatgaaatgggagaagccaggtttagaaaaatgttcgaaagacaactaaaagccggcgaggtggctgacaacgcagccgctaagcccctgatcacgacattactaccaaaaatgattgcccgtataaacgactggtttgaggaggtgaaagctaagcgtggcaagaggcccacagcgttccagttccttcaagaaattaagcctgaagcggtcgcatatattacgattaaaaccactctagcttgtcttacaagcgcggataacacaacagtacaggctgtagctagcgcgataggcagggcaatagaggacgaggccaggttcgggcgtattcgtgatctagaagctaaacattttaaaaaaaacgtggaagaacagttaaacaagagagttgggcatgtgtacaagaaagcgttcatgcaggtcgtggaggctgacatgctttcaaaaggcctgttgggaggagaagcatggagtagctggcacaaggaggactcaatccatgtcggcgtgaggtgtattgagatgttgatagagagtacaggcatggtgtcattacaccgtcaaaacgcaggtgttgtgggccaagattctgagacgatcgaattagcaccagaatacgcggaggccatagcgactcgtgccggggcgttggcaggaatatctccaatgtttcagccatgtgtagtacctccgaagccatggactggaattaccggtgggggctattgggctaatggtagaaggccgttggcactggtcagaacccactcaaaaaaagctttgatgcgttatgaagatgtttacatgcccgaggtctataaggctatcaatatcgctcaaaacactgcgtggaaaattaataagaaagttttggctgttgcgaacgttataacaaagtggaaacactgcccagtcgaggacatccctgcgatcgagcgtgaagaattgcccatgaaacctgaagatattgatatgaaccctgaagctctgacagcgtggaaaagagcagcagccgctgtttacagaaaagataaggcaagaaaaagtaggaggatctcactagagttcatgcttgagcaggccaataagtttgccaaccacaaggccatctggtttccttataacatggactggcgtggtagggtttacgcagtctccatgtttaatcctcaaggcaacgatatgaccaaggggctgcttaccttagcaaaggggaaacccattgggaaggagggatactactggctaaaaatacatggtgcaaattgtgcaggggttgataaagtcccatttccggaaagaataaaattcattgaggagaaccatgagaacataatggcctgtgctaaatcaccacttgagaatacatggtgggcggagcaagacagtcccttttgttttctggcattctgctttgagtatgcaggggtgcagcaccatggattgagctataactgttcactacccttggcatttgatgggagttgtagtgggattcaacatttcagcgctatgttgagggatgaagtcggaggtagggccgtcaatcttctaccgtctgagacggttcaagacatttacgggatagtggctaaaaaagtcaacgagattcttcaggccgacgcgattaatggcactgataacgaggtagtaacagtgactgacgaaaacacgggagaaatatccgagaaagttaaacttgggaccaaggcgctggcaggtcaatggctggcgtacggcgttacgaggtctgttacgaaaaggagtgtcatgacattagcgtatggatctaaggaatttggatttagacagcaggtactggaggacaccatacagccagcgatcgactctggcaaaggtttaatgtttacacaacccaaccaggctgctgggtatatggcaaaattgatctgggaatccgtttcagtaactgtagtagctgcagttgaggctatgaactggctgaaaagcgccgccaaactgttagcggcagaggtaaaggacaagaaaacgggcgaaatattgagaaagagatgcgcggtccattgggtcacgcctgatgggttcccagtctggcaggaatacaagaaaccaattcaaaccagactgaaccttatgtttctggggcagtttcgtttgcagcccaccatcaataccaacaaagattcagaaattgacgcgcacaaacaagagtcagggatagctccaaacttcgtgcattcacaagacgggagtcacctgagaaagacggtggtttgggcccatgagaagtatggtatcgagtctttcgccctgattcacgactcctttggtactataccagcagacgctgcaaaccttttcaaagctgttagagagactatggtcgacacatatgagtcttgcgatgtattagctgacttctatgaccaattcgcggaccagctacatgaatcccagctagacaaaatgccggcattacccgccaaagggaatctgaatctaagagatattctggaaagcgatttcgccttcgcttaaaagcttttgattaagccttctagtccaaaaaacacgtttttttgtcatttatttcattttcttagaatagtttagtttattcattttatagtcacgaatgttttatgattctatatagggttgcaaacaagcatttttcattttatgttaaaacaatttcaggtttaccttttattctgcttgtggtgacgcgtgtatccgcccgctcttttggtcacccatgtatttaattgcataaataattcttaaaagtggagctagtctatttctatttacatacctctcatttctcatttcctcccctcccgcggtggagctccagcttttgttccctttagtgagggttaattgcgcgcttggcgta

SEQ ID NO: 19 - DNA, 2673 bp, Artificial Sequence
  Nucleotide sequence of the codon pair optimized T7 RNAP gene for expression in yeast
atgaacacaatcaatattgccaaaaatgaccccaagaaaaaacgtaaggtttttagcgatatcgagctagctgcaattcctttcaacacgctagctgatcattatggtgagcgtctggcaagagaacagctggccctagagcacgaaagttatgaaatgggagaagccaggtttagaaaaatgttcgaaagacaactaaaagccggcgaggtggctgacaacgcagccgctaagcccctgatcacgacattactaccaaaaatgattgcccgtataaacgactggtttgaggaggtgaaagctaagcgtggcaagaggcccacagcgttccagttccttcaagaaattaagcctgaagcggtcgcatatattacgattaaaaccactctagcttgtcttacaagcgcggataacacaacagtacaggctgtagctagcgcgataggcagggcaatagaggacgaggccaggttcgggcgtattcgtgatctagaagctaaacattttaaaaaaaacgtggaagaacagttaaacaagagagttgggcatgtgtacaagaaagcgttcatgcaggtcgtggaggctgacatgctttcaaaaggcctgttgggaggagaagcatggagtagctggcacaaggaggactcaatccatgtcggcgtgaggtgtattgagatgttgatagagagtacaggcatggtgtcattacaccgtcaaaacgcaggtgttgtgggccaagattctgagacgatcgaattagcaccagaatacgcggaggccatagcgactcgtgccggggcgttggcaggaatatctccaatgtttcagccatgtgtagtacctccgaagccatggactggaattaccggtgggggctattgggctaatggtagaaggccgttggcactggtcagaacccactcaaaaaaagctttgatgcgttatgaagatgtttacatgcccgaggtctataaggctatcaatatcgctcaaaacactgcgtggaaaattaataagaaagttttggctgttgcgaacgttataacaaagtggaaacactgcccagtcgaggacatccctgcgatcgagcgtgaagaattgcccatgaaacctgaagatattgatatgaaccctgaagctctgacagcgtggaaaagagcagcagccgctgtttacagaaaagataaggcaagaaaaagtaggaggatctcactagagttcatgcttgagcaggccaataagtttgccaaccacaaggccatctggtttccttataacatggactggcgtggtagggtttacgcagtctccatgtttaatcctcaaggcaacgatatgaccaaggggctgcttaccttagcaaaggggaaacccattgggaaggagggatactactggctaaaaatacatggtgcaaattgtgcaggggttgataaagtcccatttccggaaagaataaaattcattgaggagaaccatgagaacataatggcctgtgctaaatcaccacttgagaatacatggtgggcggagcaagacagtcccttttgttttctggcattctgctttgagtatgcaggggtgcagcaccatggattgagctataactgttcactacccttggcatttgatgggagttgtagtgggattcaacatttcagcgctatgttgagggatgaagtcggaggtagggccgtcaatcttctaccgtctgagacggttcaagacatttacgggatagtggctaaaaaagtcaacgagattcttcaggccgacgcgattaatggcactgataacgaggtagtaacagtgactgacgaaaacacgggagaaatatccgagaaagttaaacttgggaccaaggcgctggcaggtcaatggctggcgtacggcgttacgaggtctgttacgaaaaggagtgtcatgacattagcgtatggatctaaggaatttggatttagacagcaggtactggaggacaccatacagccagcgatcgactctggcaaaggtttaatgtttacacaacccaaccaggctgctgggtatatggcaaaattgatctgggaatccgtttcagtaactgtagtagctgcagttgaggctatgaactggctgaaaagcgccgccaaactgttagcggcagaggtaaaggacaagaaaacgggcgaaatattgagaaagagatgcgcggtccattgggtcacgcctgatgggttcccagtctggcaggaatacaagaaaccaattcaaaccagactgaaccttatgtttctggggcagtttcgtttgcagcccaccatcaataccaacaaagattcagaaattgacgcgcacaaacaagagtcagggatagctccaaacttcgtgcattcacaagacgggagtcacctgagaaagacggtggtttgggcccatgagaagtatggtatcgagtctttcgccctgattcacgactcctttggtactataccagcagacgctgcaaaccttttcaaagctgttagagagactatggtcgacacatatgagtcttgcgatgtattagctgacttctatgaccaattcgcggaccagctacatgaatcccagctagacaaaatgccggcattacccgccaaagggaatctgaatctaagagatattctggaaagcgatttcgccttcgcttaa

SEQ ID NO: 20 - DNA, 604 bp, Artificial Sequence
  Nucleotide sequence of the S. cerevisiae tdh3 promoter (Ptdh3)
gtgcttagtcaaaaaattagccttttaattctgctgtaacccgtacatgcccaaaatagggggcgggttacacagaatatataacatcgtaggtgtctgggtgaacagtttattcctggcatccactaaatataatggagcccgctttttaagctggcatccagaaaaaaaaagaatcccagcaccaaaatattgttttcttcaccaaccatcagttcataggtccattctcttagcgcaactacagagaacaggggcacaaacaggcaaaaaacgggcacaacctcaatggagtgatgcaacctgcctggagtaaatgatgacacaaggcaattgacccacgcatgtatctatctcattttcttacaccttctattaccttctgctctctctgatttggaaaaagctgaaaaaaaaggttgaaaccagttccctgaaattattcccctacttgactaataagtatataaagacggtaggtattgattgtaattctgtaaatctatttcttaaacttcttaaattctacttttatagttagtcttttttttagttttaaaacaccaagaacttagtttcgaataaacacacataaacaaacaaa

SEQ ID NO: 21 - DNA, 604 bp, Artificial Sequence
  Nucleotide sequence of the S. cerevisiae enoI promoter (PenoI)
gtgcccgcggaaccgccagatattcattacttgacgcaaaagcgtttgaaataatgacgaaaaagaaggaagaaaaaaaaagaaaaataccgcttctaggcgggttatctactgatccgagcttccactaggatagcacccaaacacctgcatatttggacgacctttacttacaccaccaaaaaccactttcgcctctcccgcccctgataacgtccactaattgagcgattacctgagcggtcctcttttgtttgcagcatgagacttgcatactgcaaatcgtaagtagcaacgtgtcaaggtcaaaactgtatggaaaccttgtcacctcacttaattctagctagcctaccctgcaagtcaagaggtgtccgtgattcctagccacctcaaggtatgcctctccccggaaactgtggccttttctggcacacatgatctccacgatttcaacatataaatagcttttgataatggcaatattaatcaaatttattttacttctttcttgtaacatctctcttgtaatcccttattccttctagctatttttcataaaaaaccaagcaactgcttatcaacacacaaacactaaatcaaa

SEQ ID NO: 22 - DNA, 305 bp, Artificial Sequence
  Nucleotide sequence of the S. cerevisiae enoI terminator (TenoI)
aagcttttgattaagccttctagtccaaaaaacacgtttttttgtcatttatttcattttcttagaatagtttagtttattcattttatagtcacgaatgttttatgattctatatagggttgcaaacaagcatttttcattttatgttaaaacaatttcaggtttaccttttattctgcttgtggtgacgcgtgtatccgcccgctcttttggtcacccatgtatttaattgcataaataattcttaaaagtggagctagtctatttctatttacatacctctcatttctcatttcctcccctc

SEQ ID NO: 23 - DNA, 21 bp, Artificial Sequence
  Nucleotide sequence of forward primer to the 5' transition of the pCSN061 backbone to the T7 RNAP expression cassette
ctgtcgattcgatactaacgc

SEQ ID NO: 24 - DNA, 19 bp, Artificial Sequence
  Nucleotide sequence of reverse primer to the 5' transition of the pCSN061 backbone to the T7 RNAP expression cassette
ctgcgttgtcagccacctc

SEQ ID NO: 25 - DNA, 21 bp, Artificial Sequence
  Nucleotide sequence of forward primer to the 3' transition of the pCSN061 backbone to the T7 RNAP expression cassette
cacacaggaaacagctatgac

SEQ ID NO: 26 - DNA, 20 bp, Artificial Sequence
  Nucleotide sequence of reverse primer to the 3' transition of the pCSN061 backbone to the T7 RNAP expression cassette
ccggcattacccgccaaagg

SEQ ID NO: 27 - DNA, 15307 bp, Artificial Sequence
  Nucleotide sequence of vector pCSN070
tcgcgcgtttcggtgatgacggtgaaaacctctgacacatgcagctcccggagacggtcacagcttgtctgtaagcggatgccgggagcagacaagcccgtcagggcgcgtcagcgggtgttggcgggtgtcggggctggcttaactatgcggcatcagagcagattgtactgagagtgcaccataaacgacattactatatatataatataggaagcatttaatagacagcatcgtaatatatgtgtactttgcagttatgacgccagatggcagtagtggaagatattctttattgaaaaatagcttgtcaccttacgtacaatcttgatccggagcttttctttttttgccgattaagaattaattcggtcgaaaaaagaaaaggagagggccaagagggagggcattggtgactattgagcacgtgagtatacgtgattaagcacacaaaggcagcttggagtatgtctgttattaatttcacaggtagttctggtccattggtgaaagtttgcggcttgcagagcacagaggccgcagaatgtgctctagattccgatgctgacttgctgggtattatatgtgtgcccaatagaaagagaacaattgacccggttattgcaaggaaaatttcaagtcttgtaaaagcatataaaaatagttcaggcactccgaaatacttggttggcgtgtttcgtaatcaacctaaggaggatgttttggctctggtcaatgattacggcattgatatcgtccaactgcatggagatgagtcgtggcaagaataccaagagttcctcggtttgccagttattaaaagactcgtatttccaaaagactgcaacatactactcagtgcagcttcacagaaacctcattcgtttattcccttgtttgattcagaagcaggtgggacaggtgaacttttggattggaactcgatttctgactgggttggaaggcaagagagccccgaaagcttacattttatgttagctggtggactgacgccagaaaatgttggtgatgcgcttagattaaatggcgttattggtgttgatgtaagcggaggtgtggagacaaatggtgtaaaagactctaacaaaatagcaaatttcgtcaaaaatgctaagaaataggttattactgagtagtatttatttaagtattgtttgtgcacttgcctatgcggtgtgaaataccgcacagatgcgtaaggagaaaataccgcatcaggaaattgtaaacgttaatattttgttaaaattcgcgttaaatttttgttaaatcagctcattttttaaccaataggccgaaatcggcaaaatcccttataaatcaaaagaatagaccgagatagggttgagtgttgttccagtttggaacaagagtccactattaaagaacgtggactccaacgtcaaagggcgaaaaaccgtctatcagggcgatggcccactacgtgaaccatcaccctaatcaagttttttggggtcgaggtgccgtaaagcactaaatcggaaccctaaagggagcccccgatttagagcttgacggggaaagccggcgaacgtggcgagaaaggaagggaagaaagcgaaaggagcgggcgctagggcgctggcaagtgtagcggtcacgctgcgcgtaaccaccacacccgccgcgcttaatgcgccgctacagggcgcgtcgcgccattcgccattcaggctgcgcaactgttgggaagggcgatcggtgcgggcctcttcgctattacgccagctggcgaaagggggatgtgctgcaaggcgattaagttgggtaacgccagggttttcccagtcacgacgttgtaaaacgacggccagtgagcgcgcgtaatacgactcactatagggcgaattgggtaccttttctttttttgcggtcacccccatgtggcggggaggcagaggagtaggtagagcaacgaatcctactatttatccaaattagtctaggaactctttttctagattttttagatttgagggcaagcgctgttaacgactcagaaatgtaagcactacggagtagaacgagaaatccgccataggtggaaatcctagcaaaatcttgcttaccctagctagcctcaggtaagctagccttagcctgtcaaatttttttcaaaatttggtaagtttctactagcaaagcaaacacggttcaacaaaccgaaaactccactcattatacgtggaaaccgaaacaaaaaaacaaaaaccaaaatactcgccaatgagaaagttgctgcgtttctactttcgaggaagaggaactgagaggattgactacgaaaggggcaaaaacgagtcgtattctcccattattgtctgctaccacgcggtctagtagaataagcaaccagtcaacgctaagacaggtaatcaaaataccagtctgctggctacgggctagtttttacctcttttagaacccactgtaaaagtccgttgtaaagcccgttctcactgttggcgtttttttttttttggtttagtttcttatttttcatttttttctttcatgaccaaaaacaaacaaatctcgcgatttgtactgcggccactggggcgtggccaaaaaaatgacaaatttagaaaccttagtttctgatttttcctgttatgaggagatatgataaaaaatattactgctttattgttttttttttatctactgaaatagagaaacttacccaaggaggaggcaaaaaaaagagtatatatacagcagctaccattcagattttaatatattcttttctcttcttctacactattattataataattttactatattcatttttagcttaaaacctcatagaatattattcttcagtcactcgcttaaatacttatcaaaaatggacaagaaatactctattggtttggatatcgggaccaactccgtcggttgggctgtcatcaccgacgaatacaaggttccatccaagaaattcaaggtcttgggtaacactgacagacactctatcaagaagaatttgatcggtgctttgttgttcgactccggtgaaaccgctgaagctaccagattgaagcgtaccgctcgtcgtagatacactagacgtaaaaaccgtatttgttacttgcaagaaatcttttctaacgaaatggccaaggttgacgactctttcttccacagattggaagaatctttcttggttgaagaagacaagaagcacgaaagacatccaatcttcggtaacatcgttgacgaagttgcttaccacgaaaaataccctaccatctaccatttgagaaagaagttggtcgattccaccgacaaggctgatttgagattgatctatttggccttggctcacatgatcaagttcagaggtcacttcttgattgaaggtgacttgaacccagacaactctgacgtcgacaaattgttcatccaattggtccaaacctacaaccaattattcgaggaaaacccaattaacgcttctggtgttgatgctaaggccatcttatctgcccgtttgtccaagtctagacgtttggaaaacttgattgctcaattgcctggtgaaaagaaaaacggtttgttcggtaacttgatcgctttgtccttgggtttgaccccaaacttcaagtccaacttcgacttggctgaagatgccaagttgcaattgtccaaggacacctacgacgacgacttagacaacttgttggctcaaatcggtgaccaatacgccgacttgttcttggctgccaaaaacttatctgacgctatcttgttgtctgacatcttgagagttaacactgaaattaccaaggctccattgtctgcttctatgatcaaaagatacgacgaacaccaccaagatctgactttgttgaaggctttggttagacaacaattgccagaaaagtacaaggaaatcttcttcgaccaatccaaaaatggttacgccggttacattgacggtggtgcttctcaggaagaattctacaagttcatcaagccaattttggaaaagatggatggtactgaagaattattggttaagttgaacagagaagacttattgagaaagcaacgtaccttcgataacggttctatcccacaccaaatccacttgggtgaattgcacgccattttgagaagacaggaagatttctatccattcctaaaggacaacagagaaaagatcgaaaagatcttaactttcagaatcccatactacgtcggtccattggccagaggtaattctagattcgcttggatgaccagaaagtctgaagaaaccatcaccccatggaacttcgaagaagtcgtcgacaagggtgcttctgcccaatctttcatcgaaagaatgaccaactttgataagaacttgccaaacgagaaggtcttgccaaagcactctttgttgtacgaatacttcaccgtctacaacgaattaaccaaggttaaatacgttactgaaggtatgagaaagccagctttcctatccggtgaacaaaagaaggctattgttgacttgttgtttaagaccaacagaaaggtcactgttaagcaattgaaggaagactacttcaagaagattgaatgtttcgattccgtcgaaatctccggtgttgaagaccgtttcaatgcttctttgggcacctaccacgatttgttaaagatcatcaaggacaaggactttttagataacgaagaaaacgaagacatcttggaagatatcgttttgaccttgactcttttcgaggacagagaaatgattgaagagagattgaagacctacgctcacttgttcgacgataaagttatgaagcaactaaagagaagaagatacactggttggggtagattgtccagaaagttgattaacggtatcagagacaagcaatccggtaagactattttagactttttgaaatccgatggtttcgctaacagaaactttatgcaattgattcacgacgattctttgactttcaaggaagacattcaaaaagcccaagtctctggtcaaggtgattctttgcacgaacacatcgctaacttggctggttctccagctattaagaagggtatcttacaaaccgtcaaggtcgttgatgaattggtcaaagtcatgggtagacacaagccagaaaatattgtcatcgaaatggctagagaaaaccaaactactcaaaagggtcaaaagaactctagagaacgtatgaagagaattgaagaaggtatcaaggagttgggttctcaaattttgaaagaacacccagtcgaaaacactcaattacaaaacgaaaagctatacttgtactacttgcaaaacggtcgtgacatgtacgtcgaccaagaattggatatcaacagattgtctgactacgatgtcgatcatatcgtcccacaatcgttcttgaaggacgattccattgacaacaaagttttgactagatctgacaagaacagaggtaagtctgataacgttccatctgaagaagttgttaagaagatgaagaactactggagacaattgttgaatgctaagttgatcactcaaagaaagttcgacaacttgaccaaggctgaaagaggtggtttgtccgaattggacaaagccggtttcatcaagagacaattagtcgaaactagacaaatcaccaagcatgttgctcaaatcttggattccagaatgaacactaagtacgatgaaaacgacaaactaattagagaagttaaggtcatcactttgaagtctaagttggtttctgacttcagaaaggacttccaattttacaaggtcagagaaatcaacaactaccatcacgctcacgatgcctacttgaacgctgttgtcggtactgccttaatcaaaaagtacccaaagttggaatctgaattcgtttacggtgactacaaggtttacgatgttagaaagatgatcgccaagtctgaacaagaaattggtaaggccactgctaagtacttcttctactctaacatcatgaactttttcaagactgaaatcactttagctaacggtgaaattagaaagcgtccattgattgaaaccaatggtgaaactggtgaaattgtctgggacaagggtagagatttcgctaccgtcagaaaggttttgtctatgccacaagttaacatcgtcaagaagactgaagttcaaactggtggtttctctaaggaatccattttgccaaagagaaactctgacaagttgattgctagaaagaaggactgggatcctaagaagtacggtggtttcgactctccaactgttgcttactccgttttggtcgttgctaaggttgaaaagggtaagtctaagaagttgaagtctgttaaggaattgttgggtatcaccatcatggaaagatcctccttcgaaaagaacccaatcgactttttggaagctaagggttacaaggaagtcaagaaggatttgatcattaagttaccaaaatactccttgttcgaattggaaaacggtagaaagagaatgttggcctccgctggtgaactacaaaaaggtaacgaattggctttaccatctaagtacgttaacttcttgtacttggcttcccactacgaaaagttgaaaggttccccagaagacaacgaacaaaagcaattgtttgttgaacaacacaagcactacttggatgaaattattgaacaaatctccgaattctccaagagagtcattttggctgatgctaacttagataaggttttatccgcttacaacaagcacagagacaaaccaatcagagaacaagctgaaaacatcattcatttgttcactttaaccaacttgggtgctccagctgctttcaaatacttcgacactaccattgacagaaagagatacacttccaccaaagaagttttagatgctactttgattcaccaatctattaccggtttgtacgaaaccagaattgacttgtctcaattgggtggtgattccagagctgatccaaagaagaagagaaaggtgtaaaggagttaaaggcaaagttttcttttctagagccgttcccacaaataattatacgtatatgcttcttttcgtttactatatatctatatttacaagcctttattcactgatgcaatttgtttccaaatacttttttggagatctcataactagatatcatgatggcgcaacttggcgctatcttaattactctggctgccaggcccgtgtagagggccgcaagaccttctgtacgccatatagtctctaagaacttgaacaagtttctagacctattgccgcctttcggatcgctattgttgcggccgccagctgaagcttcgtacgctgcaggtcgacgaattctaccgttcgtataatgtatgctatacgaagttatagatctgtttagcttgcctcgtccccgccgggtcacccggccagcgacatggaggcccagaataccctccttgacagtcttgacgtgcgcagctcaggggcatgatgtgactgtcgcccgtacatttagcccatacatccccatgtataatcatttgcatccatacattttgatggccgcacggcgcgaagcaaaaattacggctcctcgctgcagacctgcgagcagggaaacgctcccctcacagacgcgttgaattgtccccacgccgcgcccctgtagagaaatataaaaggttaggatttgccactgaggttcttctttcatatacttccttttaaaatcttgctaggatacagttctcacatcacatccgaacataaacaaccatgggtaaggaaaagactcacgtttcgaggccgcgattaaattccaacatggatgctgatttatatgggtataaatgggctcgcgataatgtcgggcaatcaggtgcgacaatctatcgattgtatgggaagcccgatgcgccagagttgtttctgaaacatggcaaaggtagcgttgccaatgatgttacagatgagatggtcagactaaactggctgacggaatttatgcctcttccgaccatcaagcattttatccgtactcctgatgatgcatggttactcaccactgcgatccccggcaaaacagcattccaggtattagaagaatatcctgattcaggtgaaaatattgttgatgcgctggcagtgttcctgcgccggttgcattcgattcctgtttgtaattgtccttttaacagcgatcgcgtatttcgtctcgctcaggcgcaatcacgaatgaataacggtttggttgatgcgagtgattttgatgacgagcgtaatggctggcctgttgaacaagtctggaaagaaatgcataagcttttgccattctcaccggattcagtcgtcactcatggtgatttctcacttgataaccttatttttgacgaggggaaattaataggttgtattgatgttggacgagtcggaatcgcagaccgataccaggatcttgccatcctatggaactgcctcggtgagttttctccttcattacagaaacggctttttcaaaaatatggtattgataatcctgatatgaataaattgcagtttcatttgatgctcgatgagtttttctaatcagtactgacaataaaaagattcttgttttcaagaacttgtcatttgtatagtttttttatattgtagttgttctattttaatcaaatgttagcgtgatttatattttttttcgcctcgacatcatctgcccagatgcgaagttaagtgcgcagaaagtaatatcatgcgtcaatcgtatgtgaatgctggtcgctatactgctgtcgattcgatactaacgccgccatccagtgtcgaaaacgagctcataacttcgtataatgtatgctatacgaacggtagaattcgaatcagatccactagtgtgcttagtcaaaaaattagccttttaattctgctgtaacccgtacatgcccaaaatagggggcgggttacacagaatatataacatcgtaggtgtctgggtgaacagtttattcctggcatccactaaatataatggagcccgctttttaagctggcatccagaaaaaaaaagaatcccagcaccaaaatattgttttcttcaccaaccatcagttcataggtccattctcttagcgcaactacagagaacaggggcacaaacaggcaaaaaacgggcacaacctcaatggagtgatgcaacctgcctggagtaaatgatgacacaaggcaattgacccacgcatgtatctatctcattttcttacaccttctattaccttctgctctctctgatttggaaaaagctgaaaaaaaaggttgaaaccagttccctgaaattattcccctacttgactaataagtatataaagacggtaggtattgattgtaattctgtaaatctatttcttaaacttcttaaattctacttttatagttagtcttttttttagttttaaaacaccaagaacttagtttcgaataaacacacataaacaaacaaaatgaacacaatcaatattgccaaaaatgaccccaagaaaaaacgtaaggtttttagcgatatcgagctagctgcaattcctttcaacacgctagctgatcattatggtgagcgtctggcaagagaacagctggccctagagcacgaaagttatgaaatgggagaagccaggtttagaaaaatgttcgaaagacaactaaaagccggcgaggtggctgacaacgcagccgctaagcccctgatcacgacattactaccaaaaatgattgcccgtataaacgactggtttgaggaggtgaaagctaagcgtggcaagaggcccacagcgttccagttccttcaagaaattaagcctgaagcggtcgcatatattacgattaaaaccactctagcttgtcttacaagcgcggataacacaacagtacaggctgtagctagcgcgataggcagggcaatagaggacgaggccaggttcgggcgtattcgtgatctagaagctaaacattttaaaaaaaacgtggaagaacagttaaacaagagagttgggcatgtgtacaagaaagcgttcatgcaggtcgtggaggctgacatgctttcaaaaggcctgttgggaggagaagcatggagtagctggcacaaggaggactcaatccatgtcggcgtgaggtgtattgagatgttgatagagagtacaggcatggtgtcattacaccgtcaaaacgcaggtgttgtgggccaagattctgagacgatcgaattagcaccagaatacgcggaggccatagcgactcgtgccggggcgttggcaggaatatctccaatgtttcagccatgtgtagtacctccgaagccatggactggaattaccggtgggggctattgggctaatggtagaaggccgttggcactggtcagaacccactcaaaaaaagctttgatgcgttatgaagatgtttacatgcccgaggtctataaggctatcaatatcgctcaaaacactgcgtggaaaattaataagaaagttttggctgttgcgaacgttataacaaagtggaaacactgcccagtcgaggacatccctgcgatcgagcgtgaagaattgcccatgaaacctgaagatattgatatgaaccctgaagctctgacagcgtggaaaagagcagcagccgctgtttacagaaaagataaggcaagaaaaagtaggaggatctcactagagttcatgcttgagcaggccaataagtttgccaaccacaaggccatctggtttccttataacatggactggcgtggtagggtttacgcagtctccatgtttaatcctcaaggcaacgatatgaccaaggggctgcttaccttagcaaaggggaaacccattgggaaggagggatactactggctaaaaatacatggtgcaaattgtgcaggggttgataaagtcccatttccggaaagaataaaattcattgaggagaaccatgagaacataatggcctgtgctaaatcaccacttgagaatacatggtgggcggagcaagacagtcccttttgttttctggcattctgctttgagtatgcaggggtgcagcaccatggattgagctataactgttcactacccttggcatttgatgggagttgtagtgggattcaacatttcagcgctatgttgagggatgaagtcggaggtagggccgtcaatcttctaccgtctgagacggttcaagacatttacgggatagtggctaaaaaagtcaacgagattcttcaggccgacgcgattaatggcactgataacgaggtagtaacagtgactgacgaaaacacgggagaaatatccgagaaagttaaacttgggaccaaggcgctggcaggtcaatggctggcgtacggcgttacgaggtctgttacgaaaaggagtgtcatgacattagcgtatggatctaaggaatttggatttagacagcaggtactggaggacaccatacagccagcgatcgactctggcaaaggtttaatgtttacacaacccaaccaggctgctgggtatatggcaaaattgatctgggaatccgtttcagtaactgtagtagctgcagttgaggctatgaactggctgaaaagcgccgccaaactgttagcggcagaggtaaaggacaagaaaacgggcgaaatattgagaaagagatgcgcggtccattgggtcacgcctgatgggttcccagtctggcaggaatacaagaaaccaattcaaaccagactgaaccttatgtttctggggcagtttcgtttgcagcccaccatcaataccaacaaagattcagaaattgacgcgcacaaacaagagtcagggatagctccaaacttcgtgcattcacaagacgggagtcacctgagaaagacggtggtttgggcccatgagaagtatggtatcgagtctttcgccctgattcacgactcctttggtactataccagcagacgctgcaaaccttttcaaagctgttagagagactatggtcgacacatatgagtcttgcgatgtattagctgacttctatgaccaattcgcggaccagctacatgaatcccagctagacaaaatgccggcattacccgccaaagggaatctgaatctaagagatattctggaaagcgatttcgccttcgcttaaaagcttttgattaagccttctagtccaaaaaacacgtttttttgtcatttatttcattttcttagaatagtttagtttattcattttatagtcacgaatgttttatgattctatatagggttgcaaacaagcatttttcattttatgttaaaacaatttcaggtttaccttttattctgcttgtggtgacgcgtgtatccgcccgctcttttggtcacccatgtatttaattgcataaataattcttaaaagtggagctagtctatttctatttacatacctctcatttctcatttcctcccctcccgcggtggagctccagcttttgttccctttagtgagggttaattgcgcgcttggcgtaatcatggtcatagctgtttcctgtgtgaaattgttatccgctcacaattccacacaacataggagccggaagcataaagtgtaaagcctggggtgcctaatgagtgaggtaactcacattaattgcgttgcgctcactgcccgctttccagtcgggaaacctgtcgtgccagctgcattaatgaatcggccaacgcgcggggagaggcggtttgcgtattgggcgctcttccgcttcctcgctcactgactcgctgcgctcggtcgttcggctgcggcgagcggtatcagctcactcaaaggcggtaatacggttatccacagaatcaggggataacgcaggaaagaacatgtgagcaaaaggccagcaaaaggccaggaaccgtaaaaaggccgcgttgctggcgtttttccataggctccgcccccctgacgagcatcacaaaaatcgacgctcaagtcagaggtggcgaaacccgacaggactataaagataccaggcgtttccccctggaagctccctcgtgcgctctcctgttccgaccctgccgcttaccggatacctgtccgcctttctcccttcgggaagcgtggcgctttctcatagctcacgctgtaggtatctcagttcggtgtaggtcgttcgctccaagctgggctgtgtgcacgaaccccccgttcagcccgaccgctgcgccttatccggtaactatcgtcttgagtccaacccggtaagacacgacttatcgccactggcagcagccactggtaacaggattagcagagcgaggtatgtaggcggtgctacagagttcttgaagtggtggcctaactacggctacactagaaggacagtatttggtatctgcgctctgctgaagccagttaccttcggaaaaagagttggtagctcttgatccggcaaacaaaccaccgctggtagcggtggtttttttgtttgcaagcagcagattacgcgcagaaaaaaaggatctcaagaagatcctttgatcttttctacggggtctgacgctcagtggaacgaaaactcacgttaagggattttggtcatgagattatcaaaaaggatcttcacctagatccttttaaattaaaaatgaagttttaaatcaatctaaagtatatatgagtaaacttggtctgacagttaccaatgcttaatcagtgaggcacctatctcagcgatctgtctatttcgttcatccatagttgcctgactccccgtcgtgtagataactacgatacgggagggcttaccatctggccccagtgctgcaatgataccgcgagacccacgctcaccggctccagatttatcagcaataaaccagccagccggaagggccgagcgcagaagtggtcctgcaactttatccgcctccatccagtctattaattgttgccgggaagctagagtaagtagttcgccagttaatagtttgcgcaacgttgttgccattgctacaggcatcgtggtgtcacgctcgtcgtttggtatggcttcattcagctccggttcccaacgatcaaggcgagttacatgatcccccatgttgtgcaaaaaagcggttagctccttcggtcctccgatcgttgtcagaagtaagttggccgcagtgttatcactcatggttatggcagcactgcataattctcttactgtcatgccatccgtaagatgcttttctgtgactggtgagtactcaaccaagtcattctgagaatagtgtatgcggcgaccgagttgctcttgcccggcgtcaatacgggataataccgcgccacatagcagaactttaaaagtgctcatcattggaaaacgttcttcggggcgaaaactctcaaggatcttaccgctgttgagatccagttcgatgtaacccactcgtgcacccaactgatcttcagcatcttttactttcaccagcgtttctgggtgagcaaaaacaggaaggcaaaatgccgcaaaaaagggaataagggcgacacggaaatgttgaatactcatactcttcctttttcaatattattgaagcatttatcagggttattgtctcatgagcggatacatatttgaatgtatttagaaaaataaacaaataggggttccgcgcacatttccccgaaaagtgccacctgggtccttttcatcacgtgctataaaaataattataatttaaattttttaatataaatatataaattaaaaatagaaagtaaaaaaagaaattaaagaaaaaatagtttttgttttccgaagatgtaaaagactctagggggatcgccaacaaatactaccttttatcttgctcttcctgctctcaggtattaatgccgaattgtttcatcttgtctgtgtagaagaccacacacgaaaatcctgtgattttacattttacttatcgttaatcgaatgtatatctatttaatctgcttttcttgtctaataaatatatatgtaaagtacgctttttgttgaaattttttaaacctttgtttatttttttttcttcattccgtaactcttctaccttctttatttactttctaaaatccaaatacaaaacataaaaataaataaacacagagtaaattcccaaattattccatcattaaaagatacgaggcgcgtgtaagttacaggcaagcgatccgtcctaagaaaccattattatcatgacattaacctataaaaataggcgtatcacgaggccctttcgtc

SEQ ID NO: 28 - DNA, 15307 bp, Artificial Sequence
  Nucleotide sequence of vector pCSN071
tgccgaattgtttcatcttgtctgtgtagaagaccacacacgaaaatcctgtgattttacattttacttatcgttaatcgaatgtatatctatttaatctgcttttcttgtctaataaatatatatgtaaagtacgctttttgttgaaattttttaaacctttgtttatttttttttcttcattccgtaactcttctaccttctttatttactttctaaaatccaaatacaaaacataaaaataaataaacacagagtaaattcccaaattattccatcattaaaagatacgaggcgcgtgtaagttacaggcaagcgatccgtcctaagaaaccattattatcatgacattaacctataaaaataggcgtatcacgaggccctttcgtctcgcgcgtttcggtgatgacggtgaaaacctctgacacatgcagctcccggagacggtcacagcttgtctgtaagcggatgccgggagcagacaagcccgtcagggcgcgtcagcgggtgttggcgggtgtcggggctggcttaactatgcggcatcagagcagattgtactgagagtgcaccataaacgacattactatatatataatataggaagcatttaatagacagcatcgtaatatatgtgtactttgcagttatgacgccagatggcagtagtggaagatattctttattgaaaaatagcttgtcaccttacgtacaatcttgatccggagcttttctttttttgccgattaagaattaattcggtcgaaaaaagaaaaggagagggccaagagggagggcattggtgactattgagcacgtgagtatacgtgattaagcacacaaaggcagcttggagtatgtctgttattaatttcacaggtagttctggtccattggtgaaagtttgcggcttgcagagcacagaggccgcagaatgtgctctagattccgatgctgacttgctgggtattatatgtgtgcccaatagaaagagaacaattgacccggttattgcaaggaaaatttcaagtcttgtaaaagcatataaaaatagttcaggcactccgaaatacttggttggcgtgtttcgtaatcaacctaaggaggatgttttggctctggtcaatgattacggcattgatatcgtccaactgcatggagatgagtcgtggcaagaataccaagagttcctcggtttgccagttattaaaagactcgtatttccaaaagactgcaacatactactcagtgcagcttcacagaaacctcattcgtttattcccttgtttgattcagaagcaggtgggacaggtgaacttttggattggaactcgatttctgactgggttggaaggcaagagagccccgaaagcttacattttatgttagctggtggactgacgccagaaaatgttggtgatgcgcttagattaaatggcgttattggtgttgatgtaagcggaggtgtggagacaaatggtgtaaaagactctaacaaaatagcaaatttcgtcaaaaatgctaagaaataggttattactgagtagtatttatttaagtattgtttgtgcacttgcctatgcggtgtgaaataccgcacagatgcgtaaggagaaaataccgcatcaggaaattgtaaacgttaatattttgttaaaattcgcgttaaatttttgttaaatcagctcattttttaaccaataggccgaaatcggcaaaatcccttataaatcaaaagaatagaccgagatagggttgagtgttgttccagtttggaacaagagtccactattaaagaacgtggactccaacgtcaaagggcgaaaaaccgtctatcagggcgatggcccactacgtgaaccatcaccctaatcaagttttttggggtcgaggtgccgtaaagcactaaatcggaaccctaaagggagcccccgatttagagcttgacggggaaagccggcgaacgtggcgagaaaggaagggaagaaagcgaaaggagcgggcgctagggcgctggcaagtgtagcggtcacgctgcgcgtaaccaccacacccgccgcgcttaatgcgccgctacagggcgcgtcgcgccattcgccattcaggctgcgcaactgttgggaagggcgatcggtgcgggcctcttcgctattacgccagctggcgaaagggggatgtgctgcaaggcgattaagttgggtaacgccagggttttcccagtcacgacgttgtaaaacgacggccagtgagcgcgcgtaatacgactcactatagggcgaattgggtaccttttctttttttgcggtcacccccatgtggcggggaggcagaggagtaggtagagcaacgaatcctactatttatccaaattagtctaggaactctttttctagattttttagatttgagggcaagcgctgttaacgactcagaaatgtaagcactacggagtagaacgagaaatccgccataggtggaaatcctagcaaaatcttgcttaccctagctagcctcaggtaagctagccttagcctgtcaaatttttttcaaaatttggtaagtttctactagcaaagcaaacacggttcaacaaaccgaaaactccactcattatacgtggaaaccgaaacaaaaaaacaaaaaccaaaatactcgccaatgagaaagttgctgcgtttctactttcgaggaagaggaactgagaggattgactacgaaaggggcaaaaacgagtcgtattctcccattattgtctgctaccacgcggtctagtagaataagcaaccagtcaacgctaagacaggtaatcaaaataccagtctgctggctacgggctagtttttacctcttttagaacccactgtaaaagtccgttgtaaagcccgttctcactgttggcgtttttttttttttggtttagtttcttatttttcatttttttctttcatgaccaaaaacaaacaaatctcgcgatttgtactgcggccactggggcgtggccaaaaaaatgacaaatttagaaaccttagtttctgatttttcctgttatgaggagatatgataaaaaatattactgctttattgttttttttttatctactgaaatagagaaacttacccaaggaggaggcaaaaaaaagagtatatatacagcagctaccattcagattttaatatattcttttctcttcttctacactattattataataattttactatattcatttttagcttaaaacctcatagaatattattcttcagtcactcgcttaaatacttatcaaaaatggacaagaaatactctattggtttggatatcgggaccaactccgtcggttgggctgtcatcaccgacgaatacaaggttccatccaagaaattcaaggtcttgggtaacactgacagacactctatcaagaagaatttgatcggtgctttgttgttcgactccggtgaaaccgctgaagctaccagattgaagcgtaccgctcgtcgtagatacactagacgtaaaaaccgtatttgttacttgcaagaaatcttttctaacgaaatggccaaggttgacgactctttcttccacagattggaagaatctttcttggttgaagaagacaagaagcacgaaagacatccaatcttcggtaacatcgttgacgaagttgcttaccacgaaaaataccctaccatctaccatttgagaaagaagttggtcgattccaccgacaaggctgatttgagattgatctatttggccttggctcacatgatcaagttcagaggtcacttcttgattgaaggtgacttgaacccagacaactctgacgtcgacaaattgttcatccaattggtccaaacctacaaccaattattcgaggaaaacccaattaacgcttctggtgttgatgctaaggccatcttatctgcccgtttgtccaagtctagacgtttggaaaacttgattgctcaattgcctggtgaaaagaaaaacggtttgttcggtaacttgatcgctttgtccttgggtttgaccccaaacttcaagtccaacttcgacttggctgaagatgccaagttgcaattgtccaaggacacctacgacgacgacttagacaacttgttggctcaaatcggtgaccaatacgccgacttgttcttggctgccaaaaacttatctgacgctatcttgttgtctgacatcttgagagttaacactgaaattaccaaggctccattgtctgcttctatgatcaaaagatacgacgaacaccaccaagatctgactttgttgaaggctttggttagacaacaattgccagaaaagtacaaggaaatcttcttcgaccaatccaaaaatggttacgccggttacattgacggtggtgcttctcaggaagaattctacaagttcatcaagccaattttggaaaagatggatggtactgaagaattattggttaagttgaacagagaagacttattgagaaagcaacgtaccttcgataacggttctatcccacaccaaatccacttgggtgaattgcacgccattttgagaagacaggaagatttctatccattcctaaaggacaacagagaaaagatcgaaaagatcttaactttcagaatcccatactacgtcggtccattggccagaggtaattctagattcgcttggatgaccagaaagtctgaagaaaccatcaccccatggaacttcgaagaagtcgtcgacaagggtgcttctgcccaatctttcatcgaaagaatgaccaactttgataagaacttgccaaacgagaaggtcttgccaaagcactctttgttgtacgaatacttcaccgtctacaacgaattaaccaaggttaaatacgttactgaaggtatgagaaagccagctttcctatccggtgaacaaaagaaggctattgttgacttgttgtttaagaccaacagaaaggtcactgttaagcaattgaaggaagactacttcaagaagattgaatgtttcgattccgtcgaaatctccggtgttgaagaccgtttcaatgcttctttgggcacctaccacgatttgttaaagatcatcaaggacaaggactttttagataacgaagaaaacgaagacatcttggaagatatcgttttgaccttgactcttttcgaggacagagaaatgattgaagagagattgaagacctacgctcacttgttcgacgataaagttatgaagcaactaaagagaagaagatacactggttggggtagattgtccagaaagttgattaacggtatcagagacaagcaatccggtaagactattttagactttttgaaatccgatggtttcgctaacagaaactttatgcaattgattcacgacgattctttgactttcaaggaagacattcaaaaagcccaagtctctggtcaaggtgattctttgcacgaacacatcgctaacttggctggttctccagctattaagaagggtatcttacaaaccgtcaaggtcgttgatgaattggtcaaagtcatgggtagacacaagccagaaaatattgtcatcgaaatggctagagaaaaccaaactactcaaaagggtcaaaagaactctagagaacgtatgaagagaattgaagaaggtatcaaggagttgggttctcaaattttgaaagaacacccagtcgaaaacactcaattacaaaacgaaaagctatacttgtactacttgcaaaacggtcgtgacatgtacgtcgaccaagaattggatatcaacagattgtctgactacgatgtcgatcatatcgtcccacaatcgttcttgaaggacgattccattgacaacaaagttttgactagatctgacaagaacagaggtaagtctgataacgttccatctgaagaagttgttaagaagatgaagaactactggagacaattgttgaatgctaagttgatcactcaaagaaagttcgacaacttgaccaaggctgaaagaggtggtttgtccgaattggacaaagccggtttcatcaagagacaattagtcgaaactagacaaatcaccaagcatgttgctcaaatcttggattccagaatgaacactaagtacgatgaaaacgacaaactaattagagaagttaaggtcatcactttgaagtctaagttggtttctgacttcagaaaggacttccaattttacaaggtcagagaaatcaacaactaccatcacgctcacgatgcctacttgaacgctgttgtcggtactgccttaatcaaaaagtacccaaagttggaatctgaattcgtttacggtgactacaaggtttacgatgttagaaagatgatcgccaagtctgaacaagaaattggtaaggccactgctaagtacttcttctactctaacatcatgaactttttcaagactgaaatcactttagctaacggtgaaattagaaagcgtccattgattgaaaccaatggtgaaactggtgaaattgtctgggacaagggtagagatttcgctaccgtcagaaaggttttgtctatgccacaagttaacatcgtcaagaagactgaagttcaaactggtggtttctctaaggaatccattttgccaaagagaaactctgacaagttgattgctagaaagaaggactgggatcctaagaagtacggtggtttcgactctccaactgttgcttactccgttttggtcgttgctaaggttgaaaagggtaagtctaagaagttgaagtctgttaaggaattgttgggtatcaccatcatggaaagatcctccttcgaaaagaacccaatcgactttttggaagctaagggttacaaggaagtcaagaaggatttgatcattaagttaccaaaatactccttgttcgaattggaaaacggtagaaagagaatgttggcctccgctggtgaactacaaaaaggtaacgaattggctttaccatctaagtacgttaacttcttgtacttggcttcccactacgaaaagttgaaaggttccccagaagacaacgaacaaaagcaattgtttgttgaacaacacaagcactacttggatgaaattattgaacaaatctccgaattctccaagagagtcattttggctgatgctaacttagataaggttttatccgcttacaacaagcacagagacaaaccaatcagagaacaagctgaaaacatcattcatttgttcactttaaccaacttgggtgctccagctgctttcaaatacttcgacactaccattgacagaaagagatacacttccaccaaagaagttttagatgctactttgattcaccaatctattaccggtttgtacgaaaccagaattgacttgtctcaattgggtggtgattccagagctgatccaaagaagaagagaaaggtgtaaaggagttaaaggcaaagttttcttttctagagccgttcccacaaataattatacgtatatgcttcttttcgtttactatatatctatatttacaagcctttattcactgatgcaatttgtttccaaatacttttttggagatctcataactagatatcatgatggcgcaacttggcgctatcttaattactctggctgccaggcccgtgtagagggccgcaagaccttctgtacgccatatagtctctaagaacttgaacaagtttctagacctattgccgcctttcggatcgctattgttgcggccgccagctgaagcttcgtacgctgcaggtcgacgaattctaccgttcgtataatgtatgctatacgaagttatagatctgtttagcttgcctcgtccccgccgggtcacccggccagcgacatggaggcccagaataccctccttgacagtcttgacgtgcgcagctcaggggcatgatgtgactgtcgcccgtacatttagcccatacatccccatgtataatcatttgcatccatacattttgatggccgcacggcgcgaagcaaaaattacggctcctcgctgcagacctgcgagcagggaaacgctcccctcacagacgcgttgaattgtccccacgccgcgcccctgtagagaaatataaaaggttaggatttgccactgaggttcttctttcatatacttccttttaaaatcttgctaggatacagttctcacatcacatccgaacataaacaaccatgggtaaggaaaagactcacgtttcgaggccgcgattaaattccaacatggatgctgatttatatgggtataaatgggctcgcgataatgtcgggcaatcaggtgcgacaatctatcgattgtatgggaagcccgatgcgccagagttgtttctgaaacatggcaaaggtagcgttgccaatgatgttacagatgagatggtcagactaaactggctgacggaatttatgcctcttccgaccatcaagcattttatccgtactcctgatgatgcatggttactcaccactgcgatccccggcaaaacagcattccaggtattagaagaatatcctgattcaggtgaaaatattgttgatgcgctggcagtgttcctgcgccggttgcattcgattcctgtttgtaattgtccttttaacagcgatcgcgtatttcgtctcgctcaggcgcaatcacgaatgaataacggtttggttgatgcgagtgattttgatgacgagcgtaatggctggcctgttgaacaagtctggaaagaaatgcataagcttttgccattctcaccggattcagtcgtcactcatggtgatttctcacttgataaccttatttttgacgaggggaaattaataggttgtattgatgttggacgagtcggaatcgcagaccgataccaggatcttgccatcctatggaactgcctcggtgagttttctccttcattacagaaacggctttttcaaaaatatggtattgataatcctgatatgaataaattgcagtttcatttgatgctcgatgagtttttctaatcagtactgacaataaaaagattcttgttttcaagaacttgtcatttgtatagtttttttatattgtagttgttctattttaatcaaatgttagcgtgatttatattttttttcgcctcgacatcatctgcccagatgcgaagttaagtgcgcagaaagtaatatcatgcgtcaatcgtatgtgaatgctggtcgctatactgctgtcgattcgatactaacgccgccatccagtgtcgaaaacgagctcataacttcgtataatgtatgctatacgaacggtagaattcgaatcagatccactagtgtgcccgcggaaccgccagatattcattacttgacgcaaaagcgtttgaaataatgacgaaaaagaaggaagaaaaaaaaagaaaaataccgcttctaggcgggttatctactgatccgagcttccactaggatagcacccaaacacctgcatatttggacgacctttacttacaccaccaaaaaccactttcgcctctcccgcccctgataacgtccactaattgagcgattacctgagcggtcctcttttgtttgcagcatgagacttgcatactgcaaatcgtaagtagcaacgtgtcaaggtcaaaactgtatggaaaccttgtcacctcacttaattctagctagcctaccctgcaagtcaagaggtgtccgtgattcctagccacctcaaggtatgcctctccccggaaactgtggccttttctggcacacatgatctccacgatttcaacatataaatagcttttgataatggcaatattaatcaaatttattttacttctttcttgtaacatctctcttgtaatcccttattccttctagctatttttcataaaaaaccaagcaactgcttatcaacacacaaacactaaatcaaaatgaacacaatcaatattgccaaaaatgaccccaagaaaaaacgtaaggtttttagcgatatcgagctagctgcaattcctttcaacacgctagctgatcattatggtgagcgtctggcaagagaacagctggccctagagcacgaaagttatgaaatgggagaagccaggtttagaaaaatgttcgaaagacaactaaaagccggcgaggtggctgacaacgcagccgctaagcccctgatcacgacattactaccaaaaatgattgcccgtataaacgactggtttgaggaggtgaaagctaagcgtggcaagaggcccacagcgttccagttccttcaagaaattaagcctgaagcggtcgcatatattacgattaaaaccactctagcttgtcttacaagcgcggataacacaacagtacaggctgtagctagcgcgataggcagggcaatagaggacgaggccaggttcgggcgtattcgtgatctagaagctaaacattttaaaaaaaacgtggaagaacagttaaacaagagagttgggcatgtgtacaagaaagcgttcatgcaggtcgtggaggctgacatgctttcaaaaggcctgttgggaggagaagcatggagtagctggcacaaggaggactcaatccatgtcggcgtgaggtgtattgagatgttgatagagagtacaggcatggtgtcattacaccgtcaaaacgcaggtgttgtgggccaagattctgagacgatcgaattagcaccagaatacgcggaggccatagcgactcgtgccggggcgttggcaggaatatctccaatgtttcagccatgtgtagtacctccgaagccatggactggaattaccggtgggggctattgggctaatggtagaaggccgttggcactggtcagaacccactcaaaaaaagctttgatgcgttatgaagatgtttacatgcccgaggtctataaggctatcaatatcgctcaaaacactgcgtggaaaattaataagaaagttttggctgttgcgaacgttataacaaagtggaaacactgcccagtcgaggacatccctgcgatcgagcgtgaagaattgcccatgaaacctgaagatattgatatgaaccctgaagctctgacagcgtggaaaagagcagcagccgctgtttacagaaaagataaggcaagaaaaagtaggaggatctcactagagttcatgcttgagcaggccaataagtttgccaaccacaaggccatctggtttccttataacatggactggcgtggtagggtttacgcagtctccatgtttaatcctcaaggcaacgatatgaccaaggggctgcttaccttagcaaaggggaaacccattgggaaggagggatactactggctaaaaatacatggtgcaaattgtgcaggggttgataaagtcccatttccggaaagaataaaattcattgaggagaaccatgagaacataatggcctgtgctaaatcaccacttgagaatacatggtgggcggagcaagacagtcccttttgttttctggcattctgctttgagtatgcaggggtgcagcaccatggattgagctataactgttcactacccttggcatttgatgggagttgtagtgggattcaacatttcagcgctatgttgagggatgaagtcggaggtagggccgtcaatcttctaccgtctgagacggttcaagacatttacgggatagtggctaaaaaagtcaacgagattcttcaggccgacgcgattaatggcactgataacgaggtagtaacagtgactgacgaaaacacgggagaaatatccgagaaagttaaacttgggaccaaggcgctggcaggtcaatggctggcgtacggcgttacgaggtctgttacgaaaaggagtgtcatgacattagcgtatggatctaaggaatttggatttagacagcaggtactggaggacaccatacagccagcgatcgactctggcaaaggtttaatgtttacacaacccaaccaggctgctgggtatatggcaaaattgatctgggaatccgtttcagtaactgtagtagctgcagttgaggctatgaactggctgaaaagcgccgccaaactgttagcggcagaggtaaaggacaagaaaacgggcgaaatattgagaaagagatgcgcggtccattgggtcacgcctgatgggttcccagtctggcaggaatacaagaaaccaattcaaaccagactgaaccttatgtttctggggcagtttcgtttgcagcccaccatcaataccaacaaagattcagaaattgacgcgcacaaacaagagtcagggatagctccaaacttcgtgcattcacaagacgggagtcacctgagaaagacggtggtttgggcccatgagaagtatggtatcgagtctttcgccctgattcacgactcctttggtactataccagcagacgctgcaaaccttttcaaagctgttagagagactatggtcgacacatatgagtcttgcgatgtattagctgacttctatgaccaattcgcggaccagctacatgaatcccagctagacaaaatgccggcattacccgccaaagggaatctgaatctaagagatattctggaaagcgatttcgccttcgcttaaaagcttttgattaagccttctagtccaaaaaacacgtttttttgtcatttatttcattttcttagaatagtttagtttattcattttatagtcacgaatgttttatgattctatatagggttgcaaacaagcatttttcattttatgttaaaacaatttcaggtttaccttttattctgcttgtggtgacgcgtgtatccgcccgctcttttggtcacccatgtatttaattgcataaataattcttaaaagtggagctagtctatttctatttacatacctctcatttctcatttcctcccctcccgcggtggagctccagcttttgttccctttagtgagggttaattgcgcgcttggcgtaatcatggtcatagctgtttcctgtgtgaaattgttatccgctcacaattccacacaacataggagccggaagcataaagtgtaaagcctggggtgcctaatgagtgaggtaactcacattaattgcgttgcgctcactgcccgctttccagtcgggaaacctgtcgtgccagctgcattaatgaatcggccaacgcgcggggagaggcggtttgcgtattgggcgctcttccgcttcctcgctcactgactcgctgcgctcggtcgttcggctgcggcgagcggtatcagctcactcaaaggcggtaatacggttatccacagaatcaggggataacgcaggaaagaacatgtgagcaaaaggccagcaaaaggccaggaaccgtaaaaaggccgcgttgctggcgtttttccataggctccgcccccctgacgagcatcacaaaaatcgacgctcaagtcagaggtggcgaaacccgacaggactataaagataccaggcgtttccccctggaagctccctcgtgcgctctcctgttccgaccctgccgcttaccggatacctgtccgcctttctcccttcgggaagcgtggcgctttctcatagctcacgctgtaggtatctcagttcggtgtaggtcgttcgctccaagctgggctgtgtgcacgaaccccccgttcagcccgaccgctgcgccttatccggtaactatcgtcttgagtccaacccggtaagacacgacttatcgccactggcagcagccactggtaacaggattagcagagcgaggtatgtaggcggtgctacagagttcttgaagtggtggcctaactacggctacactagaaggacagtatttggtatctgcgctctgctgaagccagttaccttcggaaaaagagttggtagctcttgatccggcaaacaaaccaccgctggtagcggtggtttttttgtttgcaagcagcagattacgcgcagaaaaaaaggatctcaagaagatcctttgatcttttctacggggtctgacgctcagtggaacgaaaactcacgttaagggattttggtcatgagattatcaaaaaggatcttcacctagatccttttaaattaaaaatgaagttttaaatcaatctaaagtatatatgagtaaacttggtctgacagttaccaatgcttaatcagtgaggcacctatctcagcgatctgtctatttcgttcatccatagttgcctgactccccgtcgtgtagataactacgatacgggagggcttaccatctggccccagtgctgcaatgataccgcgagacccacgctcaccggctccagatttatcagcaataaaccagccagccggaagggccgagcgcagaagtggtcctgcaactttatccgcctccatccagtctattaattgttgccgggaagctagagtaagtagttcgccagttaatagtttgcgcaacgttgttgccattgctacaggcatcgtggtgtcacgctcgtcgtttggtatggcttcattcagctccggttcccaacgatcaaggcgagttacatgatcccccatgttgtgcaaaaaagcggttagctccttcggtcctccgatcgttgtcagaagtaagttggccgcagtgttatcactcatggttatggcagcactgcataattctcttactgtcatgccatccgtaagatgcttttctgtgactggtgagtactcaaccaagtcattctgagaatagtgtatgcggcgaccgagttgctcttgcccggcgtcaatacgggataataccgcgccacatagcagaactttaaaagtgctcatcattggaaaacgttcttcggggcgaaaactctcaaggatcttaccgctgttgagatccagttcgatgtaacccactcgtgcacccaactgatcttcagcatcttttactttcaccagcgtttctgggtgagcaaaaacaggaaggcaaaatgccgcaaaaaagggaataagggcgacacggaaatgttgaatactcatactcttcctttttcaatattattgaagcatttatcagggttattgtctcatgagcggatacatatttgaatgtatttagaaaaataaacaaataggggttccgcgcacatttccccgaaaagtgccacctgggtccttttcatcacgtgctataaaaataattataatttaaattttttaatataaatatataaattaaaaatagaaagtaaaaaaagaaattaaagaaaaaatagtttttgttttccgaagatgtaaaagactctagggggatcgccaacaaatactaccttttatcttgctcttcctgctctcaggtattaa

SEQ ID NO: 29 - DNA, 20 bp, Artificial Sequence
  Nucleotide sequence of the INT1 genomic target
tattagaaccagggaggtcc

SEQ ID NO: 30 - DNA, 68 bp, Artificial Sequence
  Nucleotide sequence of the Hepatitis Delta Virus ribozyme (HDVr)
ggccggcatggtcccagcctcctcgctggcgccggctgggcaacatgcttcggcatggcgaatgggac

SEQ ID NO: 31 - DNA, 47 bp, Artificial Sequence
  Nucleotide sequence of the T7 terminator
aaaaaatcaaactggctcaccttcgggtgggcctttttgcgtttata

SEQ ID NO: 32 - DNA, 23 bp, Artificial Sequence
  Nucleotide sequence of a weak strength T7 promoter that was used for gRNA expression
taatacgactcactaatactgaa

SEQ ID NO: 33 - DNA, 23 bp, Artificial Sequence
  Nucleotide sequence of a medium strength T7 promoter that was used for gRNA expression
taatacgactcactacggaagaa

SEQ ID NO: 34 - DNA, 23 bp, Artificial Sequence
  Nucleotide sequence of a strong T7 promoter that was used for gRNA expression
taatacgactcactataggggaa

SEQ ID NO: 35 - DNA, 18 bp, Artificial Sequence
  Nucleotide sequence of a wild type strength T7 promoter that was used for gRNA expression
taatacgactcactatag

SEQ ID NO: 36 - DNA, 238 bp, Artificial Sequence
  Nucleotide sequence of a guide RNA expression cassette under control of the strong T7 promoter
taatacgactcactataggggaatattagaaccagggaggtccgttttagagctagaaatagcaagttaaaataaggctagtccgttatcaacttgaaaaagtggcaccgagtcggtgcttttggccggcatggtcccagcctcctcgctggcgccggctgggcaacatgcttcggcatggcgaatgggacaaaaaatcaaactggctcaccttcgggtgggcctttttgcgtttata

SEQ ID NO: 37 - DNA, 238 bp, Artificial Sequence
  Nucleotide sequence of a guide RNA expression cassette under control of the medium T7 promoter
taatacgactcactacggaagaatattagaaccagggaggtccgttttagagctagaaatagcaagttaaaataaggctagtccgttatcaacttgaaaaagtggcaccgagtcggtgcttttggccggcatggtcccagcctcctcgctggcgccggctgggcaacatgcttcggcatggcgaatgggacaaaaaatcaaactggctcaccttcgggtgggcctttttgcgtttata

SEQ ID NO: 38 - DNA, 238 bp, Artificial Sequence
  Nucleotide sequence of a guide RNA expression cassette under control of the weak T7 promoter
taatacgactcactaatactgaatattagaaccagggaggtccgttttagagctagaaatagcaagttaaaataaggctagtccgttatcaacttgaaaaagtggcaccgagtcggtgcttttggccggcatggtcccagcctcctcgctggcgccggctgggcaacatgcttcggcatggcgaatgggacaaaaaatcaaactggctcaccttcgggtgggcctttttgcgtttata

SEQ ID NO: 39 - DNA, 233 bp, Artificial Sequence
  Nucleotide sequence of a guide RNA expression cassette under control of the wildtype T7 promoter
taatacgactcactatagtattagaaccagggaggtccgttttagagctagaaatagcaagttaaaataaggctagtccgttatcaacttgaaaaagtggcaccgagtcggtgcttttggccggcatggtcccagcctcctcgctggcgccggctgggcaacatgcttcggcatggcgaatgggacaaaaaatcaaactggctcaccttcgggtgggcctttttgcgtttata

SEQ ID NO: 40 - DNA, 21 bp, Artificial Sequence
  Nucleotide sequence of the forward primer used to obtain the T7 controlled guide RNA fragment used in transformation
catgtttgacagcttatcatc

SEQ ID NO: 41 - DNA, 21 bp, Artificial Sequence
  Nucleotide sequence of the reverse primer used to obtain the T7 controlled guide RNA fragment used in transformation
cacacaggaaacagctatgac

SEQ ID NO: 42 - DNA, 415 bp, Artificial Sequence
  Nucleotide sequence of the guide RNA fragment controlled by strong T7 promoter used in transformation flanked by 84 bp sequence of pRN1120 on the 5' side and 93 bp sequence of pRN1120 on the 3' side for in vivo assembly into the vector pRN1120
catgtttgacagcttatcatcgataatccggagctagcatgcggccgctctagaactagtggatcccccgggctgcaggaattctaatacgactcactataggggaatattagaaccagggaggtccgttttagagctagaaatagcaagttaaaataaggctagtccgttatcaacttgaaaaagtggcaccgagtcggtgcttttggccggcatggtcccagcctcctcgctggcgccggctgggcaacatgcttcggcatggcgaatgggacaaaaaatcaaactggctcaccttcgggtgggcctttttgcgtttatactcgagggggggcccggtacccagcttttgttccctttagtgagggttaattccgagcttggcgtaatcatggtcatagctgtttcctgtgtg

SEQ ID NO: 43 - DNA, 415 bp, Artificial Sequence
  Nucleotide sequence of the guide RNA fragment controlled by medium T7 promoter used in transformation flanked by 84 bp sequence of pRN1120 on the 5' side and 93 bp sequence of pRN1120 on the 3' side for in vivo assembly into the vector pRN1120
catgtttgacagcttatcatcgataatccggagctagcatgcggccgctctagaactagtggatcccccgggctgcaggaattctaatacgactcactacggaagaatattagaaccagggaggtccgttttagagctagaaatagcaagttaaaataaggctagtccgttatcaacttgaaaaagtggcaccgagtcggtgcttttggccggcatggtcccagcctcctcgctggcgccggctgggcaacatgcttcggcatggcgaatgggacaaaaaatcaaactggctcaccttcgggtgggcctttttgcgtttatactcgagggggggcccggtacccagcttttgttccctttagtgagggttaattccgagcttggcgtaatcatggtcatagctgtttcctgtgtg

SEQ ID NO: 44 - DNA, 415 bp, Artificial Sequence
  Nucleotide sequence of the guide RNA fragment controlled by weak T7 promoter used in transformation flanked by 84 bp sequence of pRN1120 on the 5' side and 93 bp sequence of pRN1120 on the 3' side for in vivo assembly into the vector pRN1120
catgtttgacagcttatcatcgataatccggagctagcatgcggccgctctagaactagtggatcccccgggctgcaggaattctaatacgactcactaatactgaatattagaaccagggaggtccgttttagagctagaaatagcaagttaaaataaggctagtccgttatcaacttgaaaaagtggcaccgagtcggtgcttttggccggcatggtcccagcctcctcgctggcgccggctgggcaacatgcttcggcatggcgaatgggacaaaaaatcaaactggctcaccttcgggtgggcctttttgcgtttatactcgagggggggcccggtacccagcttttgttccctttagtgagggttaattccgagcttggcgtaatcatggtcatagctgtttcctgtgtg

SEQ ID NO: 45 - DNA, 410 bp, Artificial Sequence
  Nucleotide sequence of the guide RNA fragment controlled by wild type T7 promoter used in transformation flanked by 84 bp sequence of pRN1120 on the 5' side and 93 bp sequence of pRN1120 on the 3' side for in vivo assembly into the vector pRN1120
catgtttgacagcttatcatcgataatccggagctagcatgcggccgctctagaactagtggatcccccgggctgcaggaattctaatacgactcactatagtattagaaccagggaggtccgttttagagctagaaatagcaagttaaaataaggctagtccgttatcaacttgaaaaagtggcaccgagtcggtgcttttggccggcatggtcccagcctcctcgctggcgccggctgggcaacatgcttcggcatggcgaatgggacaaaaaatcaaactggctcaccttcgggtgggcctttttgcgtttatactcgagggggggcccggtacccagcttttgttccctttagtgagggttaattccgagcttggcgtaatcatggtcatagctgtttcctgtgtg

SEQ ID NO: 46 - DNA, 100 bp, Artificial Sequence
  Nucleotide sequence of upper strand of the 100 bp left flank
cttcatgccagcaatagttgcgtgctgagctcaacagtgcccaacccttgaagcgacttccaatcgctttgcatatccagtaccacacccacaggcgttt

SEQ ID NO: 47 - DNA, 100 bp, Artificial Sequence
  Nucleotide sequence of the 100 bp left flank in the reverse orientation complementary to SEQ ID NO: 46
aaacgcctgtgggtgtggtactggatatgcaaagcgattggaagtcgcttcaagggttgggcactgttgagctcagcacgcaactattgctggcatgaag

SEQ ID NO: 48 - DNA, 100 bp, Artificial Sequence
  Nucleotide sequence of the 100 bp right flank in the forward orientation
agaaagcctgtatgcgaagccacaatcctttccaacagaccatactaagtattctttgtcatcagacaacttgttgagtggtactaaaggagtgcttttc

SEQ ID NO: 49 - DNA, 100 bp, Artificial Sequence
  Nucleotide sequence of the 100 bp right flank in the reverse orientation complementary to SEQ ID NO: 48
gaaaagcactcctttagtaccactcaacaagttgtctgatgacaaagaatacttagtatggtctgttggaaaggattgtggcttcgcatacaggctttct

SEQ ID NO: 50 - DNA, 1726 bp, Artificial Sequence
  Nucleotide sequence of the YFP donor DNA expression cassette
aagcgacttccaatcgctttgcatatccagtaccacacccacaggcgtttgtgcttagtcaaaaaattagccttttaattctgctgtaacccgtacatgcccaaaatagggggcgggttacacagaatatataacatcgtaggtgtctgggtgaacagtttattcctggcatccactaaatataatggagcccgctttttaagctggcatccagaaaaaaaaagaatcccagcaccaaaatattgttttcttcaccaaccatcagttcataggtccattctcttagcgcaactacagagaacaggggcacaaacaggcaaaaaacgggcacaacctcaatggagtgatgcaacctgcctggagtaaatgatgacacaaggcaattgacccacgcatgtatctatctcattttcttacaccttctattaccttctgctctctctgatttggaaaaagctgaaaaaaaaggttgaaaccagttccctgaaattattcccctacttgactaataagtatataaagacggtaggtattgattgtaattctgtaaatctatttcttaaacttcttaaattctacttttatagttagtcttttttttagttttaaaacaccaagaacttagtttcgaataaacacacataaacaaacaaaatgtctaaaggtgaagaattattcactggtgttgtcccaattttggttgaattagatggtgatgttaatggtcacaaattttctgtctccggtgaaggtgaaggtgatgctacttacggtaaattgaccttaaaattgatttgtactactggtaaattgccagttccatggccaaccttagtcactactttaggttatggtttgcaatgttttgctagatacccagatcatatgaaacaacatgactttttcaagtctgccatgccagaaggttatgttcaagaaagaactatttttttcaaagatgacggtaactacaagaccagagctgaagtcaagtttgaaggtgataccttagttaatagaatcgaattaaaaggtattgattttaaagaagatggtaacattttaggtcacaaattggaatacaactataactctcacaatgtttacatcactgctgacaaacaaaagaatggtatcaaagctaacttcaaaattagacacaacattgaagatggtggtgttcaattagctgaccattatcaacaaaatactccaattggtgatggtccagtcttgttaccagacaaccattacttatcctatcaatctgccttatccaaagatccaaacgaaaagagagatcacatggtcttgttagaatttgttactgctgctggtattacccatggtatggatgaattgtacaaataaaagcttttgattaagccttctagtccaaaaaacacgtttttttgtcatttatttcattttcttagaatagtttagtttattcattttatagtcacgaatgttttatgattctatatagggttgcaaacaagcatttttcattttatgttaaaacaatttcaggtttaccttttattctgcttgtggtgacgcgtgtatccgcccgctcttttggtcacccatgtatttaattgcataaataattcttaaaagtggagctagtctatttctatttacatacctctcatttctcatttcctcccctcagaaagcctgtatgcgaagccacaatcctttccaacagaccatactaagt

SEQ ID NO: 51 - DNA, 23 bp, Artificial Sequence
  Nucleotide sequence forward primer to obtain the 577 bp left flank for integration of the YFP donor DNA cassette
cactatagcaatctggctatatg

SEQ ID NO: 52 - DNA, 70 bp, Artificial Sequence
  Nucleotide sequence reverse primer to obtain the 577 bp left flank for integration of the YFP donor DNA cassette
aaacgcctgtgggtgtggtactggatatgcaaagcgattggaagtcgcttgactcctctgccgtcattcc

SEQ ID NO: 53 - DNA, 577 bp, Artificial Sequence
  Nucleotide sequence of the left flank for integration of YFP donor expression cassette in INT1 locus of S. cerevisiae
cactatagcaatctggctatatgatatgcagaaaatagtgattactgtgctctttgctgcatcatgcatcatatgtttggcattctgtcctgtcagatgaatgggcgaaacaattcggggagctttgttgcgacttggtacccggcaagccgcgacctatattttgcattaaacgagttcatcgtggatttatcgccatgagccttagcttatcaagcctctcacagacaattaagcaatgaaaaaggtataccatcggcgcagaatggttaactagtgggttcatactgctgtgttatagattgttacctaagtgatcaccaaaaaaaagtgcaaaaaggaaaaaaaaataagagacaggtaacttccacaagcttattcttccaaaaatcaatcttatcttcatgccagcaatagttgcgtgctgagctcaacagtgcccaacccttgtgcaccgtagaattgtagaatacaaatacataaataagtgtgttcccgaaggactaaggaatgacggcagaggagtcaagcgacttccaatcgctttgcatatccagtaccacacccacaggcgttt

SEQ ID NO: 54 - DNA, 72 bp, Artificial Sequence
  Nucleotide sequence forward primer to obtain the 581 bp right flank for integration of the YFP donor DNA expression cassette
agaaagcctgtatgcgaagccacaatcctttccaacagaccatactaagtaagcgttgaagtttcctctttg

SEQ ID NO: 55 - DNA, 20 bp, Artificial Sequence
  Nucleotide sequence reverse primer to obtain the 581 bp right flank for integration of the YFP donor DNA expression cassette
tgtcaactggagagctatcg

SEQ ID NO: 56 - DNA, 581 bp, Artificial Sequence
  Nucleotide sequence of the right flank for integration of YFP donor expression cassette in INT1 locus of S. cerevisiae
agaaagcctgtatgcgaagccacaatcctttccaacagaccatactaagtaagcgttgaagtttcctctttgtatatttgagatcttcattttatcggattctttgtcatcagacaacttgttgagtggtactaaaggagtgcttttcatcatccttttggtgaacgatttcaaatacgttagtgttttctgagctagttttgatcaattcaggtgattcgttatcagaactctcaggtttgtattcgtgtccagttgtgtagcattcgcctaacgtgtaagcacggatttcttcctcagaaatttcactgtatggaatcatgcccttctttctcgcttcttcgtcggtaaatgcaccatagtaatctttgtcatcatgtctaacagtaattttgaatgggaagaagacacatagcccccagtaaacgaaaaaagaaatcaaaaaggagaagaaagaatcaccataaaagaatttaacaatacctgagtcgtggaaatagttattgttgacttcccaagcgataccaggtagaccgggagccataccacacacccaggcaacgatagctctccagttgaca

SEQ ID NO: 57 - DNA, 31 bp, Artificial Sequence
  Nucleotide sequence of the forward primer for amplification of the YFP expression cassette
gtgcttagtcaaaaaattagccttttaattc

SEQ ID NO: 58 - DNA, 23 bp, Artificial Sequence
  Nucleotide sequence of the reverse primer for amplification of the YFP expression cassette
gaggggaggaaatgagaaatgag

SEQ ID NO: 59 - DNA, 72 bp, Artificial Sequence
  Nucleotide sequence of the forward primer for amplification of the YFP donor DNA expression cassette including connector 5 on the 5' side
aagcgacttccaatcgctttgcatatccagtaccacacccacaggcgtttgtgcttagtcaaaaaattagcc

SEQ ID NO: 60 - DNA, 73 bp, Artificial Sequence
  Nucleotide sequence of the reverse primer for amplification of the YFP donor DNA expression cassette including connector 3 on the 3' side
acttagtatggtctgttggaaaggattgtggcttcgcatacaggctttctgaggggaggaaatgagaaatgag

SEQ ID NO: 61 - DNA, 80 bp, Artificial Sequence
  Nucleotide sequence of the guide RNA structural element as described by DiCarlo
gttttagagctagaaatagcaagttaaaataaggctagtccgttatcaacttgaaaaagtggcaccgagtcggtgctttt

SEQ ID NO: 62 - DNA, 998 bp, Artificial Sequence
  Nucleotide sequence of ordered gBlock donor DNA with fwnA as target
caactggaagcaatatcaccaggactttagctcctctctccaggtcctccgcctcccagcctacaagtgggatctcaagaactactggattccctataccaacaacttctgcctgagcaagggcgctccagttgcgacagtagcggcagggccacagcatgagtacctgacaaccgcggctcagaaggtcattgagactcgaagtgatggagcaacagctacagtcgtgatagagaacgacattgctgatcccgagctcaaccgcgtcattcaaggccataaggtcaacggtactgctttgtgtccctcatcactatatgccgacatctctcaaacgcttgcagagtatctcatcaaaaagtacaagcctgagtacgacggacttggactggatgtgtgtgaggtcacagtgccacgaccactgattgcgaaaggcggacagcagctctttagagtatctgcgacagcggattgggcggagaagaagacaacccatatattcagtcactgccgaggggaagaagacggctgaccacgcaacttgcactgtccgattctttgactgcgctgctgcggaggcggaatggaaacgagtttcctaccttgtcaagaggagcattgaccgactgcatgatatcgccgaaaatggtgacgctcaccgtcttggtagaggcatggtttacaaactcttcgctgccttggttgattatgacgacaacttcaagtccattcgcgaggttattcttgacagtgaacagcacgaagcgactgcacgcgtcaagttccaagcaccacaaggcaatttccaccgaaacccgttctggattgacagttttggacacctgtctgggttcatcatgaacgcaagcgatgcaaccgactccaagaaccaggtctttgtcaatcacggatgggactccatgcgttgtttgaagaagttctcgcctgatgtcacctacaggacttatgttagaatgcagccttggaaagactccatc

SEQ ID NO: 63 - DNA, 4517 bp, Artificial Sequence
  Nucleotide sequence of TOPO vector with donor DNA (target fwnA) result of cloning gBlock donor DNA in TOPO-vector
agcgcccaatacgcaaaccgcctctccccgcgcgttggccgattcattaatgcagctggcacgacaggtttcccgactggaaagcgggcagtgagcgcaacgcaattaatgtgagttagctcactcattaggcaccccaggctttacactttatgcttccggctcgtatgttgtgtggaattgtgagcggataacaatttcacacaggaaacagctatgaccatgattacgccaagctatttaggtgacactatagaatactcaagctatgcatcaagcttggtaccgagctcggatccactagtaacggccgccagtgtgctggaattcgcccttcaactggaagcaatatcaccaggactttagctcctctctccaggtcctccgcctcccagcctacaagtgggatctcaagaactactggattccctataccaacaacttctgcctgagcaagggcgctccagttgcgacagtagcggcagggccacagcatgagtacctgacaaccgcggctcagaaggtcattgagactcgaagtgatggagcaacagctacagtcgtgatagagaacgacattgctgatcccgagctcaaccgcgtcattcaaggccataaggtcaacggtactgctttgtgtccctcatcactatatgccgacatctctcaaacgcttgcagagtatctcatcaaaaagtacaagcctgagtacgacggacttggactggatgtgtgtgaggtcacagtgccacgaccactgattgcgaaaggcggacagcagctctttagagtatctgcgacagcggattgggcggagaagaagacaacccatatattcagtcactgccgaggggaagaagacggctgaccacgcaacttgcactgtccgattctttgactgcgctgctgcggaggcggaatggaaacgagtttcctaccttgtcaagaggagcattgaccgactgcatgatatcgccgaaaatggtgacgctcaccgtcttggtagaggcatggtttacaaactcttcgctgccttggttgattatgacgacaacttcaagtccattcgcgaggttattcttgacagtgaacagcacgaagcgactgcacgcgtcaagttccaagcaccacaaggcaatttccaccgaaacccgttctggattgacagttttggacacctgtctgggttcatcatgaacgcaagcgatgcaaccgactccaagaaccaggtctttgtcaatcacggatgggactccatgcgttgtttgaagaagttctcgcctgatgtcacctacaggacttatgttagaatgcagccttggaaagactccatcaagggcgaattctgcagatatccatcacactggcggccgctcgagcatgcatctagagggcccaattcgccctatagtgagtcgtattacaattcactggccgtcgttttacaacgtcgtgactgggaaaaccctggcgttacccaacttaatcgccttgcagcacatccccctttcgccagctggcgtaatagcgaagaggcccgcaccgatcgcccttcccaacagttgcgcagcctatacgtacggcagtttaaggtttacacctataaaagagagagccgttatcgtctgtttgtggatgtacagagtgatattattgacacgccggggcgacggatggtgatccccctggccagtgcacgtctgctgtcagataaagtctcccgtgaactttacccggtggtgcatatcggggatgaaagctggcgcatgatgaccaccgatatggccagtgtgccggtctccgttatcggggaagaagtggctgatctcagccaccgcgaaaatgacatcaaaaacgccattaacctgatgttctggggaatataaatgtcaggcatgagattatcaaaaaggatcttcacctagatccttttcacgtagaaagccagtccgcagaaacggtgctgaccccggatgaatgtcagctactgggctatctggacaagggaaaacgcaagcgcaaagagaaagcaggtagcttgcagtgggcttacatggcgatagctagactgggcggttttatggacagcaagcgaaccggaattgccagctggggcgccctctggtaaggttgggaagccctgcaaagtaaactggatggctttctcgccgccaaggatctgatggcgcaggggatcaagctctgatcaagagacaggatgaggatcgtttcgcatgattgaacaagatggattgcacgcaggttctccggccgcttgggtggagaggctattcggctatgactgggcacaacagacaatcggctgctctgatgccgccgtgttccggctgtcagcgcaggggcgcccggttctttttgtcaagaccgacctgtccggtgccctgaatgaactgcaagacgaggcagcgcggctatcgtggctggccacgacgggcgttccttgcgcagctgtgctcgacgttgtcactgaagcgggaagggactggctgctattgggcgaagtgccggggcaggatctcctgtcatctcaccttgctcctgccgagaaagtatccatcatggctgatgcaatgcggcggctgcatacgcttgatccggctacctgcccattcgaccaccaagcgaaacatcgcatcgagcgagcacgtactcggatggaagccggtcttgtcgatcaggatgatctggacgaagagcatcaggggctcgcgccagccgaactgttcgccaggctcaaggcgagcatgcccgacggcgaggatctcgtcgtgacccatggcgatgcctgcttgccgaatatcatggtggaaaatggccgcttttctggattcatcgactgtggccggctgggtgtggcggaccgctatcaggacatagcgttggctacccgtgatattgctgaagagcttggcggcgaatgggctgaccgcttcctcgtgctttacggtatcgccgctcccgattcgcagcgcatcgccttctatcgccttcttgacgagttcttctgaattattaacgcttacaatttcctgatgcggtattttctccttacgcatctgtgcggtatttcacaccgcatacaggtggcacttttcggggaaatgtgcgcggaacccctatttgtttatttttctaaatacattcaaatatgtatccgctcatgagacaataaccctgataaatgcttcaataatagcacgtgaggagggccaccatggccaagttgaccagtgccgttccggtgctcaccgcgcgcgacgtcgccggagcggtcgagttctggaccgaccggctcgggttctcccgggacttcgtggaggacgacttcgccggtgtggtccgggacgacgtgaccctgttcatcagcgcggtccaggaccaggtggtgccggacaacaccctggcctgggtgtgggtgcgcggcctggacgagctgtacgccgagtggtcggaggtcgtgtccacgaacttccgggacgcctccgggccggccatgaccgagatcggcgagcagccgtgggggcgggagttcgccctgcgcgacccggccggcaactgcgtgcacttcgtggccgaggagcaggactgacacgtgctaaaacttcatttttaatttaaaaggatctaggtgaagatcctttttgataatctcatgaccaaaatcccttaacgtgagttttcgttccactgagcgtcagaccccgtagaaaagatcaaaggatcttcttgagatcctttttttctgcgcgtaatctgctgcttgcaaacaaaaaaaccaccgctaccagcggtggtttgtttgccggatcaagagctaccaactctttttccgaaggtaactggcttcagcagagcgcagataccaaatactgtccttctagtgtagccgtagttaggccaccacttcaagaactctgtagcaccgcctacatacctcgctctgctaatcctgttaccagtggctgctgccagtggcgataagtcgtgtcttaccgggttggactcaagacgatagttaccggataaggcgcagcggtcgggctgaacggggggttcgtgcacacagcccagcttggagcgaacgacctacaccgaactgagatacctacagcgtgagctatgagaaagcgccacgcttcccgaagggagaaaggcggacaggtatccggtaagcggcagggtcggaacaggagagcgcacgagggagcttccagggggaaacgcctggtatctttatagtcctgtcgggtttcgccacctctgacttgagcgtcgatttttgtgatgctcgtcaggggggcggagcctatggaaaaacgccagcaacgcggcctttttacggttcctgggcttttgctggccttttgctcacatgttctttcctgcgttatcccctgattctgtggataaccgtattaccgcctttgagtgagctgataccgctcgccgcagccgaacgaccgagcgcagcgagtcagtgagcgaggaagcggaag

SEQ ID NO: 64 - DNA, 23 bp, Artificial Sequence
  Nucleotide sequence of forward primer donor DNA PCR fragment (target fwnA)
caactggaagcaatatcaccagg

SEQ ID NO: 65 - DNA, 21 bp, Artificial Sequence
  Nucleotide sequence of reverse primer donor DNA PCR fragment (target fwnA)
gatggagtctttccaaggctg

SEQ ID NO: 66 - DNA, 31 bp, Artificial Sequence
  Nucleotide sequence of forward primer to amplify the Cas9 cassette with additional KpnI-flank for ligation in AMA-vector
cccggtaccgcaactctctggaaatgaaggc

SEQ ID NO: 67 - DNA, 30 bp, Artificial Sequence
  Nucleotide sequence of reverse primer to amplify the Cas9 cassette with additional KpnI-flank for ligation in AMA-vector
cccggtaccgaggttcatggtatgggcacg

SEQ ID NO: 68 - DNA, 19569 bp, Artificial Sequence
  Nucleotide sequence of BG-AMA17 (Cas9/hygB) - result of ligation PCR-fragment (Cas9-cassette with KpnI-flanks) and BG-AMA8
ggtaccgaggttcatggtatgggcacgaatgtcaaaaattttcaggctcaaacgggtatgtattcagtatctatctccgtgtacgacggctaattgagcccagctgcatttcgaactcttctcccagcgcattttgtgtgggagttcttcgatgctgaccatgactgcgaggctgctgagggagtgcgcggtatctaccccggcccgtatctggcttctacaaggagtgaaactagtttatactttgtagttcggaatccaatgctattaaccgtttttactttttcttttgttcgagctaagcgcttgtttaaaccttgcgcttcttcttgggatcggcacgagagtcaccaccgagctgagacaggtcgatacgagtctcgtacagaccggtaatcgactggtggatcagagtcgcatcaagcacttccttggtggaggtgtaacgcttgcggtcgatggtggtgtcaaagtacttgaaagcagcaggagcacccaggttggtgagggtgaacaggtggatgatgttctccgcctgctcgcggatgggcttgtcacggtgcttgttgtaggcagagaggaccttgtcaaggttggcatcggccaggatgacacgcttgctgaactcggagatctgctcgatgatctcatccaggtagtgcttgtgctgctcgacaaagagctgcttctgctcgttgtcctcgggagagcccttgagcttctcgtagtgggaggccaggtagaggaagttgacgtacttggaggggagggcaagctcgttacccttctggagctcaccggcggaagcaagcatgcgcttacggccgttctccagctcgaacagagagtacttggggagcttgatgatgaggtccttcttgacctctttgtaacccttggcctccaggaagtcgatagggttcttctcgaagctgctgcgttccatgatggtgataccgaggagttccttcacactcttcagcttcttgctcttgcccttctcgaccttggcgacaaccaagacggagtaggcaacggtaggcgaatcgaatccaccgtacttcttggggtcccaatccttcttgcgagcgatcagcttgtcggagttgcgcttgggaagaatcgactccttggagaaaccaccagtctgcacctcggtcttcttgacaatgttgacctggggcatagaaaggaccttgcggacggtagcgaagtcacggcccttgtcccagacgatctcaccggtttcgccgttagtctcaatcaagggacgcttgcgaatctcgccgttggccaatgttatttcggtcttgaagaagttcatgatgttgctgtagaagaagtacttggcagtggcctttccgatctcctgctcggacttagcgatcatcttgcgcacgtcgtacaccttgtagtcaccgtagacgaactcggactcgagcttgggatacttcttaatcaaagcagtaccgacgacggcgttgaggtaggcatcgtgagcgtggtggtagttgttgatctcgcggaccttgtagaactggaagtctttcctaaagtcactgaccagcttgctctttaaggtgatgaccttgacctcacggatgagcttgtcgttctcgtcgtacttggtgttcatgcgagagtccaggatctgggcaacgtgcttagtgatctgacgggtttcaaccaattgacgcttgatgaaaccggccttgtcgagctcggagagtccgccacgctcggccttggtaaggttgtcgaacttgcgctgagtgatgagcttagcgttgagcaattgtctccagtagttcttcatcttcttaacaacctcttccgaggggacgttatcgctcttgccacgattcttgtcggaacgggtgagcaccttgttgtcaatgctgtcatccttgaggaaggactgggggacgatgtggtcaacatcgtagtcggagaggcggttgatatccagctcctggtcgacgtacatgtcacgtccgttctgcaagtagtagaggtagagcttctcattctgcagctgggtgttctcgacggggtgttccttgagaatctgggaaccgagctccttgatgccttcctcgatacgcttcatgcgctcacggctgttcttctgacccttctgagtggtctggttctcacgagccatttcgatgacgatgttctcgggcttgtgacgacccatgaccttcacaagctcgtcaacaaccttcacagtctgcaggatacccttcttgatagcgggggaaccagccaggttggcaatgtgttcgtgtagcgagtcaccctggccggagacttgggccttctggatgtcctctttgaaggtcagagagtcgtcgtggatgagctgcatgaagttgcggttggcgaagccgtcggacttcaggaagtcaaggatggtcttgccagactgcttatcacggataccgttaatcaacttgcgagagaggcgaccccagccagtgtaacggcggcgcttcaactgcttcatgaccttgtcgtcgaagaggtgagcgtaggtcttcagacgttcttcgatcatctcacggtcctcgaagagggtgagggtaagaacaatgtcctcaagaatgtcttcgttctcctcgttgtcaaggaagtccttgtccttgatgatcttgagcagatcgtggtaggtgccgagagaagcgttgaagcggtcctcaacaccggagatctcaacggagtcaaagcactcgatcttcttgaagtagtcttccttgagctgcttgacggtcaccttgcggttagtcttgaacagcaggtcgacaatggccttcttctgttcgccggagaggaaagcaggcttgcgcatgccctcggtcacgtacttgaccttggtcagctcgttgtagacagtgaagtactcgtacaagagggagtgcttgggcaggactttctcgttgggcaggttcttgtcgaagttggtcatacgctcaatgaagctctgagcggaggcacccttgtcgacgacttcctcgaagttccagggggtgatggtttcctcggacttgcgggtcatccaggcgaagcgggagttaccgcgagccagaggaccgacgtagtaggggatacggaaggtcaggatcttctcaatcttctcacggttgtccttcaagaaagggtagaagtcttcctggcgacgaaggatggcgtgcaattcacccaggtggatctggtgggggatgctgccgttgtcgaaagtacgctgcttgcgcagaaggtcctcacggttcagcttaacaagaagctcctcagtgccatccatcttctcgaggataggcttaatgaacttgtagaattcttcctgggaagcaccaccgtcgatgtaaccggcgtagccgttcttggactggtcgaagaagatctccttgtacttttcggggagctgctggcggaccagagccttgagtagggtgaggtcctggtggtgctcatcgtatctcttgatcatagaggcggagagaggggccttggtgatctcagtgttgacacggaggatatctgacaggagaatggcatcggagaggttcttggcagctaggaagaggtcggcgtactgatctcctatctgggcgagaaggttatcaaggtcgtcgtcgtaggtatccttggaaagttgtaacttagcatcctcagcaagatcgaagttgctcttgaagttgggagtcagtccgagggacagggcaataaggttgccgaaaagaccgttcttcttctcaccagggagctgggcaatcaagttctcaagacggcgggacttgctcaggcgagcggagaggatggccttggcatccacgccagacgcgttgatggggttttcctcgaaaagctggttgtaggtctgaacgagctggatgaagagtttatcaacatcggagttgtcggggttgaggtcaccctcgatcaggaagtgaccacggaacttgatcatgtgcgccagagccaggtaaatgaggcggaggtcagccttgtcggtgctgtcgacgagctttttgcgtaggtggtagatggtggggtacttctcgtggtaagcgacctcatcgacaatgttaccgaagatagggtgacgctcgtgcttcttgtcttcttcaacaaggaacgactcctccagacggtggaagaaagagtcatcaaccttggccatctcgttggagaaaatctcctggaggtagcagatacggttcttgcggcgagtgtaacgacggcgagcggtacgcttcagacgggtggcctcagcagtctcaccggagtcgaagagaagcgcaccaatgaggttcttcttgatggagtgacgatcggtgtttcccaggaccttgaatttcttgctaggaaccttgtactcgtcggtgatgacagcccagccaacggagttggtgccaatgtccagaccgatgctatacttcttgtccattttgacggtggaaggtgagttggggttggtgtcatcgtgggggaagaacttggcttttatatgggtgcaggtgaggggacttaagccacgtgaaagttcattcgagagagctaaggcatattaatgcacatgtgtgggagttgcatggaacttgcatgaaaggtgcatgaaaggtgcatggtattgcagaatgcgctcgggggtctgcggagaaatccgttaggaaaagatcgtcatccttctgctgcatcaccgttagcttgaaatttagttccagcgctagtcaagggcttcagttcagattctgcaagtatcaggtccatcattactctcttcagcaggcggatcgaatatcccccgaggcacatgggaggtcttattatccgatcgttgatcaccatgccaatcgcttcgaccgaccacaagttgcatcaagcactaactgcctcaagcagatgccgagtcttcatctccgatatttaatcccgttgaatctccgccccctgtcatctccaccgtttaatctggggtggtggcggatgtccaccaattagccggctaaattatccccatcgtcagcacgctagacctgccttggaactagcgctttggtgagaaatctcttggttgtgagtctgataccacattccttgacttccatgttgttctggaggtgtgaaagtataaacaatgccacagatggactaatctccggagagatgaccctcttcaagactggtgcagtgcctaggatcgctagtatcccaaaacttcggggctgccttcatttccagagagttgcggtaccttgcccatcgaacgtacaagtactcctctgttctctccttcctttgctttgtgcggagaccggcttactaaaagccagataacagtatgcatatttgcgcgctgatttttgcggtataagaatatatactgatatgtatacccgaagtatgtcaaaaagaggtatgctatgaagcagcgtattacagtgacagttgacagcgacagctatcagttgctcaaggcatatatgatgtcaatatctccggtctggtaagcacaaccatgcagaatgaagcccgtcgtctgcgtgccgaacgctggaaagcggaaaatcaggaagggatggctgaggtcgcccggtttattgaaatgaacggctcttttgctgacgagaacaggggctggtgaaatgcagtttaaggtttacacctataaaagagagagccgttatcgtctgtttgtggatgtacagagtgatattattgacacgcccgggcgacggatggtgatccccctggccagtgcacgtctgctgtcagataaagtctcccgtgaactttacccggtggtgcatatcggggatgaaagctggcgcatgatgaccaccgatatggccagtgtgccggtttccgttatcggggaagaagtggctgatctcagccaccgcgaaaatgacatcaaaaacgccattaacctgatgttctggggaatataaggtctcgcctccggatcgatgtacacaaccgactgcacccaaacgaacacaaatcttagcagtgccctcgccggatagcttggactgtcctttaccgtcgccagcacaagaagggtatctctgaggtccgtaccgccttttctttaccactggattcgattttcgcagttggaatgatacatctggggactgcgaatggtttacccctcggccgatactatgggtcgtgaagagatggaacattccgaaagtgttttgcggataacattggtggcatcgaaaacagaatgctgaccattgatttcaacacgaacaggaggttgccaagaagcgtacccgccgtgtcgtcaagtcccagcgtgccatcgtcggtgcttccctcgacgtgatcaaggagcgccgctcccagcgccccgaggcccgtgccgccgcccgccagcaggccatcaaggacgccaaggagaagaaggctgccgctgagtccaagaagaaggctgagaaggctaagaacgccgctgctggtgccaagggtgctgctcagcgcatccagagcaagcagggtgctaagggttctgctcccaaggtcgctgccaagtctcgttaaggaatgaataacggttcggcttgggattgggtgcggaaggcaagagtttcatggacgaattttgggaggttactggagctggaatatgtgttttccctaccaccaaaaatgaaatgttccaaaactatcggcgtgcaagacggcctcttacgggtttaacggctctcagataagctctatcaatcgcgccacggatgcatgaatgaagatccagatggccgcgggatatatcgtgctagtgtaattcctacatgatcttgctgttcactccatgcgcatccagatattccaggggtcgactgttaattgatatgcctgggcttgagactccgtagacgcccagtcaatgtgcaattaatacgagggtgctgttatcggcagcaaccttgtacttctccataagatgggggaatgccatggacctgagtgatcaattgacgcaagtctcccataacgcggcggcttgacctaaaatccatataccgccccgttgagcctccgcgctccagagtcctgtcccggaatagggcacaaacctaggctaacctaattcgtcgtccgcgtctgagttcagacaaaagaacttccaagtatcagcagagtacgctgatattgataagtaggcaaacataagaccaataagcaagtagaataaaaaattataaggacactgcctccataaagcgccctcccaagacctcagggacaaaacttctcaagtggcaattcactgcctcaggccgtgtccagtgaagtgacgaagcgacactgttgcctgctgactcagccgctttccgccctgccgaatttgccatctcgcttacaggtcagcactagcgcgattcgcccacagatgctcagcgcaaagtggtgactcagtcaaaccccccctacaagattccacctcgatttttcaacttcccatctcgatccgacaagttctacatccaccgtcaaaatggcctccagcgaagatgtcatcaaggagttcatgcgcttcaaggtccgcatggaaggatccgtcaacggccacgagttcgagattgagggtgagggtgagggccgcccctacgaaggcacccagactgccaagctcaaggtcaccaagggtggtcctctccccttcgcttgggatatcctgtctcctcagttccagtacggctccaaggtctacgtcaagcaccccgccgacatccccgactacaagaagctttctttccccgagggtttcaagtgggagcgtgtcatgaacttcgaggatggtggtgttgtgaccgttactcaggacagcagcttgcaggatggctctttcatctacaaggtcaagttcattggtgtcaacttcccctccgacggccctgtcatgcagaagaagaccatgggctgggaagcgtcgactgagcgtctgtacccccgtgacggtgttctcaagggtgagatccacaaggctctcaagctcaaggacggtggtcactaccttgttgagttcaagtccatctacatggccaagaagcctgtgcagctgcccggatactactacgtggactccaagcttgacatcacctcccacaacgaagactacaccattgttgagcagtacgagcgtgctgagggccgccaccacctcttcctgacccacggaatggatgagctgtacaagtcgaaactataaataaatggtttgcgttgcgattgactgaaacgaaaaaaagcgaaaatgattctgggaatgaattgataaagcgcgggctctgcggtacggttacggttgcggtcgcggacgaatggactgggctgagctgggctggaggaagtccatcgaacaaggacaaggggtggaatatggcacgggtcgattttgttatacataccctaccatccatctatccatttaaataccaaatgagttgttgaatggattcgcggtcttctcggtttatttttgcttgcttgcgtgcttaagggatagtgtgcctcacgctttccggcatcttccagaccacagtatatccatccgcctcctgttgaagcttattttttgtatactgttttgtgatagcacgaagtttttccacggtatcttgttaaaaatatatatttgtggcgggcttacctacatcaaattaataagagactaattataaactaaacacacaagcaagctactttagggtaaaagtttataaatgcttttgacgtataaacgttgcttgtatttattattacaattaaaggtggatagaaaacctagagactagttagaaactaatctcaggtttgcgttaaactaaatcagagcccgagaggttaacagaacctagaaggggactagatatccgggtagggaaacaaaaaaaaaaaacaagacagccacatattagggagactagttagaagctagttccaggactaggaaaataaaagacaatgataccacagtctagttgacaactagatagattctagattgaggccaaagtctctgagatccaggttagttgcaactaatactagttagtatctagtctcctataactctgaagctagaataacttactactattatcctcaccactgttcagctgcgcaaacggagtgattgcaaggtgttcagagactagttattgactagtcagtgactagcaataactaacaaggtattaacctaccatgtctgccatcaccctgcacttcctcgggctcagcagccttttcctcctcattttcatgctcattttccttgtttaagactgtgactagtcaaagactagtccagaaccacaaaggagaaatgtcttaccactttcttcattgcttgtctcttttgcattatccatgtctgcaactagttagagtctagttagtgactagtccgacgaggacttgcttgtctccggattgttggaggaactctccagggcctcaagatccacaacagagccttctagaagactggtcaataactagttggtctttgtctgagtctgacttacgaggttgcatactcgctccctttgcctcgtcaatcgatgagaaaaagcgccaaaactcgcaatatggctttgaaccacacggtgctgagactagttagaatctagtcccaaactagcttggatagcttacctttgccctttgcgttgcgacaggtcttgcagggtatggttcctttctcaccagctgatttagctgccttgctaccctcacggcggatctgcataaagagtggctagaggttataaattagcactgatcctaggtacggggctgaatgtaacttgcctttcctttctcatcgcgcggcaagacaggcttgctcaaattcctaccagtcacaggggtatgcacggcgtacggaccacttgaactagtcacagattagttagcaactagtctgcattgaatggctgtacttacgggccctcgccattgtcctgatcatttccagcttcaccctcgttgctgcaaagtagttagtgactagtcaaggactagttgaaatgggagaagaaactcacgaattctcgacacccttagtattgtggtccttggacttggtgctgctatatattagctaatacactagttagactcacagaaacttacgcagctcgcttgcgcttcttggtaggagtcggggttgggagaacagtgccttcaaacaagccttcataccatgctacttgactagtcagggactagtcaccaagtaatctagataggacttgcctttggcctccatcagttccttcatagtgggaggtccattgtgcaatgtaaactccatgccgtgggagttcttgtccttcaagtgcttgaccaatatgtttctgttggcagagggaacctgtcaactagttaataactagtcagaaactagtatagcagtagactcactgtacgcttgaggcatcccttcactcggcagtagacttcatatggatggatatcaggcacgccattgtcgtcctgtggactagtcagtaactaggcttaaagctagtcgggtcggcttactatcttgaaatccggcagcgtaagctccccgtccttaactgcctcgagatagtgacagtactctggggactttcggagatcgttatcgcgaatgctcggcatactaatcgttgactagtcttggactagtcccgagcaaaaaggattggaggaggaggaggaaggtgagagtgagacaaagagcgaaataagagcttcaaaggctatctctaagcagtatgaaggttaagtatctagttcttgactagatttaaaagagatttcgactagttatgtacctggagtttggatataggaatgtgttgtggtaacgaaatgtaagggggaggaaagaaaaagtcggtcaagaggtaactctaagtcggccattcctttttgggaggcgctaaccataaacggcatggtcgacttagagttagctcagggaatttagggagttatctgcgaccaccgaggaacggcggaatgccaaagaatcccgatggagctctagctggcggttgacaaccccaccttttggcgtttctgcggcgttgcaggcgggactggatacttcgtagaaccagaaaggcaaggcagaacgcgctcagcaagagtgttggaagtgatagcatgatgtgccttgttaactaggtcaaaatctgcagtatgcttgatgttatccaaagtgtgagagaggaaggtccaaacatacacgattgggagagggcctaggtataagagtttttgagtagaacgcatgtgagcccagccatctcgaggagattaaacacgggccggcatttgatggctatgttagtaccccaatggaaagcctgagagtccagtggtcgcagataactccctaaattccctgagctaactctaagtcgaccatgccgtttatggttagcgcctcccaaaaaggaatggccgacttagagttacctcttgaccgactttttctttcctcccccttacatttcgttaccacaacacattcctatatccaaactccaggtacataactagtcgaaatctcttttaaatctagtcaagaactagatacttaaccttcatactgcttagagatagcctttgaagctcttatttcgctctttgtctcactctcaccttcctcctcctcctccaatcctttttgctcgggactagtccaagactagtcaacgattagtatgccgagcattcgcgataacgatctccgaaagtccccagagtactgtcactatctcgaggcagttaaggacggggagcttacgctgccggatttcaagatagtaagccgacccgactagctttaagcctagttactgactagtccacaggacgacaatggcgtgcctgatatccatccatatgaagtctactgccgagtgaagggatgcctcaagcgtacagtgagtctactgctatactagtttctgactagttattaactagttgacaggttccctctgccaacagaaacatattggtcaagcacttgaaggacaagaactcccacggcatggagtttacattgcacaatggacctcccactatgaaggaactgatggaggccaaaggcaagtcctatctagattacttggtgactagtccctgactagtcaagtagcatggtatgaaggcttgtttgaaggcactgttctcccaaccccgactcctaccaagaagcgcaagcgagctgcgtaagtttctgtgagtctaactagtgtattagctaatatatagcagcaccaagtccaaggaccacaatactaagggtgtcgagaattcgtgagtttcttctcccatttcaactagtccttgactagtcactaactactttgcagcaacgagggtgaagctggaaatgatcaggacaatggcgagggcccgtaagtacagccattcaatgcagactagttgctaactaatctgtgactagttcaagtggtccgtacgccgtgcatacccctgtgactggtaggaatttgagcaagcctgtcttgccgcgcgatgagaaaggaaaggcaagttacattcagccccgtacctaggatcagtgctaatttataacctctagccactctttatgcagatccgccgtgagggtagcaaggcagctaaatcagctggtgagaaaggaaccataccctgcaagacctgtcgcaacgcaaagggcaaaggtaagctatccaagctagtttgggactagattctaactagtctcagcaccgtgtggttcaaagccatattgcgagttttggcgctttttctcatcgattgacgaggcaaagggagcgagtatgcaacctcgtaagtcagactcagacaaagaccaactagttattgaccagtcttctagaaggctctgttgtggatcttgaggccctggagagttcctccaacaatccggagacaagcaagtcctcgtcggactagtcactaactagactctaactagttgcagacatggataatgcaaaagagacaagcaatgaagaaagtggtaagacatttctcctttgtggttctggactagtctttgactagtcacagtcttaaacaaggaaaatgagcatgaaaatgaggaggaaaaggctgctgagcccgaggaagtgcagggtgatggcagacatggtaggttaataccttgttagttattgctagtcactgactagtcaataactagtctctgaacaccttgcaatcactccgtttgcgcagctgaacagtggtgaggataatagtagtaagttattctagcttcagagttataggagactagatactaactagtattagttgcaactaacctggatctcagagactttggcctcaatctagaatctatctagttgtcaactagactgtggtatcattgtcttttattttcctagtcctggaactagcttctaactagtctccctaatatgtggctgtcttgttttttttttttgtttccctacccggatatctagtccccttctaggttctgttaacctctcgggctctgatttagtttaacgcaaacctgagattagtttctaactagtctctaggttttctatccacctttaattgtaataataaatacaagcaacgtttatacgtcaaaagcatttataaacttttaccctaaagtagcttgcttgtgtgtttagtttataattagtctcttattaatttgatgtaggtaagcccgccacaaatatatatttttaacaagataccgtggaaaaacttcgtgctatcacaaaacagtatacaaaaaataagctatcgaattcctgcagagatcatcctgtcttcagtcttaagacttctctcctatatcacccgcacttaccctagagtgccgcttaggtgctaagggcacattgagtattggccgtgtagaatatatagcttaagtacggccaagcagacgggaagccctgttctccacaccctatggtcgtatatatcaggcttctaccgggaaacgattaagagtgtataatggactgaaaatcaatatgaacgggacaatgctcaagttaaattagttaggcatcctaatctctactaaatgttctatctagagatcggggtactataggcccgtacgttaatcactctacgcttctctcccttaggtatagtgtaggtaggggctagacatttatatgagtcagatggtacaaacggtaggcagtgcgggcgaagaagtgaagacggagtcggttgaagctacatacaaaagatgcattggctcgtcatgaagagcctcccgggtttattcctttgccctcggacgagtgctggggcgtcggtttccactatcggcgagtacttctacacagccatcggtccagacggccgcgcttctgcgggcgatttgtgtacgcccgacagtcccggctccggatcggacgattgcgtcgcatcgaccctgcgcccaagctgcatcatcgaaattgccgtcaaccaagctctgatagagttggtcaagaccaatgcggagcatatacgcccggagccgcggcgatcctgcaagctccggatgcctccgctcgaagtagcgcgtctgctgctccatacaagccaaccacggcctccagaagaagatgttggcgacctcgtattgggaatccccgaacatcgcctcgctccagtcaatgaccgctgttatgcggccattgtccgtcaggacattgttggagccgaaatccgcgtgcacgaggtgccggacttcggggcagtcctcggcccaaagcatcagctcatcgagagcctgcgcgacggacgcactgacggtgtcgtccatcacagtttgccagtgatacacatggggatcagcaatcgcgcatatgaaatcacgccatgtagtgtattgaccgattccttgcggtccgaatgggccgaacccgctcgtctggctaagatcggccgcagcgatcgcatccatggcctccgcgaccggctgcagaacagcgggcagttcggtttcaggcaggtcttgcaacgtgacaccctgtgcacggcgggagatgcaataggtcaggctctcgctgaattccccaatgtcaagcacttccggaatcgggagcgcggccgatgcaaagtgccgataaacataacgatctttgtagaaaccatcggcgcagctatttacccgcaggacatatccacgccctcctacatcgaagctgaaagcacgagattcttcgccctccgagagctgcatcaggtcggagacgctgtcgaacttttcgatcagaaacttctcgacagacgtcgcggtgagttcaggcattttgacggtgggatcctgtgatgtctgctcaagcggggtagctgttagtcaagctgcgatgaagtgggaaagctcgaactgaaaggttcaaaggaataagggatgggaaggatggagtatggatgtagcaaagtacttacttaggggaaataaaggttcttggatgggaagatgaatatactgaagatgggaaaagaaagagaaaagaaaagagcagctggtggggagagcaggaaaatatggcaacaaatgttggactgacgcaacgaccttgtcaaccccgccgacacaccgggcggacagacggggcaaagctgcctaccagggactgagggacctcagcaggtcgagtgcagagcaccggatgggtcgactgccagcttgtgttcccggtctgcgccgctggccagctcctgagcggcctttccggtttcatacaccgggcaaagcaggagaggcacgatatttggacgccctacagatgccggatgggccaattagggagcttacgcgccgggtactcgctctacctacttcggagaaggtactatctcgtgaatcttttaccagatcggaagcaattggacttctgtacctaggttaatggcatgctatttcgccgacggctatacacccctggcttcacattctccttcgcttactgccggtgattcgatgaagctccatattctccgatgatgcaatagattcttggtcaacgaggggcacaccagcctttccacttcggggcggaggggcggccggtcccggattaataatcatccactgcacctcagagccgccagagctgtctggcgcagtggcgcttattactcagcccttctctctgcgtccgtccgtctctccgcatgccagaaagagtcaccggtcactgtacagagcggccgccaccgcggtggagctccaattcgccctatagtgagtcgtattacgcgcgctcactggccgtcgttttacaacgtcgtgactgggaaaaccctggcgttacccaacttaatcgccttgcagcacatccccctttcgccagctggcgtaatagcgaagaggcccgcaccgatcgcccttcccaacagttgcgcagcctgaatggcgaatgggacgcgccctgtagcggcgcattaagcgcggcgggtgtggtggttacgcgcagcgtgaccgctacacttgccagcgccctagcgcccgctcctttcgctttcttcccttcctttctcgccacgttcgccggctttccccgtcaagctctaaatcgggggctccctttagggttccgatttagtgctttacggcacctcgaccccaaaaaacttgattagggtgatggttcacgtagtgggccatcgccctgatagacggtttttcgccctttgacgttggagtccacgttctttaatagtggactcttgttccaaactggaacaacactcaaccctatctcggtctattcttttgatttataagggattttgccgatttcggcctattggttaaaaaatgagctgatttaacaaaaatttaacgcgaattttaacaaaatattaacgcttacaatttaggtggcacttttcggggaaatgtgcgcggaacccctatttgtttatttttctaaatacattcaaatatgtatccgctcatgagacaataaccctgataaatgcttcaataatattgaaaaaggaagagtatgagtattcaacatttccgtgtcgcccttattcccttttttgcggcattttgccttcctgtttttgctcacccagaaacgctggtgaaagtaaaagatgctgaagatcagttgggtgcacgagtgggttacatcgaactggatctcaacagcggtaagatccttgagagttttcgccccgaagaacgttttccaatgatgagcacttttcgaccgaataaatacctgtgacggaagatcacttcgcagaataaataaatcctggtgtccctgttgataccgggaagccctgggccaacttttggcgaaaatgagacgttgatcggcacgtaagaggttccaactttcaccataatgaaataagatcactaccgggcgtattttttgagttgtcgagattttcaggagctaaggaagctaaaatggagaaaaaaatcactggatataccaccgttgatatatcccaatggcatcgtaaagaacattttgaggcatttcagtcagttgctcaatgtacctataaccagaccgttcagctggatattacggcctttttaaagaccgtaaagaaaaataagcacaagttttatccggcctttattcacattcttgcccgcctgatgaatgctcatccggaattacgtatggcaatgaaagacggtgagctggtgatatgggatagtgttcacccttgttacaccgttttccatgagcaaactgaaacgttttcatcgctctggagtgaataccacgacgatttccggcagtttctacacatatattcgcaagatgtggcgtgttacggtgaaaacctggcctatttccctaaagggtttattgagaatatgtttttcgtctcagccaatccctgggtgagtttcaccagttttgatttaaacgtggccaatatggacaacttcttcgcccccgttttcaccatgggcaaatattatacgcaaggcgacaaggtgctgatgccgctggcgattcaggttcatcatgccgtttgtgatggcttccatgtcggcagaatgcttaatgaattacaacagtactgcgatgagtggcagggcggggcgtaatttttttaaggcagttattggtgcccttaaacgcctggttgctacgcctgaataagtgataataagcggatgaatggcagaaattcgaaagcaaattcgacccggtcgtcggttcagggcagggtcgttaaatagccgcttatgtctattgctggtttaccggtttattgactaccggaagcagtgtgaccgtgtgcttctcaaatgcctgaggccagtttgctcaggctctccccgtggaggtaataattgacgatatgatcctttttttctgatcaaaaaggatctaggtgaagatcctttttgataatctcatgaccaaaatcccttaacgtgagttttcgttccactgagcgtcagaccccgtagaaaagatcaaaggatcttcttgagatcctttttttctgcgcgtaatctgctgcttgcaaacaaaaaaaccaccgctaccagcggtggtttgtttgccggatcaagagctaccaactctttttccgaaggtaactggcttcagcagagcgcagataccaaatactgttcttctagtgtagccgtagttaggccaccacttcaagaactctgtagcaccgcctacatacctcgctctgctaatcctgttaccagtggctgctgccagtggcgataagtcgtgtcttaccgggttggactcaagacgatagttaccggataaggcgcagcggtcgggctgaacggggggttcgtgcacacagcccagcttggagcgaacgacctacaccgaactgagatacctacagcgtgagctatgagaaagcgccacgcttcccgaagggagaaaggcggacaggtatccggtaagcggcagggtcggaacaggagagcgcacgagggagcttccagggggaaacgcctggtatctttatagtcctgtcgggtttcgccacctctgacttgagcgtcgatttttgtgatgctcgtcaggggggcggagcctatggaaaaacgccagcaacgcggcctttttacggttcctggccttttgctggccttttgctcacatgttctttcctgcgttatcccctgattctgtggataaccgtattaccgcctttgagtgagctgataccgctcgccgcagccgaacgaccgagcgcagcgagtcagtgagcgaggaagcggaagagcgcccaatacgcaaaccgcctctccccgcgcgttggccgattcattaatgcagctggcacgacaggtttcccgactggaaagcgggcagtgagcgcaacgcaattaatgtgagttagctcactcattaggcaccccaggctttacactttatgctcccggctcgtatgttgtgtggaattgtgagcggataacaatttcacacaggaaacagctatgaccatgattacgccaagcgcgcaattaaccctcactaaagggaacaaaagctg

SEQ ID NO: 69 - DNA, 262 bp, Artificial Sequence
  Nucleotide sequence of ordered gBlock with T7 gRNA cassette - T7.pro WT sgRNA fwnA
gggggtctcggtgctaatacgactcactatagtcagatatattcagtcactggttttagagctagaaatagcaagttaaaataaggctagtccgttatcaacttgaaaaagtggcaccgagtcggtgcttttggccggcatggtcccagcctcctcgctggcgccggctgggcaacatgcttcggcatggcgaatgggacaaaaaatcaaactggctcaccttcgggtgggcctttttgcgtttatacctcggagaccgggg

SEQ ID NO: 70 - DNA, 267 bp, Artificial Sequence
  Nucleotide sequence of ordered gBlock with T7 gRNA cassette - T7.pro strong sgRNA fwnA
gggggtctcggtgctaatacgactcactataggggaatcagatatattcagtcactggttttagagctagaaatagcaagttaaaataaggctagtccgttatcaacttgaaaaagtggcaccgagtcggtgcttttggccggcatggtcccagcctcctcgctggcgccggctgggcaacatgcttcggcatggcgaatgggacaaaaaatcaaactggctcaccttcgggtgggcctttttgcgtttatacctcggagaccgggg

SEQ ID NO: 71 - DNA, 19153 bp, Artificial Sequence
  Nucleotide sequence of BG-AMA18 (Cas9/hygB/T7 wt sgRNA fwnA) - Golden Gate product BG-AMA17 with gBlock T7.pro WT sgRNA fwnA
ggtaccgaggttcatggtatgggcacgaatgtcaaaaattttcaggctcaaacgggtatgtattcagtatctatctccgtgtacgacggctaattgagcccagctgcatttcgaactcttctcccagcgcattttgtgtgggagttcttcgatgctgaccatgactgcgaggctgctgagggagtgcgcggtatctaccccggcccgtatctggcttctacaaggagtgaaactagtttatactttgtagttcggaatccaatgctattaaccgtttttactttttcttttgttcgagctaagcgcttgtttaaaccttgcgcttcttcttgggatcggcacgagagtcaccaccgagctgagacaggtcgatacgagtctcgtacagaccggtaatcgactggtggatcagagtcgcatcaagcacttccttggtggaggtgtaacgcttgcggtcgatggtggtgtcaaagtacttgaaagcagcaggagcacccaggttggtgagggtgaacaggtggatgatgttctccgcctgctcgcggatgggcttgtcacggtgcttgttgtaggcagagaggaccttgtcaaggttggcatcggccaggatgacacgcttgctgaactcggagatctgctcgatgatctcatccaggtagtgcttgtgctgctcgacaaagagctgcttctgctcgttgtcctcgggagagcccttgagcttctcgtagtgggaggccaggtagaggaagttgacgtacttggaggggagggcaagctcgttacccttctggagctcaccggcggaagcaagcatgcgcttacggccgttctccagctcgaacagagagtacttggggagcttgatgatgaggtccttcttgacctctttgtaacccttggcctccaggaagtcgatagggttcttctcgaagctgctgcgttccatgatggtgataccgaggagttccttcacactcttcagcttcttgctcttgcccttctcgaccttggcgacaaccaagacggagtaggcaacggtaggcgaatcgaatccaccgtacttcttggggtcccaatccttcttgcgagcgatcagcttgtcggagttgcgcttgggaagaatcgactccttggagaaaccaccagtctgcacctcggtcttcttgacaatgttgacctggggcatagaaaggaccttgcggacggtagcgaagtcacggcccttgtcccagacgatctcaccggtttcgccgttagtctcaatcaagggacgcttgcgaatctcgccgttggccaatgttatttcggtcttgaagaagttcatgatgttgctgtagaagaagtacttggcagtggcctttccgatctcctgctcggacttagcgatcatcttgcgcacgtcgtacaccttgtagtcaccgtagacgaactcggactcgagcttgggatacttcttaatcaaagcagtaccgacgacggcgttgaggtaggcatcgtgagcgtggtggtagttgttgatctcgcggaccttgtagaactggaagtctttcctaaagtcactgaccagcttgctctttaaggtgatgaccttgacctcacggatgagcttgtcgttctcgtcgtacttggtgttcatgcgagagtccaggatctgggcaacgtgcttagtgatctgacgggtttcaaccaattgacgcttgatgaaaccggccttgtcgagctcggagagtccgccacgctcggccttggtaaggttgtcgaacttgcgctgagtgatgagcttagcgttgagcaattgtctccagtagttcttcatcttcttaacaacctcttccgaggggacgttatcgctcttgccacgattcttgtcggaacgggtgagcaccttgttgtcaatgctgtcatccttgaggaaggactgggggacgatgtggtcaacatcgtagtcggagaggcggttgatatccagctcctggtcgacgtacatgtcacgtccgttctgcaagtagtagaggtagagcttctcattctgcagctgggtgttctcgacggggtgttccttgagaatctgggaaccgagctccttgatgccttcctcgatacgcttcatgcgctcacggctgttcttctgacccttctgagtggtctggttctcacgagccatttcgatgacgatgttctcgggcttgtgacgacccatgaccttcacaagctcgtcaacaaccttcacagtctgcaggatacccttcttgatagcgggggaaccagccaggttggcaatgtgttcgtgtagcgagtcaccctggccggagacttgggccttctggatgtcctctttgaaggtcagagagtcgtcgtggatgagctgcatgaagttgcggttggcgaagccgtcggacttcaggaagtcaaggatggtcttgccagactgcttatcacggataccgttaatcaacttgcgagagaggcgaccccagccagtgtaacggcggcgcttcaactgcttcatgaccttgtcgtcgaagaggtgagcgtaggtcttcagacgttcttcgatcatctcacggtcctcgaagagggtgagggtaagaacaatgtcctcaagaatgtcttcgttctcctcgttgtcaaggaagtccttgtccttgatgatcttgagcagatcgtggtaggtgccgagagaagcgttgaagcggtcctcaacaccggagatctcaacggagtcaaagcactcgatcttcttgaagtagtcttccttgagctgcttgacggtcaccttgcggttagtcttgaacagcaggtcgacaatggccttcttctgttcgccggagaggaaagcaggcttgcgcatgccctcggtcacgtacttgaccttggtcagctcgttgtagacagtgaagtactcgtacaagagggagtgcttgggcaggactttctcgttgggcaggttcttgtcgaagttggtcatacgctcaatgaagctctgagcggaggcacccttgtcgacgacttcctcgaagttccagggggtgatggtttcctcggacttgcgggtcatccaggcgaagcgggagttaccgcgagccagaggaccgacgtagtaggggatacggaaggtcaggatcttctcaatcttctcacggttgtccttcaagaaagggtagaagtcttcctggcgacgaaggatggcgtgcaattcacccaggtggatctggtgggggatgctgccgttgtcgaaagtacgctgcttgcgcagaaggtcctcacggttcagcttaacaagaagctcctcagtgccatccatcttctcgaggataggcttaatgaacttgtagaattcttcctgggaagcaccaccgtcgatgtaaccggcgtagccgttcttggactggtcgaagaagatctccttgtacttttcggggagctgctggcggaccagagccttgagtagggtgaggtcctggtggtgctcatcgtatctcttgatcatagaggcggagagaggggccttggtgatctcagtgttgacacggaggatatctgacaggagaatggcatcggagaggttcttggcagctaggaagaggtcggcgtactgatctcctatctgggcgagaaggttatcaaggtcgtcgtcgtaggtatccttggaaagttgtaacttagcatcctcagcaagatcgaagttgctcttgaagttgggagtcagtccgagggacagggcaataaggttgccgaaaagaccgttcttcttctcaccagggagctgggcaatcaagttctcaagacggcgggacttgctcaggcgagcggagaggatggccttggcatccacgccagacgcgttgatggggttttcctcgaaaagctggttgtaggtctgaacgagctggatgaagagtttatcaacatcggagttgtcggggttgaggtcaccctcgatcaggaagtgaccacggaacttgatcatgtgcgccagagccaggtaaatgaggcggaggtcagccttgtcggtgctgtcgacgagctttttgcgtaggtggtagatggtggggtacttctcgtggtaagcgacctcatcgacaatgttaccgaagatagggtgacgctcgtgcttcttgtcttcttcaacaaggaacgactcctccagacggtggaagaaagagtcatcaaccttggccatctcgttggagaaaatctcctggaggtagcagatacggttcttgcggcgagtgtaacgacggcgagcggtacgcttcagacgggtggcctcagcagtctcaccggagtcgaagagaagcgcaccaatgaggttcttcttgatggagtgacgatcggtgtttcccaggaccttgaatttcttgctaggaaccttgtactcgtcggtgatgacagcccagccaacggagttggtgccaatgtccagaccgatgctatacttcttgtccattttgacggtggaaggtgagttggggttggtgtcatcgtgggggaagaacttggcttttatatgggtgcaggtgaggggacttaagccacgtgaaagttcattcgagagagctaaggcatattaatgcacatgtgtgggagttgcatggaacttgcatgaaaggtgcatgaaaggtgcatggtattgcagaatgcgctcgggggtctgcggagaaatccgttaggaaaagatcgtcatccttctgctgcatcaccgttagcttgaaatttagttccagcgctagtcaagggcttcagttcagattctgcaagtatcaggtccatcattactctcttcagcaggcggatcgaatatcccccgaggcacatgggaggtcttattatccgatcgttgatcaccatgccaatcgcttcgaccgaccacaagttgcatcaagcactaactgcctcaagcagatgccgagtcttcatctccgatatttaatcccgttgaatctccgccccctgtcatctccaccgtttaatctggggtggtggcggatgtccaccaattagccggctaaattatccccatcgtcagcacgctagacctgccttggaactagcgctttggtgagaaatctcttggttgtgagtctgataccacattccttgacttccatgttgttctggaggtgtgaaagtataaacaatgccacagatggactaatctccggagagatgaccctcttcaagactggtgcagtgcctaggatcgctagtatcccaaaacttcggggctgccttcatttccagagagttgcggtaccttgcccatcgaacgtacaagtactcctctgttctctccttcctttgctttgtgctaatacgactcactatagtcagatatattcagtcactggttttagagctagaaatagcaagttaaaataaggctagtccgttatcaacttgaaaaagtggcaccgagtcggtgcttttggccggcatggtcccagcctcctcgctggcgccggctgggcaacatgcttcggcatggcgaatgggacaaaaaatcaaactggctcaccttcgggtgggcctttttgcgtttatacctccggatcgatgtacacaaccgactgcacccaaacgaacacaaatcttagcagtgccctcgccggatagcttggactgtcctttaccgtcgccagcacaagaagggtatctctgaggtccgtaccgccttttctttaccactggattcgattttcgcagttggaatgatacatctggggactgcgaatggtttacccctcggccgatactatgggtcgtgaagagatggaacattccgaaagtgttttgcggataacattggtggcatcgaaaacagaatgctgaccattgatttcaacacgaacaggaggttgccaagaagcgtacccgccgtgtcgtcaagtcccagcgtgccatcgtcggtgcttccctcgacgtgatcaaggagcgccgctcccagcgccccgaggcccgtgccgccgcccgccagcaggccatcaaggacgccaaggagaagaaggctgccgctgagtccaagaagaaggctgagaaggctaagaacgccgctgctggtgccaagggtgctgctcagcgcatccagagcaagcagggtgctaagggttctgctcccaaggtcgctgccaagtctcgttaaggaatgaataacggttcggcttgggattgggtgcggaaggcaagagtttcatggacgaattttgggaggttactggagctggaatatgtgttttccctaccaccaaaaatgaaatgttccaaaactatcggcgtgcaagacggcctcttacgggtttaacggctctcagataagctctatcaatcgcgccacggatgcatgaatgaagatccagatggccgcgggatatatcgtgctagtgtaattcctacatgatcttgctgttcactccatgcgcatccagatattccaggggtcgactgttaattgatatgcctgggcttgagactccgtagacgcccagtcaatgtgcaattaatacgagggtgctgttatcggcagcaaccttgtacttctccataagatgggggaatgccatggacctgagtgatcaattgacgcaagtctcccataacgcggcggcttgacctaaaatccatataccgccccgttgagcctccgcgctccagagtcctgtcccggaatagggcacaaacctaggctaacctaattcgtcgtccgcgtctgagttcagacaaaagaacttccaagtatcagcagagtacgctgatattgataagtaggcaaacataagaccaataagcaagtagaataaaaaattataaggacactgcctccataaagcgccctcccaagacctcagggacaaaacttctcaagtggcaattcactgcctcaggccgtgtccagtgaagtgacgaagcgacactgttgcctgctgactcagccgctttccgccctgccgaatttgccatctcgcttacaggtcagcactagcgcgattcgcccacagatgctcagcgcaaagtggtgactcagtcaaaccccccctacaagattccacctcgatttttcaacttcccatctcgatccgacaagttctacatccaccgtcaaaatggcctccagcgaagatgtcatcaaggagttcatgcgcttcaaggtccgcatggaaggatccgtcaacggccacgagttcgagattgagggtgagggtgagggccgcccctacgaaggcacccagactgccaagctcaaggtcaccaagggtggtcctctccccttcgcttgggatatcctgtctcctcagttccagtacggctccaaggtctacgtcaagcaccccgccgacatccccgactacaagaagctttctttccccgagggtttcaagtgggagcgtgtcatgaacttcgaggatggtggtgttgtgaccgttactcaggacagcagcttgcaggatggctctttcatctacaaggtcaagttcattggtgtcaacttcccctccgacggccctgtcatgcagaagaagaccatgggctgggaagcgtcgactgagcgtctgtacccccgtgacggtgttctcaagggtgagatccacaaggctctcaagctcaaggacggtggtcactaccttgttgagttcaagtccatctacatggccaagaagcctgtgcagctgcccggatactactacgtggactccaagcttgacatcacctcccacaacgaagactacaccattgttgagcagtacgagcgtgctgagggccgccaccacctcttcctgacccacggaatggatgagctgtacaagtcgaaactataaataaatggtttgcgttgcgattgactgaaacgaaaaaaagcgaaaatgattctgggaatgaattgataaagcgcgggctctgcggtacggttacggttgcggtcgcggacgaatggactgggctgagctgggctggaggaagtccatcgaacaaggacaaggggtggaatatggcacgggtcgattttgttatacataccctaccatccatctatccatttaaataccaaatgagttgttgaatggattcgcggtcttctcggtttatttttgcttgcttgcgtgcttaagggatagtgtgcctcacgctttccggcatcttccagaccacagtatatccatccgcctcctgttgaagcttattttttgtatactgttttgtgatagcacgaagtttttccacggtatcttgttaaaaatatatatttgtggcgggcttacctacatcaaattaataagagactaattataaactaaacacacaagcaagctactttagggtaaaagtttataaatgcttttgacgtataaacgttgcttgtatttattattacaattaaaggtggatagaaaacctagagactagttagaaactaatctcaggtttgcgttaaactaaatcagagcccgagaggttaacagaacctagaaggggactagatatccgggtagggaaacaaaaaaaaaaaacaagacagccacatattagggagactagttagaagctagttccaggactaggaaaataaaagacaatgataccacagtctagttgacaactagatagattctagattgaggccaaagtctctgagatccaggttagttgcaactaatactagttagtatctagtctcctataactctgaagctagaataacttactactattatcctcaccactgttcagctgcgcaaacggagtgattgcaaggtgttcagagactagttattgactagtcagtgactagcaataactaacaaggtattaacctaccatgtctgccatcaccctgcacttcctcgggctcagcagccttttcctcctcattttcatgctcattttccttgtttaagactgtgactagtcaaagactagtccagaaccacaaaggagaaatgtcttaccactttcttcattgcttgtctcttttgcattatccatgtctgcaactagttagagtctagttagtgactagtccgacgaggacttgcttgtctccggattgttggaggaactctccagggcctcaagatccacaacagagccttctagaagactggtcaataactagttggtctttgtctgagtctgacttacgaggttgcatactcgctccctttgcctcgtcaatcgatgagaaaaagcgccaaaactcgcaatatggctttgaaccacacggtgctgagactagttagaatctagtcccaaactagcttggatagcttacctttgccctttgcgttgcgacaggtcttgcagggtatggttcctttctcaccagctgatttagctgccttgctaccctcacggcggatctgcataaagagtggctagaggttataaattagcactgatcctaggtacggggctgaatgtaacttgcctttcctttctcatcgcgcggcaagacaggcttgctcaaattcctaccagtcacaggggtatgcacggcgtacggaccacttgaactagtcacagattagttagcaactagtctgcattgaatggctgtacttacgggccctcgccattgtcctgatcatttccagcttcaccctcgttgctgcaaagtagttagtgactagtcaaggactagttgaaatgggagaagaaactcacgaattctcgacacccttagtattgtggtccttggacttggtgctgctatatattagctaatacactagttagactcacagaaacttacgcagctcgcttgcgcttcttggtaggagtcggggttgggagaacagtgccttcaaacaagccttcataccatgctacttgactagtcagggactagtcaccaagtaatctagataggacttgcctttggcctccatcagttccttcatagtgggaggtccattgtgcaatgtaaactccatgccgtgggagttcttgtccttcaagtgcttgaccaatatgtttctgttggcagagggaacctgtcaactagttaataactagtcagaaactagtatagcagtagactcactgtacgcttgaggcatcccttcactcggcagtagacttcatatggatggatatcaggcacgccattgtcgtcctgtggactagtcagtaactaggcttaaagctagtcgggtcggcttactatcttgaaatccggcagcgtaagctccccgtccttaactgcctcgagatagtgacagtactctggggactttcggagatcgttatcgcgaatgctcggcatactaatcgttgactagtcttggactagtcccgagcaaaaaggattggaggaggaggaggaaggtgagagtgagacaaagagcgaaataagagcttcaaaggctatctctaagcagtatgaaggttaagtatctagttcttgactagatttaaaagagatttcgactagttatgtacctggagtttggatataggaatgtgttgtggtaacgaaatgtaagggggaggaaagaaaaagtcggtcaagaggtaactctaagtcggccattcctttttgggaggcgctaaccataaacggcatggtcgacttagagttagctcagggaatttagggagttatctgcgaccaccgaggaacggcggaatgccaaagaatcccgatggagctctagctggcggttgacaaccccaccttttggcgtttctgcggcgttgcaggcgggactggatacttcgtagaaccagaaaggcaaggcagaacgcgctcagcaagagtgttggaagtgatagcatgatgtgccttgttaactaggtcaaaatctgcagtatgcttgatgttatccaaagtgtgagagaggaaggtccaaacatacacgattgggagagggcctaggtataagagtttttgagtagaacgcatgtgagcccagccatctcgaggagattaaacacgggccggcatttgatggctatgttagtaccccaatggaaagcctgagagtccagtggtcgcagataactccctaaattccctgagctaactctaagtcgaccatgccgtttatggttagcgcctcccaaaaaggaatggccgacttagagttacctcttgaccgactttttctttcctcccccttacatttcgttaccacaacacattcctatatccaaactccaggtacataactagtcgaaatctcttttaaatctagtcaagaactagatacttaaccttcatactgcttagagatagcctttgaagctcttatttcgctctttgtctcactctcaccttcctcctcctcctccaatcctttttgctcgggactagtccaagactagtcaacgattagtatgccgagcattcgcgataacgatctccgaaagtccccagagtactgtcactatctcgaggcagttaaggacggggagcttacgctgccggatttcaagatagtaagccgacccgactagctttaagcctagttactgactagtccacaggacgacaatggcgtgcctgatatccatccatatgaagtctactgccgagtgaagggatgcctcaagcgtacagtgagtctactgctatactagtttctgactagttattaactagttgacaggttccctctgccaacagaaacatattggtcaagcacttgaaggacaagaactcccacggcatggagtttacattgcacaatggacctcccactatgaaggaactgatggaggccaaaggcaagtcctatctagattacttggtgactagtccctgactagtcaagtagcatggtatgaaggcttgtttgaaggcactgttctcccaaccccgactcctaccaagaagcgcaagcgagctgcgtaagtttctgtgagtctaactagtgtattagctaatatatagcagcaccaagtccaaggaccacaatactaagggtgtcgagaattcgtgagtttcttctcccatttcaactagtccttgactagtcactaactactttgcagcaacgagggtgaagctggaaatgatcaggacaatggcgagggcccgtaagtacagccattcaatgcagactagttgctaactaatctgtgactagttcaagtggtccgtacgccgtgcatacccctgtgactggtaggaatttgagcaagcctgtcttgccgcgcgatgagaaaggaaaggcaagttacattcagccccgtacctaggatcagtgctaatttataacctctagccactctttatgcagatccgccgtgagggtagcaaggcagctaaatcagctggtgagaaaggaaccataccctgcaagacctgtcgcaacgcaaagggcaaaggtaagctatccaagctagtttgggactagattctaactagtctcagcaccgtgtggttcaaagccatattgcgagttttggcgctttttctcatcgattgacgaggcaaagggagcgagtatgcaacctcgtaagtcagactcagacaaagaccaactagttattgaccagtcttctagaaggctctgttgtggatcttgaggccctggagagttcctccaacaatccggagacaagcaagtcctcgtcggactagtcactaactagactctaactagttgcagacatggataatgcaaaagagacaagcaatgaagaaagtggtaagacatttctcctttgtggttctggactagtctttgactagtcacagtcttaaacaaggaaaatgagcatgaaaatgaggaggaaaaggctgctgagcccgaggaagtgcagggtgatggcagacatggtaggttaataccttgttagttattgctagtcactgactagtcaataactagtctctgaacaccttgcaatcactccgtttgcgcagctgaacagtggtgaggataatagtagtaagttattctagcttcagagttataggagactagatactaactagtattagttgcaactaacctggatctcagagactttggcctcaatctagaatctatctagttgtcaactagactgtggtatcattgtcttttattttcctagtcctggaactagcttctaactagtctccctaatatgtggctgtcttgttttttttttttgtttccctacccggatatctagtccccttctaggttctgttaacctctcgggctctgatttagtttaacgcaaacctgagattagtttctaactagtctctaggttttctatccacctttaattgtaataataaatacaagcaacgtttatacgtcaaaagcatttataaacttttaccctaaagtagcttgcttgtgtgtttagtttataattagtctcttattaatttgatgtaggtaagcccgccacaaatatatatttttaacaagataccgtggaaaaacttcgtgctatcacaaaacagtatacaaaaaataagctatcgaattcctgcagagatcatcctgtcttcagtcttaagacttctctcctatatcacccgcacttaccctagagtgccgcttaggtgctaagggcacattgagtattggccgtgtagaatatatagcttaagtacggccaagcagacgggaagccctgttctccacaccctatggtcgtatatatcaggcttctaccgggaaacgattaagagtgtataatggactgaaaatcaatatgaacgggacaatgctcaagttaaattagttaggcatcctaatctctactaaatgttctatctagagatcggggtactataggcccgtacgttaatcactctacgcttctctcccttaggtatagtgtaggtaggggctagacatttatatgagtcagatggtacaaacggtaggcagtgcgggcgaagaagtgaagacggagtcggttgaagctacatacaaaagatgcattggctcgtcatgaagagcctcccgggtttattcctttgccctcggacgagtgctggggcgtcggtttccactatcggcgagtacttctacacagccatcggtccagacggccgcgcttctgcgggcgatttgtgtacgcccgacagtcccggctccggatcggacgattgcgtcgcatcgaccctgcgcccaagctgcatcatcgaaattgccgtcaaccaagctctgatagagttggtcaagaccaatgcggagcatatacgcccggagccgcggcgatcctgcaagctccggatgcctccgctcgaagtagcgcgtctgctgctccatacaagccaaccacggcctccagaagaagatgttggcgacctcgtattgggaatccccgaacatcgcctcgctccagtcaatgaccgctgttatgcggccattgtccgtcaggacattgttggagccgaaatccgcgtgcacgaggtgccggacttcggggcagtcctcggcccaaagcatcagctcatcgagagcctgcgcgacggacgcactgacggtgtcgtccatcacagtttgccagtgatacacatggggatcagcaatcgcgcatatgaaatcacgccatgtagtgtattgaccgattccttgcggtccgaatgggccgaacccgctcgtctggctaagatcggccgcagcgatcgcatccatggcctccgcgaccggctgcagaacagcgggcagttcggtttcaggcaggtcttgcaacgtgacaccctgtgcacggcgggagatgcaataggtcaggctctcgctgaattccccaatgtcaagcacttccggaatcgggagcgcggccgatgcaaagtgccgataaacataacgatctttgtagaaaccatcggcgcagctatttacccgcaggacatatccacgccctcctacatcgaagctgaaagcacgagattcttcgccctccgagagctgcatcaggtcggagacgctgtcgaacttttcgatcagaaacttctcgacagacgtcgcggtgagttcaggcattttgacggtgggatcctgtgatgtctgctcaagcggggtagctgttagtcaagctgcgatgaagtgggaaagctcgaactgaaaggttcaaaggaataagggatgggaaggatggagtatggatgtagcaaagtacttacttaggggaaataaaggttcttggatgggaagatgaatatactgaagatgggaaaagaaagagaaaagaaaagagcagctggtggggagagcaggaaaatatggcaacaaatgttggactgacgcaacgaccttgtcaaccccgccgacacaccgggcggacagacggggcaaagctgcctaccagggactgagggacctcagcaggtcgagtgcagagcaccggatgggtcgactgccagcttgtgttcccggtctgcgccgctggccagctcctgagcggcctttccggtttcatacaccgggcaaagcaggagaggcacgatatttggacgccctacagatgccggatgggccaattagggagcttacgcgccgggtactcgctctacctacttcggagaaggtactatctcgtgaatcttttaccagatcggaagcaattggacttctgtacctaggttaatggcatgctatttcgccgacggctatacacccctggcttcacattctccttcgcttactgccggtgattcgatgaagctccatattctccgatgatgcaatagattcttggtcaacgaggggcacaccagcctttccacttcggggcggaggggcggccggtcccggattaataatcatccactgcacctcagagccgccagagctgtctggcgcagtggcgcttattactcagcccttctctctgcgtccgtccgtctctccgcatgccagaaagagtcaccggtcactgtacagagcggccgccaccgcggtggagctccaattcgccctatagtgagtcgtattacgcgcgctcactggccgtcgttttacaacgtcgtgactgggaaaaccctggcgttacccaacttaatcgccttgcagcacatccccctttcgccagctggcgtaatagcgaagaggcccgcaccgatcgcccttcccaacagttgcgcagcctgaatggcgaatgggacgcgccctgtagcggcgcattaagcgcggcgggtgtggtggttacgcgcagcgtgaccgctacacttgccagcgccctagcgcccgctcctttcgctttcttcccttcctttctcgccacgttcgccggctttccccgtcaagctctaaatcgggggctccctttagggttccgatttagtgctttacggcacctcgaccccaaaaaacttgattagggtgatggttcacgtagtgggccatcgccctgatagacggtttttcgccctttgacgttggagtccacgttctttaatagtggactcttgttccaaactggaacaacactcaaccctatctcggtctattcttttgatttataagggattttgccgatttcggcctattggttaaaaaatgagctgatttaacaaaaatttaacgcgaattttaacaaaatattaacgcttacaatttaggtggcacttttcggggaaatgtgcgcggaacccctatttgtttatttttctaaatacattcaaatatgtatccgctcatgagacaataaccctgataaatgcttcaataatattgaaaaaggaagagtatgagtattcaacatttccgtgtcgcccttattcccttttttgcggcattttgccttcctgtttttgctcacccagaaacgctggtgaaagtaaaagatgctgaagatcagttgggtgcacgagtgggttacatcgaactggatctcaacagcggtaagatccttgagagttttcgccccgaagaacgttttccaatgatgagcacttttcgaccgaataaatacctgtgacggaagatcacttcgcagaataaataaatcctggtgtccctgttgataccgggaagccctgggccaacttttggcgaaaatgagacgttgatcggcacgtaagaggttccaactttcaccataatgaaataagatcactaccgggcgtattttttgagttgtcgagattttcaggagctaaggaagctaaaatggagaaaaaaatcactggatataccaccgttgatatatcccaatggcatcgtaaagaacattttgaggcatttcagtcagttgctcaatgtacctataaccagaccgttcagctggatattacggcctttttaaagaccgtaaagaaaaataagcacaagttttatccggcctttattcacattcttgcccgcctgatgaatgctcatccggaattacgtatggcaatgaaagacggtgagctggtgatatgggatagtgttcacccttgttacaccgttttccatgagcaaactgaaacgttttcatcgctctggagtgaataccacgacgatttccggcagtttctacacatatattcgcaagatgtggcgtgttacggtgaaaacctggcctatttccctaaagggtttattgagaatatgtttttcgtctcagccaatccctgggtgagtttcaccagttttgatttaaacgtggccaatatggacaacttcttcgcccccgttttcaccatgggcaaatattatacgcaaggcgacaaggtgctgatgccgctggcgattcaggttcatcatgccgtttgtgatggcttccatgtcggcagaatgcttaatgaattacaacagtactgcgatgagtggcagggcggggcgtaatttttttaaggcagttattggtgcccttaaacgcctggttgctacgcctgaataagtgataataagcggatgaatggcagaaattcgaaagcaaattcgacccggtcgtcggttcagggcagggtcgttaaatagccgcttatgtctattgctggtttaccggtttattgactaccggaagcagtgtgaccgtgtgcttctcaaatgcctgaggccagtttgctcaggctctccccgtggaggtaataattgacgatatgatcctttttttctgatcaaaaaggatctaggtgaagatcctttttgataatctcatgaccaaaatcccttaacgtgagttttcgttccactgagcgtcagaccccgtagaaaagatcaaaggatcttcttgagatcctttttttctgcgcgtaatctgctgcttgcaaacaaaaaaaccaccgctaccagcggtggtttgtttgccggatcaagagctaccaactctttttccgaaggtaactggcttcagcagagcgcagataccaaatactgttcttctagtgtagccgtagttaggccaccacttcaagaactctgtagcaccgcctacatacctcgctctgctaatcctgttaccagtggctgctgccagtggcgataagtcgtgtcttaccgggttggactcaagacgatagttaccggataaggcgcagcggtcgggctgaacggggggttcgtgcacacagcccagcttggagcgaacgacctacaccgaactgagatacctacagcgtgagctatgagaaagcgccacgcttcccgaagggagaaaggcggacaggtatccggtaagcggcagggtcggaacaggagagcgcacgagggagcttccagggggaaacgcctggtatctttatagtcctgtcgggtttcgccacctctgacttgagcgtcgatttttgtgatgctcgtcaggggggcggagcctatggaaaaacgccagcaacgcggcctttttacggttcctggccttttgctggccttttgctcacatgttctttcctgcgttatcccctgattctgtggataaccgtattaccgcctttgagtgagctgataccgctcgccgcagccgaacgaccgagcgcagcgagtcagtgagcgaggaagcggaagagcgcccaatacgcaaaccgcctctccccgcgcgttggccgattcattaatgcagctggcacgacaggtttcccgactggaaagcgggcagtgagcgcaacgcaattaatgtgagttagctcactcattaggcaccccaggctttacactttatgctcccggctcgtatgttgtgtggaattgtgagcggataacaatttcacacaggaaacagctatgaccatgattacgccaagcgcgcaattaaccctcactaaagggaacaaaagctg

SEQ ID NO: 72 - DNA, 19158 bp, Artificial Sequence
  Nucleotide sequence of BG-AMA19 (Cas9/hygB/T7 strong sgRNA fwnA) G- olden Gate product BG-AMA17 with gBlock T7.pro strong sgRNA fwnA
ggtaccgaggttcatggtatgggcacgaatgtcaaaaattttcaggctcaaacgggtatgtattcagtatctatctccgtgtacgacggctaattgagcccagctgcatttcgaactcttctcccagcgcattttgtgtgggagttcttcgatgctgaccatgactgcgaggctgctgagggagtgcgcggtatctaccccggcccgtatctggcttctacaaggagtgaaactagtttatactttgtagttcggaatccaatgctattaaccgtttttactttttcttttgttcgagctaagcgcttgtttaaaccttgcgcttcttcttgggatcggcacgagagtcaccaccgagctgagacaggtcgatacgagtctcgtacagaccggtaatcgactggtggatcagagtcgcatcaagcacttccttggtggaggtgtaacgcttgcggtcgatggtggtgtcaaagtacttgaaagcagcaggagcacccaggttggtgagggtgaacaggtggatgatgttctccgcctgctcgcggatgggcttgtcacggtgcttgttgtaggcagagaggaccttgtcaaggttggcatcggccaggatgacacgcttgctgaactcggagatctgctcgatgatctcatccaggtagtgcttgtgctgctcgacaaagagctgcttctgctcgttgtcctcgggagagcccttgagcttctcgtagtgggaggccaggtagaggaagttgacgtacttggaggggagggcaagctcgttacccttctggagctcaccggcggaagcaagcatgcgcttacggccgttctccagctcgaacagagagtacttggggagcttgatgatgaggtccttcttgacctctttgtaacccttggcctccaggaagtcgatagggttcttctcgaagctgctgcgttccatgatggtgataccgaggagttccttcacactcttcagcttcttgctcttgcccttctcgaccttggcgacaaccaagacggagtaggcaacggtaggcgaatcgaatccaccgtacttcttggggtcccaatccttcttgcgagcgatcagcttgtcggagttgcgcttgggaagaatcgactccttggagaaaccaccagtctgcacctcggtcttcttgacaatgttgacctggggcatagaaaggaccttgcggacggtagcgaagtcacggcccttgtcccagacgatctcaccggtttcgccgttagtctcaatcaagggacgcttgcgaatctcgccgttggccaatgttatttcggtcttgaagaagttcatgatgttgctgtagaagaagtacttggcagtggcctttccgatctcctgctcggacttagcgatcatcttgcgcacgtcgtacaccttgtagtcaccgtagacgaactcggactcgagcttgggatacttcttaatcaaagcagtaccgacgacggcgttgaggtaggcatcgtgagcgtggtggtagttgttgatctcgcggaccttgtagaactggaagtctttcctaaagtcactgaccagcttgctctttaaggtgatgaccttgacctcacggatgagcttgtcgttctcgtcgtacttggtgttcatgcgagagtccaggatctgggcaacgtgcttagtgatctgacgggtttcaaccaattgacgcttgatgaaaccggccttgtcgagctcggagagtccgccacgctcggccttggtaaggttgtcgaacttgcgctgagtgatgagcttagcgttgagcaattgtctccagtagttcttcatcttcttaacaacctcttccgaggggacgttatcgctcttgccacgattcttgtcggaacgggtgagcaccttgttgtcaatgctgtcatccttgaggaaggactgggggacgatgtggtcaacatcgtagtcggagaggcggttgatatccagctcctggtcgacgtacatgtcacgtccgttctgcaagtagtagaggtagagcttctcattctgcagctgggtgttctcgacggggtgttccttgagaatctgggaaccgagctccttgatgccttcctcgatacgcttcatgcgctcacggctgttcttctgacccttctgagtggtctggttctcacgagccatttcgatgacgatgttctcgggcttgtgacgacccatgaccttcacaagctcgtcaacaaccttcacagtctgcaggatacccttcttgatagcgggggaaccagccaggttggcaatgtgttcgtgtagcgagtcaccctggccggagacttgggccttctggatgtcctctttgaaggtcagagagtcgtcgtggatgagctgcatgaagttgcggttggcgaagccgtcggacttcaggaagtcaaggatggtcttgccagactgcttatcacggataccgttaatcaacttgcgagagaggcgaccccagccagtgtaacggcggcgcttcaactgcttcatgaccttgtcgtcgaagaggtgagcgtaggtcttcagacgttcttcgatcatctcacggtcctcgaagagggtgagggtaagaacaatgtcctcaagaatgtcttcgttctcctcgttgtcaaggaagtccttgtccttgatgatcttgagcagatcgtggtaggtgccgagagaagcgttgaagcggtcctcaacaccggagatctcaacggagtcaaagcactcgatcttcttgaagtagtcttccttgagctgcttgacggtcaccttgcggttagtcttgaacagcaggtcgacaatggccttcttctgttcgccggagaggaaagcaggcttgcgcatgccctcggtcacgtacttgaccttggtcagctcgttgtagacagtgaagtactcgtacaagagggagtgcttgggcaggactttctcgttgggcaggttcttgtcgaagttggtcatacgctcaatgaagctctgagcggaggcacccttgtcgacgacttcctcgaagttccagggggtgatggtttcctcggacttgcgggtcatccaggcgaagcgggagttaccgcgagccagaggaccgacgtagtaggggatacggaaggtcaggatcttctcaatcttctcacggttgtccttcaagaaagggtagaagtcttcctggcgacgaaggatggcgtgcaattcacccaggtggatctggtgggggatgctgccgttgtcgaaagtacgctgcttgcgcagaaggtcctcacggttcagcttaacaagaagctcctcagtgccatccatcttctcgaggataggcttaatgaacttgtagaattcttcctgggaagcaccaccgtcgatgtaaccggcgtagccgttcttggactggtcgaagaagatctccttgtacttttcggggagctgctggcggaccagagccttgagtagggtgaggtcctggtggtgctcatcgtatctcttgatcatagaggcggagagaggggccttggtgatctcagtgttgacacggaggatatctgacaggagaatggcatcggagaggttcttggcagctaggaagaggtcggcgtactgatctcctatctgggcgagaaggttatcaaggtcgtcgtcgtaggtatccttggaaagttgtaacttagcatcctcagcaagatcgaagttgctcttgaagttgggagtcagtccgagggacagggcaataaggttgccgaaaagaccgttcttcttctcaccagggagctgggcaatcaagttctcaagacggcgggacttgctcaggcgagcggagaggatggccttggcatccacgccagacgcgttgatggggttttcctcgaaaagctggttgtaggtctgaacgagctggatgaagagtttatcaacatcggagttgtcggggttgaggtcaccctcgatcaggaagtgaccacggaacttgatcatgtgcgccagagccaggtaaatgaggcggaggtcagccttgtcggtgctgtcgacgagctttttgcgtaggtggtagatggtggggtacttctcgtggtaagcgacctcatcgacaatgttaccgaagatagggtgacgctcgtgcttcttgtcttcttcaacaaggaacgactcctccagacggtggaagaaagagtcatcaaccttggccatctcgttggagaaaatctcctggaggtagcagatacggttcttgcggcgagtgtaacgacggcgagcggtacgcttcagacgggtggcctcagcagtctcaccggagtcgaagagaagcgcaccaatgaggttcttcttgatggagtgacgatcggtgtttcccaggaccttgaatttcttgctaggaaccttgtactcgtcggtgatgacagcccagccaacggagttggtgccaatgtccagaccgatgctatacttcttgtccattttgacggtggaaggtgagttggggttggtgtcatcgtgggggaagaacttggcttttatatgggtgcaggtgaggggacttaagccacgtgaaagttcattcgagagagctaaggcatattaatgcacatgtgtgggagttgcatggaacttgcatgaaaggtgcatgaaaggtgcatggtattgcagaatgcgctcgggggtctgcggagaaatccgttaggaaaagatcgtcatccttctgctgcatcaccgttagcttgaaatttagttccagcgctagtcaagggcttcagttcagattctgcaagtatcaggtccatcattactctcttcagcaggcggatcgaatatcccccgaggcacatgggaggtcttattatccgatcgttgatcaccatgccaatcgcttcgaccgaccacaagttgcatcaagcactaactgcctcaagcagatgccgagtcttcatctccgatatttaatcccgttgaatctccgccccctgtcatctccaccgtttaatctggggtggtggcggatgtccaccaattagccggctaaattatccccatcgtcagcacgctagacctgccttggaactagcgctttggtgagaaatctcttggttgtgagtctgataccacattccttgacttccatgttgttctggaggtgtgaaagtataaacaatgccacagatggactaatctccggagagatgaccctcttcaagactggtgcagtgcctaggatcgctagtatcccaaaacttcggggctgccttcatttccagagagttgcggtaccttgcccatcgaacgtacaagtactcctctgttctctccttcctttgctttgtgctaatacgactcactataggggaatcagatatattcagtcactggttttagagctagaaatagcaagttaaaataaggctagtccgttatcaacttgaaaaagtggcaccgagtcggtgcttttggccggcatggtcccagcctcctcgctggcgccggctgggcaacatgcttcggcatggcgaatgggacaaaaaatcaaactggctcaccttcgggtgggcctttttgcgtttatacctccggatcgatgtacacaaccgactgcacccaaacgaacacaaatcttagcagtgccctcgccggatagcttggactgtcctttaccgtcgccagcacaagaagggtatctctgaggtccgtaccgccttttctttaccactggattcgattttcgcagttggaatgatacatctggggactgcgaatggtttacccctcggccgatactatgggtcgtgaagagatggaacattccgaaagtgttttgcggataacattggtggcatcgaaaacagaatgctgaccattgatttcaacacgaacaggaggttgccaagaagcgtacccgccgtgtcgtcaagtcccagcgtgccatcgtcggtgcttccctcgacgtgatcaaggagcgccgctcccagcgccccgaggcccgtgccgccgcccgccagcaggccatcaaggacgccaaggagaagaaggctgccgctgagtccaagaagaaggctgagaaggctaagaacgccgctgctggtgccaagggtgctgctcagcgcatccagagcaagcagggtgctaagggttctgctcccaaggtcgctgccaagtctcgttaaggaatgaataacggttcggcttgggattgggtgcggaaggcaagagtttcatggacgaattttgggaggttactggagctggaatatgtgttttccctaccaccaaaaatgaaatgttccaaaactatcggcgtgcaagacggcctcttacgggtttaacggctctcagataagctctatcaatcgcgccacggatgcatgaatgaagatccagatggccgcgggatatatcgtgctagtgtaattcctacatgatcttgctgttcactccatgcgcatccagatattccaggggtcgactgttaattgatatgcctgggcttgagactccgtagacgcccagtcaatgtgcaattaatacgagggtgctgttatcggcagcaaccttgtacttctccataagatgggggaatgccatggacctgagtgatcaattgacgcaagtctcccataacgcggcggcttgacctaaaatccatataccgccccgttgagcctccgcgctccagagtcctgtcccggaatagggcacaaacctaggctaacctaattcgtcgtccgcgtctgagttcagacaaaagaacttccaagtatcagcagagtacgctgatattgataagtaggcaaacataagaccaataagcaagtagaataaaaaattataaggacactgcctccataaagcgccctcccaagacctcagggacaaaacttctcaagtggcaattcactgcctcaggccgtgtccagtgaagtgacgaagcgacactgttgcctgctgactcagccgctttccgccctgccgaatttgccatctcgcttacaggtcagcactagcgcgattcgcccacagatgctcagcgcaaagtggtgactcagtcaaaccccccctacaagattccacctcgatttttcaacttcccatctcgatccgacaagttctacatccaccgtcaaaatggcctccagcgaagatgtcatcaaggagttcatgcgcttcaaggtccgcatggaaggatccgtcaacggccacgagttcgagattgagggtgagggtgagggccgcccctacgaaggcacccagactgccaagctcaaggtcaccaagggtggtcctctccccttcgcttgggatatcctgtctcctcagttccagtacggctccaaggtctacgtcaagcaccccgccgacatccccgactacaagaagctttctttccccgagggtttcaagtgggagcgtgtcatgaacttcgaggatggtggtgttgtgaccgttactcaggacagcagcttgcaggatggctctttcatctacaaggtcaagttcattggtgtcaacttcccctccgacggccctgtcatgcagaagaagaccatgggctgggaagcgtcgactgagcgtctgtacccccgtgacggtgttctcaagggtgagatccacaaggctctcaagctcaaggacggtggtcactaccttgttgagttcaagtccatctacatggccaagaagcctgtgcagctgcccggatactactacgtggactccaagcttgacatcacctcccacaacgaagactacaccattgttgagcagtacgagcgtgctgagggccgccaccacctcttcctgacccacggaatggatgagctgtacaagtcgaaactataaataaatggtttgcgttgcgattgactgaaacgaaaaaaagcgaaaatgattctgggaatgaattgataaagcgcgggctctgcggtacggttacggttgcggtcgcggacgaatggactgggctgagctgggctggaggaagtccatcgaacaaggacaaggggtggaatatggcacgggtcgattttgttatacataccctaccatccatctatccatttaaataccaaatgagttgttgaatggattcgcggtcttctcggtttatttttgcttgcttgcgtgcttaagggatagtgtgcctcacgctttccggcatcttccagaccacagtatatccatccgcctcctgttgaagcttattttttgtatactgttttgtgatagcacgaagtttttccacggtatcttgttaaaaatatatatttgtggcgggcttacctacatcaaattaataagagactaattataaactaaacacacaagcaagctactttagggtaaaagtttataaatgcttttgacgtataaacgttgcttgtatttattattacaattaaaggtggatagaaaacctagagactagttagaaactaatctcaggtttgcgttaaactaaatcagagcccgagaggttaacagaacctagaaggggactagatatccgggtagggaaacaaaaaaaaaaaacaagacagccacatattagggagactagttagaagctagttccaggactaggaaaataaaagacaatgataccacagtctagttgacaactagatagattctagattgaggccaaagtctctgagatccaggttagttgcaactaatactagttagtatctagtctcctataactctgaagctagaataacttactactattatcctcaccactgttcagctgcgcaaacggagtgattgcaaggtgttcagagactagttattgactagtcagtgactagcaataactaacaaggtattaacctaccatgtctgccatcaccctgcacttcctcgggctcagcagccttttcctcctcattttcatgctcattttccttgtttaagactgtgactagtcaaagactagtccagaaccacaaaggagaaatgtcttaccactttcttcattgcttgtctcttttgcattatccatgtctgcaactagttagagtctagttagtgactagtccgacgaggacttgcttgtctccggattgttggaggaactctccagggcctcaagatccacaacagagccttctagaagactggtcaataactagttggtctttgtctgagtctgacttacgaggttgcatactcgctccctttgcctcgtcaatcgatgagaaaaagcgccaaaactcgcaatatggctttgaaccacacggtgctgagactagttagaatctagtcccaaactagcttggatagcttacctttgccctttgcgttgcgacaggtcttgcagggtatggttcctttctcaccagctgatttagctgccttgctaccctcacggcggatctgcataaagagtggctagaggttataaattagcactgatcctaggtacggggctgaatgtaacttgcctttcctttctcatcgcgcggcaagacaggcttgctcaaattcctaccagtcacaggggtatgcacggcgtacggaccacttgaactagtcacagattagttagcaactagtctgcattgaatggctgtacttacgggccctcgccattgtcctgatcatttccagcttcaccctcgttgctgcaaagtagttagtgactagtcaaggactagttgaaatgggagaagaaactcacgaattctcgacacccttagtattgtggtccttggacttggtgctgctatatattagctaatacactagttagactcacagaaacttacgcagctcgcttgcgcttcttggtaggagtcggggttgggagaacagtgccttcaaacaagccttcataccatgctacttgactagtcagggactagtcaccaagtaatctagataggacttgcctttggcctccatcagttccttcatagtgggaggtccattgtgcaatgtaaactccatgccgtgggagttcttgtccttcaagtgcttgaccaatatgtttctgttggcagagggaacctgtcaactagttaataactagtcagaaactagtatagcagtagactcactgtacgcttgaggcatcccttcactcggcagtagacttcatatggatggatatcaggcacgccattgtcgtcctgtggactagtcagtaactaggcttaaagctagtcgggtcggcttactatcttgaaatccggcagcgtaagctccccgtccttaactgcctcgagatagtgacagtactctggggactttcggagatcgttatcgcgaatgctcggcatactaatcgttgactagtcttggactagtcccgagcaaaaaggattggaggaggaggaggaaggtgagagtgagacaaagagcgaaataagagcttcaaaggctatctctaagcagtatgaaggttaagtatctagttcttgactagatttaaaagagatttcgactagttatgtacctggagtttggatataggaatgtgttgtggtaacgaaatgtaagggggaggaaagaaaaagtcggtcaagaggtaactctaagtcggccattcctttttgggaggcgctaaccataaacggcatggtcgacttagagttagctcagggaatttagggagttatctgcgaccaccgaggaacggcggaatgccaaagaatcccgatggagctctagctggcggttgacaaccccaccttttggcgtttctgcggcgttgcaggcgggactggatacttcgtagaaccagaaaggcaaggcagaacgcgctcagcaagagtgttggaagtgatagcatgatgtgccttgttaactaggtcaaaatctgcagtatgcttgatgttatccaaagtgtgagagaggaaggtccaaacatacacgattgggagagggcctaggtataagagtttttgagtagaacgcatgtgagcccagccatctcgaggagattaaacacgggccggcatttgatggctatgttagtaccccaatggaaagcctgagagtccagtggtcgcagataactccctaaattccctgagctaactctaagtcgaccatgccgtttatggttagcgcctcccaaaaaggaatggccgacttagagttacctcttgaccgactttttctttcctcccccttacatttcgttaccacaacacattcctatatccaaactccaggtacataactagtcgaaatctcttttaaatctagtcaagaactagatacttaaccttcatactgcttagagatagcctttgaagctcttatttcgctctttgtctcactctcaccttcctcctcctcctccaatcctttttgctcgggactagtccaagactagtcaacgattagtatgccgagcattcgcgataacgatctccgaaagtccccagagtactgtcactatctcgaggcagttaaggacggggagcttacgctgccggatttcaagatagtaagccgacccgactagctttaagcctagttactgactagtccacaggacgacaatggcgtgcctgatatccatccatatgaagtctactgccgagtgaagggatgcctcaagcgtacagtgagtctactgctatactagtttctgactagttattaactagttgacaggttccctctgccaacagaaacatattggtcaagcacttgaaggacaagaactcccacggcatggagtttacattgcacaatggacctcccactatgaaggaactgatggaggccaaaggcaagtcctatctagattacttggtgactagtccctgactagtcaagtagcatggtatgaaggcttgtttgaaggcactgttctcccaaccccgactcctaccaagaagcgcaagcgagctgcgtaagtttctgtgagtctaactagtgtattagctaatatatagcagcaccaagtccaaggaccacaatactaagggtgtcgagaattcgtgagtttcttctcccatttcaactagtccttgactagtcactaactactttgcagcaacgagggtgaagctggaaatgatcaggacaatggcgagggcccgtaagtacagccattcaatgcagactagttgctaactaatctgtgactagttcaagtggtccgtacgccgtgcatacccctgtgactggtaggaatttgagcaagcctgtcttgccgcgcgatgagaaaggaaaggcaagttacattcagccccgtacctaggatcagtgctaatttataacctctagccactctttatgcagatccgccgtgagggtagcaaggcagctaaatcagctggtgagaaaggaaccataccctgcaagacctgtcgcaacgcaaagggcaaaggtaagctatccaagctagtttgggactagattctaactagtctcagcaccgtgtggttcaaagccatattgcgagttttggcgctttttctcatcgattgacgaggcaaagggagcgagtatgcaacctcgtaagtcagactcagacaaagaccaactagttattgaccagtcttctagaaggctctgttgtggatcttgaggccctggagagttcctccaacaatccggagacaagcaagtcctcgtcggactagtcactaactagactctaactagttgcagacatggataatgcaaaagagacaagcaatgaagaaagtggtaagacatttctcctttgtggttctggactagtctttgactagtcacagtcttaaacaaggaaaatgagcatgaaaatgaggaggaaaaggctgctgagcccgaggaagtgcagggtgatggcagacatggtaggttaataccttgttagttattgctagtcactgactagtcaataactagtctctgaacaccttgcaatcactccgtttgcgcagctgaacagtggtgaggataatagtagtaagttattctagcttcagagttataggagactagatactaactagtattagttgcaactaacctggatctcagagactttggcctcaatctagaatctatctagttgtcaactagactgtggtatcattgtcttttattttcctagtcctggaactagcttctaactagtctccctaatatgtggctgtcttgttttttttttttgtttccctacccggatatctagtccccttctaggttctgttaacctctcgggctctgatttagtttaacgcaaacctgagattagtttctaactagtctctaggttttctatccacctttaattgtaataataaatacaagcaacgtttatacgtcaaaagcatttataaacttttaccctaaagtagcttgcttgtgtgtttagtttataattagtctcttattaatttgatgtaggtaagcccgccacaaatatatatttttaacaagataccgtggaaaaacttcgtgctatcacaaaacagtatacaaaaaataagctatcgaattcctgcagagatcatcctgtcttcagtcttaagacttctctcctatatcacccgcacttaccctagagtgccgcttaggtgctaagggcacattgagtattggccgtgtagaatatatagcttaagtacggccaagcagacgggaagccctgttctccacaccctatggtcgtatatatcaggcttctaccgggaaacgattaagagtgtataatggactgaaaatcaatatgaacgggacaatgctcaagttaaattagttaggcatcctaatctctactaaatgttctatctagagatcggggtactataggcccgtacgttaatcactctacgcttctctcccttaggtatagtgtaggtaggggctagacatttatatgagtcagatggtacaaacggtaggcagtgcgggcgaagaagtgaagacggagtcggttgaagctacatacaaaagatgcattggctcgtcatgaagagcctcccgggtttattcctttgccctcggacgagtgctggggcgtcggtttccactatcggcgagtacttctacacagccatcggtccagacggccgcgcttctgcgggcgatttgtgtacgcccgacagtcccggctccggatcggacgattgcgtcgcatcgaccctgcgcccaagctgcatcatcgaaattgccgtcaaccaagctctgatagagttggtcaagaccaatgcggagcatatacgcccggagccgcggcgatcctgcaagctccggatgcctccgctcgaagtagcgcgtctgctgctccatacaagccaaccacggcctccagaagaagatgttggcgacctcgtattgggaatccccgaacatcgcctcgctccagtcaatgaccgctgttatgcggccattgtccgtcaggacattgttggagccgaaatccgcgtgcacgaggtgccggacttcggggcagtcctcggcccaaagcatcagctcatcgagagcctgcgcgacggacgcactgacggtgtcgtccatcacagtttgccagtgatacacatggggatcagcaatcgcgcatatgaaatcacgccatgtagtgtattgaccgattccttgcggtccgaatgggccgaacccgctcgtctggctaagatcggccgcagcgatcgcatccatggcctccgcgaccggctgcagaacagcgggcagttcggtttcaggcaggtcttgcaacgtgacaccctgtgcacggcgggagatgcaataggtcaggctctcgctgaattccccaatgtcaagcacttccggaatcgggagcgcggccgatgcaaagtgccgataaacataacgatctttgtagaaaccatcggcgcagctatttacccgcaggacatatccacgccctcctacatcgaagctgaaagcacgagattcttcgccctccgagagctgcatcaggtcggagacgctgtcgaacttttcgatcagaaacttctcgacagacgtcgcggtgagttcaggcattttgacggtgggatcctgtgatgtctgctcaagcggggtagctgttagtcaagctgcgatgaagtgggaaagctcgaactgaaaggttcaaaggaataagggatgggaaggatggagtatggatgtagcaaagtacttacttaggggaaataaaggttcttggatgggaagatgaatatactgaagatgggaaaagaaagagaaaagaaaagagcagctggtggggagagcaggaaaatatggcaacaaatgttggactgacgcaacgaccttgtcaaccccgccgacacaccgggcggacagacggggcaaagctgcctaccagggactgagggacctcagcaggtcgagtgcagagcaccggatgggtcgactgccagcttgtgttcccggtctgcgccgctggccagctcctgagcggcctttccggtttcatacaccgggcaaagcaggagaggcacgatatttggacgccctacagatgccggatgggccaattagggagcttacgcgccgggtactcgctctacctacttcggagaaggtactatctcgtgaatcttttaccagatcggaagcaattggacttctgtacctaggttaatggcatgctatttcgccgacggctatacacccctggcttcacattctccttcgcttactgccggtgattcgatgaagctccatattctccgatgatgcaatagattcttggtcaacgaggggcacaccagcctttccacttcggggcggaggggcggccggtcccggattaataatcatccactgcacctcagagccgccagagctgtctggcgcagtggcgcttattactcagcccttctctctgcgtccgtccgtctctccgcatgccagaaagagtcaccggtcactgtacagagcggccgccaccgcggtggagctccaattcgccctatagtgagtcgtattacgcgcgctcactggccgtcgttttacaacgtcgtgactgggaaaaccctggcgttacccaacttaatcgccttgcagcacatccccctttcgccagctggcgtaatagcgaagaggcccgcaccgatcgcccttcccaacagttgcgcagcctgaatggcgaatgggacgcgccctgtagcggcgcattaagcgcggcgggtgtggtggttacgcgcagcgtgaccgctacacttgccagcgccctagcgcccgctcctttcgctttcttcccttcctttctcgccacgttcgccggctttccccgtcaagctctaaatcgggggctccctttagggttccgatttagtgctttacggcacctcgaccccaaaaaacttgattagggtgatggttcacgtagtgggccatcgccctgatagacggtttttcgccctttgacgttggagtccacgttctttaatagtggactcttgttccaaactggaacaacactcaaccctatctcggtctattcttttgatttataagggattttgccgatttcggcctattggttaaaaaatgagctgatttaacaaaaatttaacgcgaattttaacaaaatattaacgcttacaatttaggtggcacttttcggggaaatgtgcgcggaacccctatttgtttatttttctaaatacattcaaatatgtatccgctcatgagacaataaccctgataaatgcttcaataatattgaaaaaggaagagtatgagtattcaacatttccgtgtcgcccttattcccttttttgcggcattttgccttcctgtttttgctcacccagaaacgctggtgaaagtaaaagatgctgaagatcagttgggtgcacgagtgggttacatcgaactggatctcaacagcggtaagatccttgagagttttcgccccgaagaacgttttccaatgatgagcacttttcgaccgaataaatacctgtgacggaagatcacttcgcagaataaataaatcctggtgtccctgttgataccgggaagccctgggccaacttttggcgaaaatgagacgttgatcggcacgtaagaggttccaactttcaccataatgaaataagatcactaccgggcgtattttttgagttgtcgagattttcaggagctaaggaagctaaaatggagaaaaaaatcactggatataccaccgttgatatatcccaatggcatcgtaaagaacattttgaggcatttcagtcagttgctcaatgtacctataaccagaccgttcagctggatattacggcctttttaaagaccgtaaagaaaaataagcacaagttttatccggcctttattcacattcttgcccgcctgatgaatgctcatccggaattacgtatggcaatgaaagacggtgagctggtgatatgggatagtgttcacccttgttacaccgttttccatgagcaaactgaaacgttttcatcgctctggagtgaataccacgacgatttccggcagtttctacacatatattcgcaagatgtggcgtgttacggtgaaaacctggcctatttccctaaagggtttattgagaatatgtttttcgtctcagccaatccctgggtgagtttcaccagttttgatttaaacgtggccaatatggacaacttcttcgcccccgttttcaccatgggcaaatattatacgcaaggcgacaaggtgctgatgccgctggcgattcaggttcatcatgccgtttgtgatggcttccatgtcggcagaatgcttaatgaattacaacagtactgcgatgagtggcagggcggggcgtaatttttttaaggcagttattggtgcccttaaacgcctggttgctacgcctgaataagtgataataagcggatgaatggcagaaattcgaaagcaaattcgacccggtcgtcggttcagggcagggtcgttaaatagccgcttatgtctattgctggtttaccggtttattgactaccggaagcagtgtgaccgtgtgcttctcaaatgcctgaggccagtttgctcaggctctccccgtggaggtaataattgacgatatgatcctttttttctgatcaaaaaggatctaggtgaagatcctttttgataatctcatgaccaaaatcccttaacgtgagttttcgttccactgagcgtcagaccccgtagaaaagatcaaaggatcttcttgagatcctttttttctgcgcgtaatctgctgcttgcaaacaaaaaaaccaccgctaccagcggtggtttgtttgccggatcaagagctaccaactctttttccgaaggtaactggcttcagcagagcgcagataccaaatactgttcttctagtgtagccgtagttaggccaccacttcaagaactctgtagcaccgcctacatacctcgctctgctaatcctgttaccagtggctgctgccagtggcgataagtcgtgtcttaccgggttggactcaagacgatagttaccggataaggcgcagcggtcgggctgaacggggggttcgtgcacacagcccagcttggagcgaacgacctacaccgaactgagatacctacagcgtgagctatgagaaagcgccacgcttcccgaagggagaaaggcggacaggtatccggtaagcggcagggtcggaacaggagagcgcacgagggagcttccagggggaaacgcctggtatctttatagtcctgtcgggtttcgccacctctgacttgagcgtcgatttttgtgatgctcgtcaggggggcggagcctatggaaaaacgccagcaacgcggcctttttacggttcctggccttttgctggccttttgctcacatgttctttcctgcgttatcccctgattctgtggataaccgtattaccgcctttgagtgagctgataccgctcgccgcagccgaacgaccgagcgcagcgagtcagtgagcgaggaagcggaagagcgcccaatacgcaaaccgcctctccccgcgcgttggccgattcattaatgcagctggcacgacaggtttcccgactggaaagcgggcagtgagcgcaacgcaattaatgtgagttagctcactcattaggcaccccaggctttacactttatgctcccggctcgtatgttgtgtggaattgtgagcggataacaatttcacacaggaaacagctatgaccatgattacgccaagcgcgcaattaaccctcactaaagggaacaaaagctg

SEQ ID NO: 73 - DNA, 20 bp, Artificial Sequence
  Nucleotide sequence of forward primer used to check the cloned T7 gRNA cassette in AMA-vector (BG-AMA18 and BG-AMA19) by GoldenGate
ttgcccatcgaacgtacaag

SEQ ID NO: 74 - DNA, 23 bp, Artificial Sequence
  Nucleotide sequence of reverse primer used to check the cloned T7 gRNA cassette in AMA-vector (BG-AMA18 and BG-AMA19) by GoldenGate
tgctaagatttgtgttcgtttgg

SEQ ID NO: 75 - DNA, 21 bp, Artificial Sequence
  Nucleotide sequence of forward primer to amplify part of the fwnA gene to produce DNA fragments for sequencing and primer also used for sequencing reaction to check correct integration of door DNA in the genome
acagtcttgcgagccttcatc

SEQ ID NO: 76 - DNA, 23 bp, Artificial Sequence
  Nucleotide sequence of reverse primer to amplify part of the fwnA gene to produce DNA fragments for sequencing
caactggaggtaggaccgtatcg